European Patent Specification EP 4 308 729 B1, published October 29, 2025. Title: COMPOSITIONS AND METHODS FOR DISCRIMINATING BACTERIAL AND VIRAL INFECTIONS IN A HUMAN SUBJECT. Applicant: Cepheid Wallace, Stacey Baig, Rebekah Lu, Xixi Kaldate, Rajesh. The sequence listing filed with the application follows.

SEQUENCE LISTING (6 sequences)

SEQ ID NO: 1 - DNA, 1005 bp, Homo sapiens
atgcgtatccccgtagatgccagcacgagccgccgcttcacgccgccttccaccgcgctgagcccaggcaagatgagcgaggcgttgccgctgggcgccccggacgccggcgctgccctggccggcaagctgaggagcggcgaccgcagcatggtggaggtgctggccgaccacccgggcgagctggtgcgcaccgacagccccaacttcctctgctccgtgctgcctacgcactggcgctgcaacaagaccctgcccatcgctttcaaggtggtggccctaggggatgttccagatggcactctggtcactgtgatggctggcaatgatgaaaactactcggctgagctgagaaatgctaccgcagccatgaagaaccaggttgcaagatttaatgacctcaggtttgtcggtcgaagtggaagagggaaaagcttcactctgaccatcactgtcttcacaaacccaccgcaagtcgccacctaccacagagccatcaaaatcacagtggatgggccccgagaacctcgaaactctttgacctggcctcggtatcctcacatttaaaatgaggagttggcttatatgattggctggcatatttggctcatctcgaagactgtctattatagaagggcaaatggtagtgcctcattgcaggtgtggagcctttgacttgaggtatgcgtgcaatctgccacaacttgtatcttaaaggcagtctcaaggaatctgaaaaggcagaaagaatatgaagagaaacagaaaaattaaaagctctggaatccagcaggtgattctccaaggcaaaacataagtttttttttaatcacagtattatagattattatatttgaaaaaaaaacttagaaatcacctggtcttccctataaaggaattcttttcataatgtatctgctaaatcacagctttaatactagttatgaactattaaaaggtctaaatttttttattgtggtaaaataataaaattcactattcgaa

SEQ ID NO: 2 - DNA, 4742 bp, Homo sapiens
ttttctgcccttctttgctttggtggcttccttgtggttcctcagtggtgcctgcaacccctggttcacctccttccaggttctggctccttccagccatggctctcagagtccttctgttaacagccttgaccttatgtcatgggttcaacttggacactgaaaacgcaatgaccttccaagagaacgcaaggggcttcgggcagagcgtggtccagcttcagggatccagggtggtggttggagccccccaggagatagtggctgccaaccaaaggggcagcctctaccagtgcgactacagcacaggctcatgcgagcccatccgcctgcaggtccccgtggaggccgtgaacatgtccctgggcctgtccctggcagccaccaccagcccccctcagctgctggcctgtggtcccaccgtgcaccagacttgcagtgagaacacgtatgtgaaagggctctgcttcctgtttggatccaacctacggcagcagccccagaagttcccagaggccctccgagggtgtcctcaagaggatagtgacattgccttcttgattgatggctctggtagcatcatcccacatgactttcggcggatgaaggagtttgtctcaactgtgatggagcaattaaaaaagtccaaaaccttgttctctttgatgcagtactctgaagaattccggattcactttaccttcaaagagttccagaacaaccctaacccaagatcactggtgaagccaataacgcagctgcttgggcggacacacacggccacgggcatccgcaaagtggtacgagagctgtttaacatcaccaacggagcccgaaagaatgcctttaagatcctagttgtcatcacggatggagaaaagtttggcgatcccttgggatatgaggatgtcatccctgaggcagacagagagggagtcattcgctacgtcattggggtgggagatgccttccgcagtgagaaatcccgccaagagcttaataccatcgcatccaagccgcctcgtgatcacgtgttccaggtgaataactttgaggctctgaagaccattcagaaccagcttcgggagaagatctttgcgatcgagggtactcagacaggaagtagcagctcctttgagcatgagatgtctcaggaaggcttcagcgctgccatcacctctaatggccccttgctgagcactgtggggagctatgactgggctggtggagtctttctatatacatcaaaggagaaaagcaccttcatcaacatgaccagagtggattcagacatgaatgatgcttacttgggttatgctgccgccatcatcttacggaaccgggtgcaaagcctggttctgggggcacctcgatatcagcacatcggcctggtagcgatgttcaggcagaacactggcatgtgggagtccaacgctaatgtcaagggcacccagatcggcgcctacttcggggcctccctctgctccgtggacgtggacagcaacggcagcaccgacctggtcctcatcggggccccccattactacgagcagacccgagggggccaggtgtccgtgtgccccttgcccagggggagggctcggtggcagtgtgatgctgttctctacggggagcagggccaaccctggggccgctttggggcagccctaacagtgctgggggacgtaaatggggacaagctgacggacgtggccattggggccccaggagaggaggacaaccggggtgctgtttacctgtttcacggaacctcaggatctggcatcagcccctcccatagccagcggatagcaggctccaagctctctcccaggctccagtattttggtcagtcactgagtgggggccaggacctcacaatggatggactggtagacctgactgtaggagcccaggggcacgtgctgctgctcaggtcccagccagtactgagagtcaaggcaatcatggagttcaatcccagggaagtggcaaggaatgtatttgagtgtaatgatcaggtggtgaaaggcaaggaagccggagaggtcagagtctgcctccatgtccagaagagcacacgggatcggctaagagaaggacagatccagagtgttgtgacttatgacctggctctggactccggccgcccacattcccgcgccgtcttcaatgagacaaagaacagcacacgcagacagacacaggtcttggggctgacccagacttgtgagaccctgaaactacagttgccgaattgcatcgaggacccagtgagccccattgtgctgcgcctgaacttctctctggtgggaacgccattgtctgctttcgggaacctccggccagtgctggcggaggatgctcagagactcttcacagccttgtttccctttgagaagaattgtggcaatgacaacatctgccaggatgacctcagcatcaccttcagtttcatgagcctggactgcctcgtggtgggtgggccccgggagttcaacgtgacagtgactgtgagaaatgatggtgaggactcctacaggacacaggtcaccttcttcttcccgcttgacctgtcctaccggaaggtgtccacgctccagaaccagcgctcacagcgatcctggcgcctggcctgtgagtctgcctcctccaccgaagtgtctggggccttgaagagcaccagctgcagcataaaccaccccatcttcccggaaaactcagaggtcacctttaatatcacgtttgatgtagactctaaggcttcccttggaaacaaactgctcctcaaggccaatgtgaccagtgagaacaacatgcccagaaccaacaaaaccgaattccaactggagctgccggtgaaatatgctgtctacatggtggtcaccagccatggggtctccactaaatatctcaacttcacggcctcagagaataccagtcgggtcatgcagcatcaatatcaggtcagcaacctggggcagaggagcctccccatcagcctggtgttcttggtgcccgtccggctgaaccagactgtcatatgggaccgcccccaggtcaccttctccgagaacctctcgagtacgtgccacaccaaggagcgcttgccctctcactccgactttctggctgagcttcggaaggcccccgtggtgaactgctccatcgctgtctgccagagaatccagtgtgacatcccgttctttggcatccaggaagaattcaatgctaccctcaaaggcaacctctcgtttgactggtacatcaagacctcgcataaccacctcctgatcgtgagcacagctgagatcttgtttaacgattccgtgttcaccctgctgccgggacagggggcgtttgtgaggtcccagacggagaccaaagtggagccgttcgaggtccccaaccccctgccgctcatcgtgggcagctctgtcgggggactgctgctcctggccctcatcaccgccgcgctgtacaagctcggcttcttcaagcggcaatacaaggacatgatgagtgaagggggtcccccgggggccgaaccccagtagcggctccttcccgacagagctgcctctcggtggccagcaggactctgcccagaccacacgtagcccccaggctgctggacacgtcggacagcgaagtatccccgacaggacgggcttgggcttccatttgtgtgtgtgcaagtgtgtatgtgcgtgtgtgcaagtgtctgtgtgcaagtgtgtgcacatgtgtgcgtgtgcgtgcatgtgcacttgcacgcccatgtgtgagtgtgtgcaagtatgtgagtgtgtccaagtgtgtgtgcgtgtgtccatgtgtgtgcaagtgtgtgcatgtgtgcgagtgtgtgcatgtgtgtgctcaggggcgtgtggctcacgtgtgtgactcagatgtctctggcgtgtgggtaggtgacggcagcgtagcctctccggcagaagggaactgcctgggctcccttgtgcgtgggtgaagccgctgctgggttttcctccgggagaggggacggtcaatcctgtgggtgaagacagagggaaacacagcagcttctctccactgaaagaagtgggacttcccgtcgcctgcgagcctgcggcctgctggagcctgcgcagcttggatggagactccatgagaagccgtgggtggaaccaggaacctcctccacaccagcgctgatgcccaataaagatgcccactgaggaatgatgaagcttcctttctggattcatttattatttcaatgtgactttaattttttggatggataagcttgtctatggtacaaaaatcacaaggcattcaagtgtacagtgaaaagtctccctttccagatattcaagtcacctccttaaaggtagtcaagattgtgttttgaggtttccttcagacagattccaggcgatgtgcaagtgtatgcacgtgtgcacacacaccacacatacacacacacaagcttttttacacaaatggtagcatactttatattggtctgtatcttgctttttttcaccaatatttctcagacatcggttcatattaagacataaattactttttcattcttttataccgctgcatagtattccattgtgtgagtgtaccataatgtatttaaccagtcttcttttgatatactattttcattctcttgttattgcatcaatgctgagttaataaatcaaatatatgtcatttttgcatatatgtaaggataa

SEQ ID NO: 3 - DNA, 2591 bp, Homo sapiens
aaactacaacgaaaaaagacagagctcataatggatgctatccataaacaaaagagcttacaattcaagaaaaccatggatgcaaagaagaactatgagcagaaatgccgggacaaagatgaggcagaacaggccgtcagccggagtgccaacctggtgaacccgaagcaacaagaaaagctttttgtgaaactggcaacttcaaagaccgcagtagaggactcagacaaagcatacatgctgcacatcggcaccctggataaggtccgagaagagtggcagagtgagcacatcaaggcctgcgaggcatttgaggctcaagaatgtgaacgaataaacttcttccggaatgcattgtggttacatgtgaatcagctgtcacaacaatgtgtcaccagtgatgaaatgtacgaacaagtccgaaagagtttagaaatgtgcagcattcagagggacattgaatactttgtgaatcaacgcaaaactggacagattccaccagcacccatcatgcatgagaatttctactcctcccagaagaatgcagtcccagcaggaaaggctacagggcctaacttggcaaggagaggacccctcccaattcctaaaagctcaccagatgatcccaattactctttggttgatgactacagtttgctctatcagtaaaatcaatgaaaccagagctttttccggctagtgcttctgtgatatggaaagggcacccagagcagcaggacctatagccacgttatgtcagcaatgaagactttgaagtgaacccttgctataattttttagagatttaaaatttatggtagacatttaggacaacataagcaagtagagttctgcagttttttgaagtttacaaattgccccattctgaagaattattctttcccagttactcaggttatgaatgaattaggttttcaacatgggaagcatgaaatccacttctggatttggagcatccacttgaggagcagaggtggcagcagaggattctgagccaccaactgcagtagtggctcctttggctttgggcagcctggctgtggagtttccacggcgacacacagcctcagtggtgcaagatttaaaattaccttcctttttggctggaagacttagaagccgcctgatcatactttctcattttacagatgaggaaataaagcctacaagtgtgaaattaatttccttacagttttcctagctgatgagggacagaaccagaactagagcctgagcccaacccacatcactattcttctaacccttcctgaagttgtgatgctcatgctgaaatttaagatgccaaatatttttgccagcactttttcagttgggagaatcaccagggtttaaatgtcagatttatttttatgtggatccctgtgtatgctgaactacagagcatgatgtttaatctaatttaaggagccactgattgtaaaacatgccattattttatgttgcactaagaaggtggggtcgaggagttgccaataaacttgggacagactattgatggccaagcccatctgaatttaagatgctaaagtatgaaaaaaatacatcttagaatcaatgaaataccatattttgattccattcctcaagataattttagagttataaaaccagtcctcaattttgggtcttcacagagaatctttcccttgctagaccccagaattttaaatgcatccgtcttacactttcacaaatatttgggttttcctttttcactcacaaacagcagggaggtcatgtactttttgtacaacacctgtgcactatgagaaaatggtaccttttagttattgacaagttaaaatagcactctcagtttttcagtattacagagagcaaatagtttcctctcctgctctgtgcagtagcttttccagaactatggacaaattgatcagaagaagattgattatttcctcatctttttttcttttttttgaggcagagtctctctctgtcccccaggctgaagtgcagcggcatgatctcagctcactgcaacctctgcctcccgggttcaagtgattctcctgcctcagcctcctgagtagctgggattacaggcacccaccaccacacctggctaattttttgtatttttagtagagacagggttttaccatgttggtcaggctggtctcaaactcctgacctcaggtgatccacctgcctcggcctcccaaagtgctgggattacaggcgtgagccactgcgcccggcctatttccccacctttcgtgtaaggtgctactgaacatgacagcttcttgtcatgacaggaaacttgcatcagttggatatccttttgagaaactgaattttgcaaagggccaaatttccccaaactgaacgggctcaggaaatgttcctttacactcagaacattctattttaagtatattatttattgttggcagttcctcagggatttcccttttctctgtattggtcagtgtagttgatgtaaaaccgttttgtggatggaaaatatttttattttattgctcttttagtttggtaggttaaataaaggttcttggtaatttggg

SEQ ID NO: 4 - DNA, 5543 bp, Homo sapiens
  misc_feature (354)..(354): n is a, c, g, or t
  misc_feature (732)..(733): n is a, c, g, or t
  misc_feature (899)..(899): n is a, c, g, or t
  misc_feature (906)..(906): n is a, c, g, or t
  misc_feature (913)..(913): n is a, c, g, or t
  misc_feature (936)..(937): n is a, c, g, or t
  misc_feature (1343)..(1343): n is a, c, g, or t
  misc_feature (1397)..(1397): n is a, c, g, or t
  misc_feature (1399)..(1401): n is a, c, g, or t
  misc_feature (1548)..(1549): n is a, c, g, or t
  misc_feature (5145)..(5145): n is a, c, g, or t
  misc_feature (5289)..(5291): n is a, c, g, or t
ctgcagagacagaaccccctgccctcaccgccaacattccagaggggaagatgccctgcctgtgccccacgtaagacccagaggcagggactcccccgggccacagcctactggaggctcctgtccccagagacagctgggccatcgccccaaagctgtggaagccccacccacgatgccatcataccacggccaggacatctcgtgacacacacagccccagcctcagcctccatacacacacacagbcaccacacacactcactcatgcaaaacacacacacagccacattgactgcacccctagatttgagacaggggtgttacaggtgtcttgtcagccccagccccctnctgaaccacatggccacctgccccaccctcacatttccccacaccctccccctactcccgtgtggggttcagaagacccctccctggtgctcgccctgtcacccagaaaggaaacgcactgtcaactggagaacaggcggtgcagagccccagcgcccacagccctcggagagggctggcgggaggagaggcacccaccgatgcagagcctcagtgccctcgcagaagccagcacccacaacctcccacctcccaaccccttgccggtctccccacccccgcctgagggatggccaaggaacagcccagctggagcgggaagcaggcacaagatgcacctcaggaatcccaggctgagggggtgcctgcgtcctccgnncccgagctccactccgcaggcgagacccccaacactgctccccgacactctccgaggcacccctcctccgtgctcacacccaaacacgtctgctcacccgtgggcttcccaccccgaacacaacgaggactgtccaggtgtcagtgacggtcaccccgacctggtnccctgcncggcctngccaggtcagcacccgtccgtcnncacagcagggtccgggtggaaggaggtccgggcctggtccgtggctcagctccacctcactgggaaactgggaggtggtctcagaacttctgggcctcagcttccccatctatcccaaggagccggggtagcctgggcggcgcggggacccccaccgggctcgccgactccgcccgcggaggcccctcccgtccgcccctgcccccccggggcgcgcggctgcctgggaggctccggccagccgcggtccagagcgcgcgaggttcggggagctccgccaggctgctggtacctgcgtccgcccggcggtgagtccgcgcggccccggcgggacgcccccgccacctgcgcgcaccgtcagacccggcggcctcggctgcggtgcacgcggcccggctcagccacngcggcggaaggccctgcgggggcgggggagagggtgggagagagcaagaggggngnnnggggaggggcaggagaggggctggggctgccggtgggttggtccccagagagctgagcttctcctcccatcccccgcaggcctccccgaatgtttccaaagatctggggcgggacggggcggagactgccgcaggagcctcccggcnnccccaggctgcgcagccactggagcccatcacccaactccagacgctcctggctcctctacgtgggccgggagggacagccttgaggactaggggagggggcacgggaccttgcagagctcctggccggaaagggaggattgaccgcccccggcatatcaccccggagcactggaacccgcccccgcttcttgttttggcactggtggtgcttgcggtgaggtccaaggagcccagcctccctgagtggaccgccgggcccctccccgttccgggacacaggagagctcccgccccttgctggctgggcagcccctagatacctggctcccaggggccagcttccctgagcctggggatgagccatgagcctgcagcctggccccagggcggccccccacggcctgccggctggctccctccggctccatggcccacccggccttcctaattgccttcgcgtcccaccggtgccttagctcagcctggtggcccagcggttgggtgccacccagtgagcaggtggcggcaccagctggacctgtttgtggccctgtatgctaggacttcctcagagacagctcagggaccccccccacctaccagaacctcacttagggggtgggggaaaaggaattggagatccttcctcctcggctactccctggaggcggggatagccccagccggacttggcactgtttttggccacctggggctcccactcccaaccccaggatgtcagcccaggtctcactgtcctggcctgctgctctccccttaggcctctgcgggcccctctccagatctgttctctgagggcatcctccttacccccagtgcccagcactagctccccaggcccgggatgtccctcccactcctctgcccacgcgtgtcccctgaagaaggcagcagctccccctccaacaccatgcactcacaaaacagagaatcacgaccccagctggtgtgttccagattctttctccagcagtgcagagggtcctgtgcagaggccgaggagcagtacagcgacccatctggccctttcctgctggtgggaaccagtggcaacgcagccttgtctctcggagcccatttcccagccacagaatggggagtagcagatactgagtggggtgctttcctcggaactgagtaacatcaggaatggggagtgctttccccctcagccatgccccacctggccccaggtctccatgtgaggggagctgcctgggctcaaaaccactgagccatcccaaggaaaattctagatacagattagctaatatacactgacagatacacatatagatgtgtatatagatttctcttttttttgagacagggtctcactctgttgcccaggctgcaggaatgcatggcatgatcatagtatacaacttcagtacttgaacatccctagagcatcaagagatccatcccacctcagacctcccaagatagcatgaccacaggcacgtaccacgcccggctaatttttgtattttttgtagaaaacaggaggtctccactgtgttgcccagggtggtctcaaacccctggcctcatatgatcctcctgccttggcctcacatagcatggagattacaggctgagccctgtacccagccccagactagctaatattatgactgatcaccattccccattccccattccccccaaccccaggaccactggcagaggccactcactctgccttcttttctgtggttctgagaaggctgctgagtttcctcctcttgcctgtgcagccccttccatgcaggtttcaggagggagatagcctagagcatgtctgcactgagtgaggagtgggtcaggagagaagtcagggaagccttgtgtgctggcaggtcccttcccctctgctgtctgtgtcctcatctgcaaagtgggggtgcatggtcttggggaggagtgaggcaccaccccgggcccccgtaaccagtgtgtctctccagagcaggacaggctgctttggtttgtgacctccaggcaggacggccatcctctccagaatgaagatcttcttgccagtgctgctggctgcccttctgggtgtggagcgaggtgaggtgcccttggggaccccagacctttgtccagctgtgccctgctccactccctctccacccctctcccctgagcagacgctccaggggtccttccaggccgctcccagcagagggctcacccggcctggccacactgtctcactgtgtgtttgagtgtcgcttgacctgctcgacggccagggtggggtgtcactgtctttgctctgccttcagcccagggcctggtatacagtaatttctcagtaaatgtccactggggtcaggcctgggagggacactggaggcttccctgaacaggtgtgtcctccttcgcagccagctcgctgatgtgcttctcctgcttgaaccagaagagcaatctgtactgcctgaagccgaccatctgctccgaccaggacaactactgcgtgactgtgtctgctagtgccggcattggtgagtgccaggctcagaccgtgccttcctcccctggccatctccctagcccgggccggggctcagcagaggccattgctgtctgtctgcagccgtctgtctctcccctgacagcctcatttcccatgcagggaatctcgtgacatttggccacagcctgagcaagacctgttccccggcctgccccatcccagaaggcgtcaatgttggtgtggcttccatgggcatcagctgctgccagagctttctgtgcaatttcagtgcggccgatggcgggctgcgggcaagcgtcaccctgctgggtgccgggctgctgctgagcctgctgccggccctgctgcggtttggcccctgaccgcccagaccctgtcccccgatcccccagctcaggaaggaaagcccagccctttctggatcccacagtgtatgggagcccctgactcctcacgtgcctgatctgtgcccttggtcccaggtcaggcccaccccctgcacctccacctgccccagcccctgcctctgcccaagtgggccagctgccctcacttctggggtggatgatgtgaccttccttgggggactgcggaagggacgagggttccctggagtcttacggtccaacatcagaccaagtcccatggacatgctgacagggtccccagggagaccgtgtcagtagggatgtgtgcctggctgtgtacgtgggtgtgcagtgcacgtgagagcacgtggcggcttctgggggccatgtttggggagggaggtgtgccagcagcctggagagcctcagtccctgtagccccctgccctggcacagctgcatgcacttcaagggcagcctttgggggttggggtttctgccacttccgggtctaggccctgcccaaatccagccagtcctgccccagcccacccccacattggagccctcctgctgctttggtgcctcaaataaatacagatgtcccccagcttcctgctctgagtgtggctgcttgcgggagaggcagagcaccccaggtttggagggtcctggggtcttctgtggtatggncaggggggtggtgggggaggaggagtcatccccctgagccacagccagctgcttgcctgacctcagagggagcccctccccagtgctctgccctttcttctgccccaggttcagcaggtcaagtgagttcctcctccacacagnnnaaggaggatgttggggagcatggaggaaagaaagcgggtgcaagaaggagcacgctcaggctgggcagcacccagggcgtagacttgggaatggagggtgtctgtctggacccgctggtgcagagggcacaaaagctgggctggggcaggacagacgggccggagtgtagtgagtggccctgtgggaggggcagggggctcccacgcagaagctctgcgagcagccctgacccatccgtgcctggactgcag

SEQ ID NO: 5 - DNA, 1593 bp, Homo sapiens
aggatggcatcaggcagggcacgctgcacccgaaaactccggaactgggtggtggagcaagtggagagtgggcagtttcccggagtgtgctgggatgatacagctaagaccatgttccggattccctggaaacatgcaggcaagcaggacttccgggaggaccaggatgctgccttcttcaaggcctgggcaatatttaagggaaagtataaggagggggacacaggaggtccagctgtctggaagactcgcctgcgctgtgcactcaacaagagttctgaatttaaggaggttcctgagaggggccgcatggatgttgctgagccctacaaggtgtatcagttgctgccaccaggaatcgtctctggccagccagggactcagaaagtaccatcaaagcgacagcacagttctgtgtcctctgagaggaaggaggaagaggatgccatgcagaactgcacactcagtccctctgtgctccaggactccctcaataatgaggaggagggggccagtgggggagcagtccattcagacattgggagcagcagcagcagcagcagccctgagccacaggaagttacagacacaactgaggccccctttcaaggggatcagaggtccctggagtttctgcttcctccagagccagactactcactgctgctcaccttcatctacaacgggcgcgtggtgggcgaggcccaggtgcaaagcctggattgccgccttgtggctgagccctcaggctctgagagcagcatggagcaggtgctgttccccaagcctggcccactggagcccacgcagcgcctgctgagccagcttgagaggggcatcctagtggccagcaacccccgaggcctcttcgtgcagcgcctttgccccatccccatctcctggaatgcaccccaggctccacctgggccaggcccgcatctgctgcccagcaacgagtgcgtggagctcttcagaaccgcctacttctgcagagacttggtcaggtactttcagggcctgggccccccaccgaagttccaggtaacactgaatttctgggaagagagccatggctccagccatactccacagaatcttatcacagtgaagatggagcaggcctttgcccgatacttgctggagcagactccagagcagcaggcagccattctgtccctggtgtagagcctgggggacccatcttccacctcacctctttgttcttcctgtctcctttgaagtagactcattcttcacacgattgacctgtcctctttgtgataattctcagtagttgtccgtgataatcgtgtcctgaaaatcctcgcacacactggctggtggagaactcaaggctaattttttatccttttttttttttaattttgagatatacgccctctttcatctgtaagggactaggaaattccaaatggtgtgaacccagggggcctttccctcttccctgacctcccaactctaaagccaagcactttatattttcctcttagatattcactaaggacttaaaataaaattttattgaaagggggaaaaaaaaaaaaaaaaaaaaaaaaaaaaaaaaaaaaaaaa

SEQ ID NO: 6 - DNA, 179713 bp, Homo sapiens
  misc_feature (35963)..(36062): n is a, c, g, or t
  misc_feature (61355)..(61355): n is a, c, g, or t
  misc_feature (95075)..(95174): n is a, c, g, or t
gatcatgttaccagtgaataaaaacacttttacctgttccatcctaattgggatgtcttttatttctttttcttgccttattgcatggtccaagacctccagcaatagaagattctagatagaggccaatgatctgggtctgaaactccactctgccattcactagctgtgtgatcttgggcaagtcaattaatatctctgtgcctcaggttcctcacatgtaaagtggagtgatatttagctcctaaggttgacatgaggatcaaatgggataatgtctatatgtgaatacatacatgactcagtgcttggcacatagtatgtgctcaataaattggaatctttgttaatacaagcatgcctttggcgggtgagaagggtggcagatgctcctaccactcaccccactgggcagcccccagaggacatctgaggcagctgtttgcactcccttccttcagccctttctgatgcccattcttttttttttttttttttttttagacggagtcttgctctgtctcctaggctggagtgcagtggcacgatctcagctcactgcaacctctgcctgctcagttcaagcaattctcctattctcctgcctcagcctctcaagtagctgtgactacaggcatgcaccactatgcccggctaattttttatatttttagtagagatagggtttcaccacattggccaggctggtctcgaactcctgacctcccaaagtgctgggattacagatgtgagccaccgcgctcggccgatgcccactattcttgaatcccttgaactagaggaacggacactctgagtttccagcttccctcctgccttgcaggtggcctgctgggatgtatgtctgtggatgagcagaggaagttatggacagtggcaggttagttgccaggcatggctgtttcttcacaatatgattgcctcaggatagtcagacttcttatgtgtcagctcagggcttcaaaggcaagtgtttcaagagaaccaggagggccgggcgcagtggctcacgcctgtaatctcagcactttgggaggccgaggcgggcggatcatgaggtcaggagattgagaccattctggctaacatggtgaaaccccatctctactaaaaacacaaacaattagccaggcgtggtggcgggtgcctgtagtcccagctactcaggaggctgaggcaggagaatggcatgaatctgggaggtggagcttgcagtgagctgagatcaggccactgcactccagcctgggctacagagtgagactctgtctcaaaaaaaaaaaaaaaaaaaaaaaaaaaaggagaaccaggaggaagtggcatggtctattctgacctagcttttgaagtcacacagaggcatttctgacatatgctgtccatcaaagcagtcagaatcctgtcctgtggcaggagaggatgcacagaacccacttctttttttttttttttttttttttaatacggagttttgctcttcttgcccaggctgcggtgcagtggcacaatctcggctcactgcaacctctgcctcctgggttcgagcaattctcctgcctcagcctcccgagtagctgggattacaggcgcctgccaccacacctggctaattttgtgtttttagtagagacggggttttaccatgttggtgaggctggtctcgagctcccgacctcaagtgatccaccggcctcagcctcccaaagtgctgggattacaggcctgagccaccactcctggccagaccccacttcttgattgaagaagtatgaaaatattcagggacatgcttaatatgaccatagacattgacactgtttctaatactttcagaacaagtgatgctttgatgagcatccttaggctgaaatctgtgtgcacgtctctgcttagaaagtttatgcagttggccaggcgtagtggttcacgcctatagtcccagcactttgggaggcacaggtgggcggatcacttgaggctgggagttcgacaccagcctggccaacatggggaaaccccagctctactgaaaatataaaaattagctgggcgtggtggcaggcgcctataatcccacctacttgggaggctgaggcacaagaatcacttgagcctgggaagtggaagttgcagtgcgccaagatcgcaccattgtactccagcgagactctgtctcaaaaaaaaaaaaaaaaaaaggtttatgcagttatttttaccattttactatttcaatggaacacgaggtgaacccagtaggtagatgaggattgaaccaagagttttgggctagagagtccctgctgcctctgttttcatgtttttcagaatttccttgccagttactttcacctggagttcacctgttccccaccccaactcctcagggtccatggttccctcatttcaaggctcattcaaatgcttcctctgtcaggcaagcttttctgtctgtcctccctctcccttccccatctttgaacatcttagcactttgatgactggggcctcaaatgatccagctctgtggtcccacagcacatagctggtgcccagcaaatgcctgctgaaaaagtttattcatcaattcaacagagatttactgagagatttgttgttgttgttgttgtttgtttgtttgttttaatggagtctcactctgtcaaccaggcttgagtggaatggcacaatctcggctcactgcaacctccacctcccaggttcaagcaattctcctgtctcagccccttgagtagctgagattacaggcacctgccaccatgcccggctaatttttgtatttttagtagagatagtgtttcaccatgttggccaggctggtcttgaactcctgacctcaagtgatccacccacccagcctcctacagagctgggattacagacgtgagccactgcgcccagcagagagctgtttcaagggtcctgaaatctgacatggtatgccaacatggaaatctttgttctagaaacaagaggcagggtgcgccatgcagagccgcacaggaaagcaccgggttggtcaggaggcagagggaaggaggggtaaacatgagcaagagcctttattgtggtttccatgggaaggaatgggtgaggcaaggtaagcagccttaggattggttggtttgaataactgcagtaggtgctggggtttatataagggctttccctagctgtctggtgtctggccttgggatgatcagggcagttggatactggccctgagtaagagagcctaataaaggaggtgtttgtgggtgtgggctctggattgggtggcatgcatttgcaagggacctcctgggtgagttcttcactatctccaggaaccagttaaccctggttggggcagtccctctgggaagagcaagtccccaagatctcaaagcatctgagtacagaaaagcaaaggctctgggcacagtggctcatacctgtaatcccagcactttgggaggccgaggcgggtggatcaccaggttaggagttcgagaacagcctggccaacatggtgaaaccccgtctctactaaaaatacagaaattagccaggcgtggtggcaggtgcctaaaatcccagctactcaggaggctgcagtaggttcaagaggagaatcgcttgagcccaggaggcagaggttgcagtgagcagagaccacactattgcactctagcctgggcgacagagcaggattccgtctcaaaaaaaaaaaaaaaaaaaaaaaaaaagagcaaatgcatgcttaatacaagggcctactatatatcaagcatatatacgaaatgggcagtgaaccaaatggacagtctgggtattggtggggctcatatcctgtgggaagacaggcgatgagcagacaagcaaatctgtattttgtaaatatattgtatttttttcaacaaatattttatggctgccctgtgtgccaggcctggatctaagcattgatatatgatgaacagaatagataaagtccctgttttcagcaatgcatgttctagtggggggagactgcaatcaatgaacaaaaaaaaaaaaaaaaagaaagaaaattgaagcccaggcatggtggctcacacctgtaatcccagcactgtgggaggccaaggtgggcagatcacttcaggtcaggagattgaaacaagcctggccaacatggtgaaaccccgtatttcctaaaaatacaaaaattagctgggcgtggtgatgggttcctgtaatcccagctactccggaggctgaggcaggagaatctctttaacccaggaggcagaggttgcagtgagctgagatcgcgccattgcactccagcctgggtgacaagaccaagtctctctctcaaaaaagaaagaaaagaaaagaaaaagaaaaatcagtgacaagaagtaaaacaggatcaagggattaaaaaaaaggactggaaagttattccagataaggtgatcagggaagtcttctctgaggaggtgatgtttgagcaagccatgagtgaggagaaggagccagccacacaaaagcctgggagaagagaattcatgcagaaagagaccagagtgaagggccctggagtgatgagaagcttggtgctgtggaaccgaggggaagccagctagtcttgaggcaggagaatagggtctggaggcagggaacataaggctgattcacactgactttctagaactaaatcaaaaggaaaaccccaactttccacgtccaagtaaccaaaggaccagaggctactccctttgcaatcccagcttttctgtgtgcagatgaaaaactgaaagtacctctgattgctcccttcccactaccagtcaggctggtaggtggccaagtcttcatttgcatgggagtataactttgtaacttcacttcagcctctgattgataactttccacagccaatcagacattggcgtagggtgtaacttttaacttcagcctctgattggccactttccacaaccaatcagactgatcacgggccactccttcatttacacagggcgtacaccaaataaccaatgggaaacctttagagggtatttaaaccccagaaacttctgtaaggagcctgttgagtttctttgcttgagctgttcttgccctgtagagtgtactttcgttttcaataaatctctgcttttgttgctttattctttccttgttttgtctgtatgttttgtccaagacgccgagaagctgggcaccctccaccgttaacagtccggctgcagcatagtgagtaacgcagtgggttaggacgagcgtgaggtcagagacaggcaggagtcaagaagtgctggaagcagagaagtgatttaatctgtttttaaagctctctctggctgctgtgcggagattggatgataggaaggacaaaagtagaattaggaagacaagctaggaggttatctccctggtaagagatgccgttgatcagcctggggcagtggctgcggagatgcacagatgtgtggcatcagtgaatcttagaccttttccgccattgaaattacatagggagttaaaacacgcacagacttctggaccttacctttgcagagccttgtgaaaggcaaataaatcttggggccccaaaatcactaagctaaagggaaaagtaagtcaagctgggaactgcttagggcaaacctgcctcccgttctattcaaagtcacccctctgctcactgagataaatgcatacctgattgcctcctttggagacgctaatcagaaactaaaaatacaaaaaatgcaaccatttgtttcttttttctttctttttttttttttttttttttgagacggagtctcactctgtcgcccaggctggagtacagcggtgcgatctcggctcactgcaaactccgcgtcccgggttgaagccattctcctgcctcagcctcccgagtaactgggactacaggcaccagccaccatacccggctaatttttttttttttttttttttgtatttttagtagagacggggtttcaccgtgttagccagggtagtctcgatctcctgacctcgtgatccgcccacctcggcctcccaaagtgctgggattacaggcgtgagccaccgcgcctggcctcaaccatttgtttcttatctacctatcaccaggaagccccttcccagcttcgagttgtccagcctttccagaccgaaccaatattcatctcacatatgttgattgatgcctcatgtctccccaaaatgtataaaaccaaactgcgctccgaccaccttgggcacaggttgtcaggacctcctgagcttgtgccacaggcacatcctcaatcttggtgaaataaactttctaaattaactgagacctgtctcagatattcggggtttacagactcaatgcctaaggaatctatactttttacaagccccctgggatgtgctgcttcgtctccgggtacccacttgtctactggtcgtaaaggggtaagtgtggccgggcttggtggctcatgcctgtaatcccagcactttgggaggccaaggtgggcggatcacttgagtttaggagttcgagatcaggttgggcaacacggtgaaaccctgtcttcacaagacaaatacaaaaaattagccgagcctggtggcatgtgcctgtagtccaagctattcaagaggctgaggtggtaggattacctgagcccaggaggacgaggctgcagtaagccataatcgtgtcattgtactccagcctgggtgacaaagactctgtctcgaaaaaaataaaaataaaaaaaggtgcgtgtgatgatgcagaaagaggagcactggggatgggagagggggagtccctgtcgttttggattctagtcccagttacgggtctgtttggggggctcggtggccccaagtgatcatcagggatagcaatgcctatctcgaagatgggctgaaagtgaggaatacataacatagtatttgtaaagcactcagcaaaggaccagccgaagcactcgggctatttctggtaaagggtgcaggctctggggtaaatcgcgtgcagttggaacacacatcggctttgcagccatctgctaatgtgaattccattccttttggggcctcgatttcctcctccataaactggtatccacaatgccaaccttgtgaacgctgtgagaatgcgcggggtaaaggcgacgtctctccctcccgggaagaacttggatggtgtcaggcctacactctcgctccgcctagggccgctcgctgggcctggctccccggctgccgggctacgcgagctcagaggacaccatcgccctcttatggccgcggcaggactggaccgaggggctgggctctagtgccttcctccaggcacggcagagggcgagggtctggcagcccgcttacccagggcctcggggcactagcattcatgtcatcgactgcctggcagggctggctttcttaagtgtggtcgtgagacttgcttaagtggaagaaatgctgtcgctttggagatttataaaacaattggctcgatggatctttcttcaggaggcggacttggtttaccggctttactgaccacagctgatgccaatgatttcatttaatcgtctttagagtccctgtgcatggggagttaccatccccaattagtttcttgtgaatgcagggcaaggagagggagagggtagtgggggacggggagaaggggcgaggggtaccctcctattaaaacggagccgcagaaaaacccacagagacatccgtctgttccccgctgagtccttagaacagcgcctggcacacagagagcgctcaactcgctgtgtaactaaatgcaagccaagatcttcgcattgtgtgtgctcttcccttccctaccaaatatacctggcttgcaaggtttgacctgttttcttagacgatttttaacttgtttccaaaagaaatattggagtaaattagcttgttcaaaggagtccttatgaaaggacagaaccaagtgagaagtatctggagcccggtttggggttatagatgatgatgttgagccagcacccacggggcggccgcaatgtagaatcctggcgctactgggaaccgtgtggaaaggggctcttctttctgttcaaatagtgttttctgtagatcccatctctccatcctcctgagctctctcttacaaaatatcggatttcagcagcttagaattggacagaaactcagaggtccgtttctcaattatctctaaccctggtaaacaataaatgggatgatgagtacaagacagttttggtaaaaagtcacacgccacacaacgtgagattttattattccacgggtgcttccttgccaatagtagacatggcagctcggctcccttcccttcgggttcgccttattgttgccaattgtaaacatggcctctaggccgtgagttctcattggcagctgctctgagtccccgcccttccccgcccctccgaacgcggcctggagttgtggagtcggatatcgcagctcccgactgagctgcgcctgcgcaactcattggcgccaagatggcgatggagatgaggcttccagtggctcgcaagcctcttagcgagagactgggccgcgacactaagaaacatctagtggtgccgggggatacaatcactacggacacaggattcatgcggtacgtggggacttgggggagtcgaggcttcagagagcggcttcagggctctctgcacgtggtccaggcctcgtatccctgtgtgtgtaactccccgcgggacccagggcacttcgtctgagcatcctacacacctcgcttccgagcctcgtgcttcttgctccctgcatcttgtgtgtccccgtctgcatttgtctcagctccctgaaaccctccactcctgacctccggtggctgtgacttttgggtcttctgcctgaagtccaaatctttgatccttccttgtgggagacctggaaagctggggagggttaggtgcaggctcttttccagttttcagctctctgaggggacggtgggcgttcttggctgcctcctcttcagtttagaatccgtaattgttcgatcttagggcaaacagttacattgtgctgcatgcacccatttatacacattttgaatctaaggggtgtagtgcagtgtattgtggttaagagggaaggctcttgagtcagacagttggggttccggtcctgctaccatcacatcttattagcggcattgcctctccacggtcagtttcctcatctgtaagatagtgataataacagtatgatacggtaatgaggattaaatgagacaattatgtaagaaaagaagtaaaaccagccattatatcatcatagataacactagtgtttcaacctttattattattatttttttacttgtatatgtacaaggggcacagcattcatagcattgccctttaacctgttagtttaaggttagtggataccaggaaatttttttttcttttttgagacggagtctgtcttagatcagtcgtgcgatctcggctcactgcaacctctgcctcctgggttcaagtgattctcctgcctcagcctcctgagtagctgggattacaggtgcacgccaccatgcccagctaatttttggttttttttttttttagtagagacagggtttcactgtgttggccaggctggtctcgatcccctgacctcaagtgtgatctgcccgcctcggcctcccaaagtgctgggattacaggcatgagccaccatgcctggcccctaggaaatcttaagattcattctttcattaatgctttcaacatatattttgtgcagttgggttattatggcagagtgaaaaatctctgtcctggtggagttctaacagggagagatagataataagcgcaatgaataagttattcagaatgttaggcaataatgcaatagggaaaaaagtggagcagggtcaatggtatgtggggggaatggtggcaacagggtgggctgtgttttcaatggcacagtcaaggtaggcctgctgcagaaagtgacacctgagcagacctgagtgagaggagtgatgtccaagtagctgtctggagaaggagcactgaaggcagagggagcagccagcacagaagccacgctttgcagggggagcctgttagctttgaggaacacgttgttcttgaagggagagaagtcatttcgagttaccctcgtatcctttctttgtatcttcgccttgcatcaggggccatggaacgtatatgggagaagagaagctcattgcatctgttgctggctctgtggagagagtaaacaagttgatctgtgtgaaagctttgaaaaccaggtgagaacaaaaggtgtgtattccctttcttgcagcatcaggttgtacaaccaggcttttcctgccccctccttatcccccaccccacccctgcctgccctgtcatgctgtaagtctgaggttttgaccatgactgtaggtggggtggtgcagatcagtgcaggcttcagaggtttccccatgttatgtcaccactccaagccttggttacctcctctgcaaagtgagtataatagcatggcctacttcataggattttctctttttttttttttttttttttccgagatggagtcttactctgttgccgaggctggagtgcagtggcgtgatctcggctcactacaaccttcgcctcccgggttcaaacaattctccttcttcagcctcccgagtagctgggattacaggcgccctccaccacgcctggctaatttttttcgatttttagtagagacagggtttcaccatgttggccaggctggtctcgaactgctgacctctgatgatttccccccacttggcctcccaaagtgctgggattacaggcgtgagccactgtgcctggcctaggattttctttagaattcagtgagatggtgcctgtaaagtatttagcacagagcctgatacctagaagcattcaatgaaggttagccccagaaagcaagccagtggggttggaacagagtgagtgagggggagagaaggggcagatgtaagcagagagctgaggtgggcgggcgtgggcctgccttgtagccagagtaagcattttggcttctactttgtgtaatctgggaagcactggaaggggtggagcagaggagggacttgatctggacttaagctcactctggctgctgatgggagattgaagggggatagggcaagcttagggaggtggattagggaccatactcatgatctgaagtgatggtggcttcaactaaggtgggagcagtggaaggtggaggagtgattggaatctacacagattttattttccgagtgtttttttaaaatcatgaaaagctgttgggttttgtattctttgggctttactgtgcataggaccccgtcaactgtgaatagaaataagtttacttcttcctttccaatttggatgccttttatttcctgcatatgttttaagggtagagccaacaggttttgctactggacttgtcctggagcgtgagagagagagaggaatcaaggaactctccgaggtttttggcctgagcaactgaggggatggagtcaccgttgactgagatggggacaactcatcccctatctcggtttgctatggaggactggagggggctgcgggaaagcttagttttgtgcttgatacatttgaaaatgcctgttagtcatctagatggcagagttgggtagctagcagttgagtaggatttggaattcaggagagtggcacagtcacagcacagagtggtgttttaaaggtattagattgagtggccgaaaagtgaagaggtctaaggacttagcctcagcactgagtacgtctcattagaatcgcgggtaaggaactagcaaaggggcttgagaggagcaggcagtgagtaagtggaggagacgtgagcagacttgtgtggttggagtcctggctcagatttcctttctcttcctttggctggtgcagaactcatccatgtgccacaggaaaatagtccgtgtttttcattgtcgtgtaatcgaacaaaatagggtttttgggctaaatgaactacttggaatggtgatatgtctaaggatagttaatggagactttatacgtggaggaatgtttgaagttagcagtttctgaaagtaagtccagacaatatagttacatgaatttgctgaatgtggcgcctgttccaggctttcaccctgttgaaccgacatctcaaatggtgtgtggtcttgtcagaaagtctgctcacagatggatgaaccccttgtgttttgtctttcagatacattggtgaagtaggagacatcgtagtgggacgaatcacagaggtaacgtcgatatcagattggtgtttacaaagtcgaggcaggctggcgatttcattcatgggacagtcattccacttgtagttacatgaaaaaggcattcattgcatttggccgttgtgtggcttctgatgtaaatatgtggcttgttcgatttcagattactggttcatgtttttttttttttgagatggagtctcgctctgtcgcccaggctggagtgcagtggcatgatcttggctcactgcaacctccacctcccaggttcaagcgattctcctgcctcagcctcccaagtagctgggattacaggcacccgccaccacgcccagctaatttttgtatttttagtagagatggggtttcattatattggtcaggctggtctcaaactcctgacctcaagtgatccaccagcttcggcctcccaaagtgctgggattacaggcgtgagccaccacatctggccttactggttatttatgatatgacacatgaacatggagcatgtgtccaggtgtggaacttggcttataggttcaacagaagaggtggaaggtggagaccaactccaggctggattcggtcttgctgctctcgtccatgaaccttcctggaggagagctggtaagggctacagctggggccatggactagggcccagtgggctggggggagccgtgggaccctttgttccaccagaggactttgatttacactgaggttgcccctttgactcctgtttgtctgctgtgaagtttgctgcctagatgtgtatgtagacttttcaccctgtccaggtctcccgaaagagggagcagttggcatatggtaggatcagaaacatccatggggtgggatcccaacagagagttggggagagaagcccttagatgctggttgttaacagttttccttttggatataacagccttgcatagtgaagatgttccttgaaaagttgtctttacattaggtttttgtgaattgaaaggcatttcattcaaccatgtgtggaatgtggttgctggcattccagacaaccacagtaactaagccacagccttttgtaaaatgccatggttcaccttgatcttcagtccagcgtgtatttacagagaggcttactgtgccaagctctgtgccgagtgccaagcacgattgagttccccagcaggggatataagataactgacctagtccctggcagtagaagaataaataagctgtggttatacaaaaggaaatttcagtgagagaagcttgtaggaaagacaggcattggagttgatcctggaaggatggagagactttgaatgactagttcagggaatctgagataaagggaaatgtatgagcagagatatatccaagcaggagttagtctggtcctgctggaccacagagggctgtcatggaagatgactatggaaatgttggctaggtgagattgggaggggtctgaatgttcctcagagaagggagggaaagaggaagaggagctgtggaaaagtcttttgagatggaaagtcgtgattatcactgattcccctcaagtggcttgggttacctactcttgctatagttctcagtgcttgaatattgtggttggcctcaaacatctcaaaaggaagtgaaagagaagtgatggagacctttctgaggatctggcttaagtaatgtcatttctttgtgtatttcagaggagaagatctgcagaagatgagcttgcaatgagaggtttcttacaggaaggggaccttatcagtgtatcctgcgctttgcactccagcctcttgatgcttttctgtgggactgggaaatgggccttccattgtatgtctctgacggaagaaccatgtcatccttgcagggatccgagtcttagaccaagtgtcgggctctgctgcatcctttctcagtctccttaattcaggctgactccccagctcttgttgggacctgctgctaagtcatttctttgggtcttgtaacttacggtggcctgtgctttagactaggcttttgttaatggtgttaacttttagcgcagggagtggagaaggtgttgttcacgtcaagatattaatgacaggccgagtgtggtgactcatgcctgtaatcccagcgctttggaaggccaaggagggaggactgcttgagcctaagagttcaagaccagcctgggcaacatagcaagacccccctctctacaaaaaaattaaaaaagaattagccgggcgtggtggcacatgcctgtagtcctagctactcaggaggctggggccagagggttgcttgagcccaggagctcaaggctacagtaagctatgatcacaccactgcattccagcttgggtgacagaacaagactctgtctctattttatgttattttttaaatttttctttttttttaatgacggagtcttgctctgttgcccagactggagtgcagtggcgcgatctcggctcactgcaacgtccgcctcttggattcaagcaattctgccttagcctcccaaatagctaggattaccggcgtgcgtcatgcctggctaatttttgtatttttagtagagacaggtttcaccatattggccaggctggtctcaaactcctgacctcaggtgatctgcccacctcggcctcccaaagtgctgggattacgggcatgagccaccatgcctggcctctgtctttattttatttatttatttatttatttatttatttatttatttatttttttgagacggagtttcactcttgttgcccaggctggagtgcaatggtgggatctcggctcactgcaacctctgcctcccgggttcaagcgattctcctgcctcagcctcctgagtagctgggattacaggcatgcgccactatgcccgactaattttgtacttttagtagagacggggtttctccatgttggtcaggctggtctagaactcctgacctcaggtgatcgacctgcctcagcctcccaaagtgctgggattacaggtgtgagccaccgcacctggccttctgtctgtatttttaaaaaaaagatattcatgacaaccaaggggagaggtaaggtcacagtgatgtgctctgggtcaaagattgttgagcctggaccattggagaggggaggaaaagatggaggtgtggggtcaaggggagaggctgcagaggacaggacagtgtgtggccaaggctgctgtttgttccttcatcaccctggccaggctgaggtccaggcagtgttctctgacggagctgtctctttgcacacgaggagcctgaaatatggaaaagtaagtcgggctcttgatgttcctgtttgctgactgagactacaaggctatttttgaatccccatagctctctggaattctggcctaaagaaccccagtagctaagcattaatagaggctggcatcccacaaactgatcgtgttccttaaacgtaacatcaggacggtcagggttcacagggtcatgggtcagtagccttgtaaagaacaagttttatcctttttctccaaggagactgactttcaccagaagagcccctccaactgtgggctgggaggtgcagctgtctctcttcctccagggggcgctgcagctcagcactggggctgaggctgtcctgggaacaaaggcaggctgggtctggttaaacagcccttagacaaacgtccaatcagtccagtggatgttattgctggcaaagcttgctctgtcatctgagcctctaaatggaatttcactgcttttcttgtacgaggttgcattattgaagctatttactattttaaggagagcatacttcctaaaacaaattaggatttactagtctcttagctttatctgggtgaacgtttttattttctgagtggaacaaaaacctcttcccttaatggagtggctgcagacagccacgttgatgtacatggagtaggcagaggactgctgcagtatgctgactttcacaaccctgggtcctgcggactcttccttggcaggacgtggacttgagctgtcctgccaggaccagacatggatttgcacccagctccacccatctccttacctacccagaggcacacatctcacaggcaagatgagtgtttggggttcaggtatgagctagggtcatggaacaacgcagtgctcctgggccagcaggaggctccagctcacttcctcattggcttcagcttctctaatgtctggcacatgagttctggcttagagtgcaaggaagactgcaaagggaaatgacagagaagagtattgaaggtcaccttctgctgggatgtatgaatagcctctgagtcccaaagcgttctctgcaaaaatgtgtactatgtgtatgcatgtaggcgacagcaattataaacaggaaggacaccaatttgaatatacttaggatgtatattctgtagtctccttttcattcatcccgccaatcttgcagtgacctagcttcgtgatatatttctttagctaggtcagggggttttggtccaggtttccccctccctggtgaaacggcagaagacccactttcatgatttgccatgtggtgcctcagtgattctcggtaacaacggcttcatctggatttacccaacacctgagcacaaagaagaggaagcagggggcttcattgcaaacctggaggtgagcaaacactgtggccattttcagtgggatggagggggctcagtctttgctgtgtttttgtggccagtgaagttggttgtttttagctatgttactggtgtaggctgagtcactttgactttccatcacggtatgttcatgaagcccatattatcttctcttctaaggagatgaattcagtgaatggtttggtgtttgttggtggaggtggcaaagttgcagggtaatagccgaagagccagtgaagaagccattctttttctgtttttttgtttgtttgtttgttttgttttgttttgttttgagacggagtcttgctctgtcgcccaggctggagtgcagtggtgccatctcggctcactgcaagctccacctcctgggttcaagtgattctcctgcctcagcctcctgagtagctgggattacaggtgtgccccaccatgctctgctaatttatctatttttagtagagatggggtttcaccatgttggtcaggctggtcttgaattcctgaccttgtgatccacccacctcggcctcccaaagtgctgggattacagacatgagacactgcaccctgccccattccttttaatctcccttggaattagctgtttggttgatttggagttccagggtgatactgtctgagtcataaatgatttatttgtgaatttctgtggctggtcacgtattttggtcctgtttgtatttcccttcccctctctgtgtctccttatagcctgtctctcttgctgatcgagaggtgatatcccggcttcggaactgcatcatctcgctggtaactcagaggatgatgctgtatgataccagcatcctgtactgctatgaagcatcccttccacatcaggtactctccccagggcctctcccttcttcactgatctgtgagctgctctgttgtttgttcagagacaatatgcacatctccccaatactttcccaacatccgtcagtatgaactggcctgaaacagccttaatgagtgtctggtagatctttccctaagaaacttgcaatattctcaatgcctagtgtcagtctaaggattttggggcaggaggtgtcaggtgggactagtttatgagagcaacctctggactacatcttacctctcccaaatttcagccagcttttggatgaatgtcagaataatatctttgttcttgtcgactatatcccagagcatcttgctgatttattaggctgcttctagcagatcatatcttgtaacgcttagtctctgagacatgaaaggaatacagaaagtttatgttaacggcttgatttatgtttggattggcttggtggtctgtttatggttggtttcttttctgaacaaatgccttttccctttttcagatcaaagacatcttaaagccagaaataatggaggagattgtgatggaaacacgccagaggcttttggaacaggagggataaggaggtgctccagaagcacgggactgtggaccttgcaggagtgaagactgtgatgtgtggtccccatatgtggctcagcaaagactcgagagatcatccctttgtctgcattgacggccctgtgacggcctccagcccacaggcctgctttctcctgtcctaacaccaagcctgggtggcagatgaacagtgcttccttgggttgccagctgagtcccggtattagggaatagtttcagctctttcaaagtgcacagtgttacagtcgaatgggctcccatcctggaataatatggagaatcctttgtcttccactcactgtcattcacaaggcacagtgccccatgaaattgccccaatagaaaacatggcatccctgacctccaaatggtctgttttggcctccattcctatatcctttaaatgactgagaatgcagctggtaaagttggaagaataaagttaaccaagcaggccaggcacggtggctcacgcctataatcccagcacttagggaggccaaggcgggcagatcacctgaggtcaatagttcgagaccagcctggccaacaaggtgaaaccccatctctactaaaaatacaaaaaattagccaggtgtggtggtgtgcacctgtagtcccagctatttgggaggctgaggtgggagaatcacttgaacctgggaggcggaggttgcagtgagctgaaatcgcgtaccacactccagcctgggtgacagagcgagactgtgtttcaaagaaaaaaaaaaacaagcagccttttgcttggttggaatctgattttctgttgcgtgttccttgtagccatagatgtgattatgtccacaccgggctgccttaatctgtcctgcttggagagtgacttgtaagatgctgaattattcatgataatacagtgaatgttctgggtccatgtactcagataaacatgaagaaaataagcaaagaaaaatggagactgggaaagcaaagctgttttcatcctataattgaagtagtgtggagcattaacttgtggatgattcagagttaaaagataaaaagacgccagagttctcgctgaagaatgtgagaattcctgtgcattgttttttctgatgactatctaaaaatggtgccctgatgtaggtttgggggaacattcttaaaaacaagggtgctatgtgcctgtaatccagcactttgggaagctgagtgggcagatcacctgaggtcaggagttcaagaccagcccggccaatacagtgaaacctcgtctttaccaaaaatacaaaaattagccgggtgtggtggcacaagcctgtatgtagtcagctactcaggaggctgaggcatgagaatcgcttgaattcgggaggcggagttgcagtgagctgagatcgcaccattgcacttcagcctaggtgacacagtgagactgtctcgaaagaaaaaaaggaaaagaaaaggcggccggacgtggtggctcatgcctgtaatcccagcactttgggaggctgaggtgggtggatcacaaggtcagatcgagaccatcctggctaacatggtgaaaccccgtctccactaaaaatacagaaaaaacaaaccatagcctggcatggtggctggcacctgtagtctctactacttgggaggctgaggcaggaaaatgacgtgaacccgggaggtggagcttgcagtgagctgagatcgtgccactgcattccagcctgggtgacagagtgagactgtctcaaaaaaaaaaaaaaaaagggacactatatgcaagcgctgtcttcacatatgtggcaaacttgtttgtttgtttttgagacagagtgtcgctgtgtcgctaggctggagtgcagtggctcgatctcggctcactgcaacctccacctcctgggttcaagcaattctgcctcagcctcccaagtagctgggactataggcatgcgccaacacgcccagctaatttttgtgtttttagtggagatcgtttcaccatgttgaccaggctggtctcgatctcttgaccttgtgatccacccgcctcggcctcccaaagtgtttggattacaggtatgaaccactgcacccagccatattttttgatatttatagacgtcttttttttttttgtttttttgagacggagtcttgctctgtcaccaggttggagtgcagtggcgcgatctcggctcactgcaacctccgcctcctgggtttaagcgattctcctgcctaagcctcccgagtagctgggattacaggcacgtgccaccacgcccaactaatttttgtatttttagtagaggtggcattctaccatgttggccaggatggttttgatttcctgaccttgtgatccccccgcctcagcctgccaaagtgctgggattacaggcgtgagccactgagcccagctatagatgtcttaacatcattgttttctgttcttttgttccgggtaataataaggagctgaggacagctgaggaagggcttggctgacaaaatgccttccgacagagccctaactactccacgtaaacctaggacagtctcaatggtagtaactttgaacactgcatttgataactttcaaatacaacttggctctttttcattaaatggtatgcttctctataacaacacaataaacaacttcttacctcactttctttttttgagacagggtctcactctgtcacccaggctggagtggggtggcatggatcacagatcactggagcctctacctcccaggctcaagtgaacctatcttagcctcccgagtagctgggtccacaggcatgtgacgtaccaccatgcctggcttttttttttttttttttttttgagacagggtcttgctctgtcacctaggctggactgcagtggcacaatcacgtctcaacctcctggtctcaaccagtttccaacttcagccttctgagtagctgggactacaggtgctgagccaccacatccagctaattgtttttgttttttgtttttcggcagagatgaagtctcactatgttgcccaggctggtcttgaactcctgacctcaagcaaccctcctgctcaagccatcttcccaccttagcctcccagagtgttgagattacaggcatgagccaccacacgctgcctattttttttatttttacgaatttttttgttgttgcccaggctcaagcgatccacccacctttgcctcccaaagtgctgggattatgtgtgtgagccacagctcctggcctctttttttgtttttcctatcccaagttgtattactagttttggggagtttgcagacaattgaatattctataggctgtgttgcagctttagatggatcgacctgtcatgtttttgaggttatccaggctgtatatctctggagagaagggaatggcaaagagtgggagtctgagtcaagtttggttttgtttttttaagagacaaggtctctgtaatccaggctgcagtacactggcatgaccatggctcactatagacttgggctcagccaatcttcctgcctcagcctcctgagtagctgggtttggttttccccagggccatatgtcagcttatttaccctcctcacttggtgtctcccagcctgccagcccatgctgttcatccagtatctgctgaatggtgattacctattaagtggaactaacacaaaattgcttatctaaaagcaattattggtgattatttccttgcagtggcccactagagggcgccattgttaagtgtaattccagtaggtgttttgtgttttttttttttaatggaataaactgaaatctttacatggtactgaatccctttagcaacttggggggttgctttaactgaatcacttttaatgaagatatatgaacttgaagggatttattcaatatatgacaatattactcaatattacttttttttttttttttttttgagacaaagtctcgccctatcccccaggctggagtacagtgacgggatgtcagctcactgcaacctccgcctcccgggttcacgtgatactcttgcctcagcttcctgcatagctgggactacaggcacccaccaccacgcccagctaatttttttgtttgtttgtttgtttgttttcctgagacggagtctcactgtcacccaggctggagtgcagtggcgtaatcttggctcactgcaacctccacctcccgggttcaagcgattctcctgcctcagcctcttgagtagctggaactacaggcacgtgccaccatgcccagctaattttgtgtatgtttagtagagacgaggtttcactgtgttaaccaggatggtctctatcttctgacctcgtgatctgcccgcctcagcctcccaaagtgctgggattacaggaatgagccactgcgcccagctgaatttttatatttttagtagagatggggtttcgccatgttggtcagcctgctcttgaactcttgaactcaggtgatctgcctgccttggcctcctgaagtgttgggattacaggtgtgagccaccacacccagccaagcaatatttatttccgattgtcaggcatttgccaggctttggattctagtttttaagcccttaacagtatcattcagggcctatgttctcaggacctcttgagactgtgcctcggtttttaaaaaaagtatcattctacagtattatacaggcatttttaaagtacagtgcattggccgggtgcggtggctcacacctgtaatcccagcactgtgggaggctgaggcgggcggatcacctgaggtcgggagtttgagatcagcctggctaacatggggaaaccccatctctactaaagatacaaaatgagctgggcgtggtggtgggtgcctgtaatccctcaggaggctgaggcaggtgaatcgcttgaacccgggaggtggaggttgcaatgatccgggatcgtgccactgcactccagccggggtgacagagtgagactctgtctccaaaaaaaaaaaaaaaaaaaaaatacagtgcatctctagaaaaaaatactagagtctgggcattgggcatggggctcacctaaaacaagaaaatggcaaagtggaaaactagggataaggctttagatcaggtgcagctgacctctgctgtgactcccaggaagcatagtcccaatctttgtggaaaaccaaatgagatctagtttgatcctcatgaaccctgtctctacaaaacaacaacaacaaaaaaacgtaggtgtggtggcatgtccctgtagtcccagctacttgggaggctgaggccagaggatcaccagaacccagaaagtcgaggctgcagtgagctgagattgtgccagtgcactccagcctggccaacagagtaaggccctgtcttcaaacaaacaaatcaaattaaacaaaaaacccaaaacccttgtaaagtaagctatgacctccatttacgggtgaagaaatgaactcagaattaaagggacttgatgaagcccctttgaattgtgaatcaatgtagatttaagctctagggaggtgtcataatgcagtcctttagaggatggactggactgactgaaagtttatggacccagaaatttaattccagcattgaggctgatcttttgtttggattgttattttgcttattgcccatccttccatgtaggttccatgaggacaagggtgggtttcttcccccaccactgtgtctcagcacctaaagcagtgcttcacatacagatgttcaataaatgcttcttaagtgaattgttatttattttttgagacatggtctctgtctcccagactggagggcagtggcgcaatctcagctcactgcatcctctgcctcccagactcaagcaattctcctgcctcagcctcccaagtagctgggattacaggcatatgccaccacgcccggctaatttctgtatttttagtagtgaggggtttcaccatgttggccaggctggtctcaaaactcgtgacctcaagtgatccacctgcctcggcctcccaaagtcctgggattacaagtgtgagccaccgcacccggccatgaattgttagtttaaaaaaatgtgtattaggggttctgatttgactgctcaattttaagctaaactagagaataaagcatgtgcgcggtggctcacacctgtaatgccagcactttgggaggctgaggtgggtggatcacgaagtcaggagatcgagaccatcctggctaacacggtgaaaccctgtctctactaaacatgcaaaaaaaattagccaggtatggtggcgggctcctgtagtcccagctactccagaggctgaggcaggagaatggcgtgaacccgggaggcggagcttgcagtgagctgagattgcaccactgcactccagcctgggcgactgagcgagactccgtctcaaaaaaaaaaaaaagaatctggagaaaatgactaaagtatgaatgggaataaaaagaaagcacaatctccagaaggaataattaggatataatcaggataagataatgggtaaataggccaagtacaatggctcatgcctgtaataccaacactttgggaggccaagagggcggatcacctgaggtcgggagtttgagaccagcctggccaacatggtgaaaccccatctctacaaaaatacagaaattagccaggtgtgtggcatgtgcctgtaatcccagctacttgggaggcaggagaatcgcttcagcctgggtggtggaggttgcaatgagcagagatcgtgtcactgcactccagcctgggcaacagagcaagactgcctcaaaataaataagtaaataataaataatgggtaaataaagcagaacaagggcattcacagttgaagaatgacactacagatcagaactaagattgtcagccagataattttgtgagagaacaaagctaaaccaaatcacatctgaatttataaattccagttctaaatctacgcacaatttttcatgttttccattccgtaccttccaagtaactaattcctcttgaaaccagtatcaaaaataagtgtcatctttcaatgcgacagaaatatttctaaaatacttaatataatagctgaatgtacaacactcatcgtgcagctgttcctccgatatcagtagcaacttgtgaaaaatcagtggtctcagatcaacaggtttttgatactgaatggtacagtgggaaccatgggttttggagcaaggtcagtctgggatgaaattgtgactctgtcacacattggccaagtgaccttgggtaggtaagtcacatctctgtttccccatctgtattatggggaatagtattacatgcctcactgggctatagtgaggattacatgagataatgcagtttatggaaagtgtaaacagtgctcggtgtaaagtaggagctgtgataagtggatccctccttagaaatgggatctcgggccaggagcagtggctcacgcctgtaatcccaccactttgggaggccaaggtgggtggatcgcttgaggtcaggagttcgagaccagcctggccaacatggtgaaaccctgtctctactaaaaatacaaaaattaggcacgtgtgatggtgtatgcctgtaatcccagctactcgggaggctgaggcaggagaatcgcttgaatccgggaggtgaaggttgcagtgagctgaaatcctgttactgcatcgcagcctgggcgacaagagcaaaactccatctgaaaaaaaaaaaaaggaaagaaagaaggaaagagaaggaaagaaagaaggaaagagaaaggaaggaaagaaagaaagaggaaaaaaggaaaggaaaaggaaaaagaaaagaaagaaaaggaaggaaagggagaaatgggatgcctgtcaggtgcagcgctctggggaggcgtggagagcctataatagggaccaaggtgctttttagtcgcagaacatggattatttgttaggtgtggctttggcacatctaggtcattggttctgccgacttgctaaacccaaccatctgggcattttctcggctaatatagaggatgttttcatgtgaacacgtgtccacctgtgaaatgtttataatgttaaaggttcgttctggggcaaacatctgatagcgcctggcaaacccaacaaatgccttttctgtaatgagtaagcctcctaatgcccaaagaaacagttgaattcgttagcaacatgtcggatgttttccctatgtctgtatatttcttcgctagtttttttttttttttctttttgagacggagtttcgctcttgttgcccaggctagagtgcaatggtgccatctcgcctcaccgcaacctctacctcccgggttcaagcgagtctcctgcctcaacgtcctgagtagctgggattacaggcatgtgccaccacgcttggctaattttgtatttttagtagagacggggtttctccatgttggtcaggctggtctcgaactcccgacctcaggtgatccgcccgtctcggcctcccaaagtgctgggattaccggcgtgagccaccgcgcccggcccgctagttctaatatttatgctttttggagggtgaagggcttgaaaggcatcaaaaaccttggtttctaggagcgagccaaattttctcccttagagactgaaggaggttatccgactccgcttccaggaaaatccaatccgcaatttttccctcgctttggctcttccaggtctcactactcgcgccggggagacgcggtccggcctacgctaggccggcaagaatctaccaggtcccaggagggcggggccgagccccagaagtcggggcccgggccaggagtcttggtgcaggcggactcgggcgcgtgccatgggaccacaactcccggcacgcaccgcggactgcgccgaacacggttggctgggagatccaaccctactgctcccaccggccaatgggacggaggaaagaggcctgacccggattctcggaggccaatggcaatacagaggaggcgggtgcttccttaccactcaccttgcgctcagagaagccacatttaaaaggtcgtgccgggccgggctttcgcaggcagtgggaccagagccgggaggggcggcggtgtcccgggaaagcggctcttggggcatccgggtcccctcgaggcgggctccggacgtcgccgtgggcggggccgagggcggggcctggcctcgttgtggagcggctcgtaatccatcatggcggccgcggggtttggtgtctgtgcctgagcagcgctggagccggagccggttcccgggtcctgcggctgaggagcccctccgctgtccacggcccctaccggcggggggcggctgggtccctcggcggagctcgggagatgtgactgcctgagggcggtggtggtgtcagcgtccggggccgggggagggggtgtctcgggcagagacccccgggcttggggcagctgaggcggccgggcctcctctacacggggcccgccttccgctgtctgggccgcgagagtccttcgtcccttacagccccgccccggctttgggacactgcgggtggtctgtttcccccagcttgggacaccccgttttctgaggcgtggaagagcgtcgccccggagtaagctgcccgtgccgcgccccgacagcttccctcagccccaagccgccccttattccggatcccggccccaactttggccacggagcctcccattcaaatccctcccttgctgtcaaggggtctccccttcccccaaggtggctcccgcgagcctctaatgccctgacttcttccaatgtcacctacggcccccttagtctcagctcagccaaaaactttaatgcaaaggaaaagtctggattggttccacaggccttttaaaaagcggacttaaaagttgctggcaatgcattccttttcgtcagagtcgagggcaaactcgctgaaatctgggtgacccgtgtccttttccggagagcaaagcagagaagcgagagcggccactagttcggcaggaaatttgttggaagatgaagaagctaagatagggggttggtgacttccacaggaaaagttctggaggagtagccaaagaccatcagcgtttcctttatgtgtgagaattgaaatgactagcattattgacccttttcagcatcccctgtgaatatttctgtttaggtttttcttcttgaaaagaaattgttattcagcccgtttaaaacaaatcaagaaacttttgggtaacattgcaattacatgaaattgataaccgcgaaaataattggaactcctgcttgcaagtgtcaacctaaaaaaagtgcttccttttgttatggaagatgtctttctgtgattgacttcaattgctgacttgtggagatgcagcgaatgtgaaatcccacgtatatgccatttccctctacgctcgctgaccgttctggaagatcttgaaccctcttctggaaaggggtacctattattactttatggggcagcagcctggaaaagtacttggggaccaaagaaggccaagcttgcctgccctgcattttatcaaaggagcagggaagaaggaatcatcgaggcatgggggtccacactgcaatgtttttgtggaacatggtgagtgcttttcaaaatttctgctcatggttttcctcatgcattcatcttaggccttcaaggaactttgaacaacagtacttgcgacagttccttccaattccacttaataaatttgttactgtagttatctcttagtggaactttctttgtataagaaaaagttacttcgtgacttcggctttattcaaaatctatttgagttgcttatttcttgcctgattcctctgctaattcactgttgaccttggacaagccactttactgttccagggctttagtttcctgaggggctggacttcagtggtttcttagggtccctggttctatgattctgctctaaccgaagtcgtgggctcttctgacaagcatggattctttactgctttgtctacagagagcttttatcatattctcaaagtggtttgtgttcctgagaaagttaagaatcatagatactggttgacgctaatatccttgaccttttccttcgtaagtaggacttgaaaatactcactttggagccatgtgggaaaaatcaagtggggaagcagcattccttgtgaattttagatagacagcttctgtcttaccttccataaggagtaatctcttcctcgttgatgaagctttcatcctgtcttctccctgtttagaatgatatttgggccaataaaggttatctgtgacatttttatgaacatatttggcatttgaatgctgcccgtacattttatgttgttcatgtccagtaattctgtgcgaagttaaagctaagggtcggcttacactgatgtctataaccagttaattagggttactgtttgtactgttgcagcctgacattttttggattgtgtcctttatattaaaaaatcagttgagcccacctatcctataagcaaacgtatgaagtgtgccagtggcttatactttgaaattcattcagaaataccccaacattgggtgactgcagtcaacaaaggcttctgttggatgaacttgcatttgacagctgaagttttactttcttacgggaaaatattcacttcatctaaataaatccgggtgcttggattttactttgccttgaaacattagttctattttagctttgtttttaggcaggcaaatatggtaatgtgttgttatgatggttcccaaattcaggatttaaaaagtgaattatttacattttaactagtgatgatcatgcaccttacatagtgaaaattggaacagactttttggagagctttggcggaacttatcagaatttgaaatgtacgtgccaatgacccagtaatcccattctgggaagctagtagagaaagcagtgtagttccctgtgtgtccctgatatctcttcaggggttgagaggctaaaactattttcttgttaatagagtaccaaggtcttgtctcttttgctgtgttgacgtttgcagtaatggtacaaaagtaaagcaggtgtcttagcatgattcagggttgtggcacctaactatacttgtagtcattgcattcttcatgacgtgcactcacagttaaacaaactaaatatatatatacacacacacacacacacatatatatccacttttcactgaaaaatgtcctttttttttttttttttttttttgagtcagagtctctgtgtgtcacccaggctggagtgcaggagtgcagtgtggcgatctcggctcactgtaacttctgcctcctgggttcaagcgattctcctgcctcagcctcccaagtaggtgggactacaggcacgcgtcactgacgcccggctaatttttgtattttttagtagagacggggtttcgccatgttggccaggctggtcctgaactcttgacctcaggtgatccacccaccttggcctcccaaagtgctgggattacaggagtgagccactgcgcctggctagttttcactggacaataccttgatgaagcagcaaaaattattaattttattacattttgacccttgtgtatgtcttcttaatattctgtgggttaaaaaggggggtatgcatcaagcacttctgtacagtaaagtataatgattatctccaggaaaagcactttcgtggttgggttgcaaactgaactagccacttttttcatggactgccatttttacttgaaactatgacaaactatggttattcagactaaaaagtgtatgaaggaatctttcaaagaaaacaacaggtagcatttgttgccaatgatgaaattttagctttccagtgaaaattaggattttggagaattttttttttttcctcttcggggtagagtttcgctcttgtcgcccgggctggagtgctgtggtgcaatctcggctcactgcaacctctgcctcccgggttcaagcgattctcctgcctcagcctcccaagtagctgggattacaggtgtgcaccaccatgcctggctaatggagaatttttatctgcctctgtgatatagagattggtggtaatatttacagatgccatattttaatatcttataatgaaatgtattatttggaagatctacataaatcagtaaatcaatattttcttttttgtttgtttttgcgacagagtcttgctgtgttgtctaggctggagtgtagtggcatgatctcggctcactacaacctccacctcccaggtttaagcaattctcgtgcctcagcctcctgagtagctgggattacaggcatgcaccaccacaagtgaataatttttgtatttttagtagagatggagtttcaccatgttagccaggctggtcttgaactcctgacttcaaatgatctggccacctcagcctcccaaaatgctgggattacaggtgtgagccaccgtgcccagccaaaccattattttctaaatgatcaatgcatgatataaaatcatgcacaggttaaagatccattcaaagtgcaaaatggaggccaggtgctgtggctcgtgcttgtaatcccagcactttgggaggccgaggcaggtggatcacctgaggtcaggagttcgaacccagctgtgcaatctagtgagatcttacctctacagaaatttaaaaaattagccaagctcccactggagccaaagagtcgaggctgcggtgagccatgaacacagcactgcattccaatttgggcaatagagggagaccgtgtctctcgggggtaaaaaaaaaaaaaaatacagttcattggtagagtttcttaaaggcagccagcctttaagaaattcctggctaggccgggcacagtggctcacgcctgtaatcccagcactttgggaggccgaagtgggcagatcacctgaggtcgggagttcaggaccagcctgactaacatggagaaaccctgtctctaccaaaagtaaaaaattagccgggcgtggtggcacatgcctctaatcccagctactcaggaggctgaggcaggagaattgcttgaaccccggagcggaggttgcattgagacgagatcacaccattgcactccagcctgggcaacaagagcgaaactcttgtctcaaaaaaaaaaaaagaaattcctggctgggtgtggtggctcacgcctgtaatcccagcactttgggaggatgaggcaggcggatcacttgaggtcagtagttcgaaactggcctggccaacgtgatgaaaccccgtctgtactaaaaatacaaaaattagatgggcgtggtggcatgcacctgtaatctcagctactcaggaggctgaggcaggagaatatcttgagccccgggggaagaggttgcagtgacctgagatcgcaccactgcacttcagcctgggtaacagaatgagactctgtctcaaaaaaaaaaaaaaaaaaaagaaactaccatttaccatgttttgatgtagcatcaaagaacaatatctacggttatctagaaagtctgttttggggggagaaaacagttattttccagtaataaaaatatttgtttttaaatgaataattatgtttttaaatttcagtattcatttctaatgtggtaactattgatgagataacctacacaaactaagcctcttaggggccttcagttatttttcaagagtgtgacaagggcctgagattaaaaagtttgaggccaggcactgtggcttatgcctgtaatttcacactttgggaggccaaaggcgggtggattgcttgagcccaggagttcaagatcatcctgggcaacataagaagaccctgtctctacaacaagaacaaaagaaattagccagacgtgttatcacacctgtgttcccagctacttgagtggctgaggtgggagggtcacttgagctcgggaggccaatgctgcagtgagccatgatcacgccactgcactgcagcctgggtaacagagcaagaccccatctcaaaacaaagtttgagaactgttgctatggaaagtctatcaagaaggcacatagggatgtttcttgctgaagtactaacactgaatgatgtctgtgttgtggtgagtagaaaaaaagcaatttgaaaatcattatttatggtatggccccatttttgtaaaacaaaaatatctgtttatttgtgtatgtccaggaaaaaaaagtatggaaggattttacaccgaaatttttatctctagggacttggagctttaggtggaatcggagaaaactttctctttttggtttgtgtgatgttccaagtgtctttttacaacaaacttgggttatcttataatacgaaaaattcgaagatttaaaaactgaggccaggcacggtggctcatgcctataatcccagcactttgggaggttgacacatgtggatcacctgaggtcaggagtttgagaccagcttgaccaagaaggtaaaaccctgtctctactaaaaatacaaaaattagctgggcgtggttgcaggtgcctgtagtcccagctactcgggaggctgagacaggagagttgcttagacccaggaggtcgaggttgcaacgagctgagattgcacgccactgcactcccagcctgggtgacggagtgagactccatctcaaaataaataaataaataaaaataaaaactgaattgatgacagcccaacctgtcacttttttcagatccctttttatgaaagaatttgcttaagttgtgtctgaagacaaaccaattactttggaccctgggtattctttttctaagggaataccatgttattttgtgttacagattgtttgcgatctttcatagcctgatctttctagagttggttaatatccatgtaggttagattgaaaaacttgaattcagaaatgtacggtgttggagcagacatggatctggaagccaagaatagcgttggtgttgttgttgatggtgaatctgaaagagtgggcagatggcaactttttgccagaatcattcagggtcaaagggctagtcatatttacaagggaaaagaggaaaccatgttattaaatatttcatgcaccatatgttcctttcaaatttcagtggcttgactaagaaaattcacttttgggagagttggtacaacaattgaaagcacttagtagtcaactttttccttagtgtttccttcttccttcaacaaacatttattttattgagcacagactatgacaggtcgtgttgtagtcactgatgatatatttgtaaacaaaacaatccctgccctcctagaacttacattctagtgggaggagacacatcataaataagctaagtaaataaaatacagatatgttagtgatatgtgctgaggagaagaataacatagagaaggggacagggaatggggtaggaggtgtaattttagttagggtggctagagaggcctgactgagagggcggcatttgattaaagacccgaaggaggaagatgagcagcaggccctgttgaaatatgtgaaagaatttcaggccgagggaaccaggatgcagaaacctgaggcagagcttgctagtttcaaggagcagcctagaggccactgcaccagagcaaagagcaaaaggagagatgcaggaggtaaaatggagggtgggaagagaatggctgaaggagagggtggccttattggcccatttcaaggattttgactttgattcatatgatgtgggaaggccttggagaattttccgaggggactatactatctgatgtatgtttcagtatgaaatagaatctctctggctgctatgatctgaaggaggacaagggagcagggattccacgggggcattgattgcacagagccaggtaagagtgatgatgcttggaccaaagtggtggcactgggtggagggtcagaaccgacaagatttgctctcggattagatgtgggatatgggggtgtgagaggggccaagtgtgactctcaggttttcgaactgaataactggaagaatagagttgccttttattgaaatgaaggtcgaggctgcagtggtaagctgtgattgcgccactgcactccagcctgggcaacagagcaagaccctgtctcaaaaaaaaaaaaatatttaccatcaggtaaaaccacttatggttctcaaaactttatttaaaataatagacacttgataaatcaacactgtaggccgggcgctgtgactcacgcctgtcatcccagcactttaggaggccaaggcgggcggatcnnnnnnnnnnnnnnnnnnnnnnnnnnnnnnnnnnnnnnnnnnnnnnnnnnnnnnnnnnnnnnnnnnnnnnnnnnnnnnnnnnnnnnnnnnnnnnnnnnnnggttttatcagcttccatacccaaacagaaatacccttaaggattttcttctctgattgcactaaatctataggtttctttgatcctagaaatgaataatagaatataaagaattcttattgatgaaagaaagctatttcaggaaacttttttttttctgttaatgataaaggctaaatgattcctgtcaattgtttcaaattttcaactttcaaaatacctgctgcttctttccaattcacctttctctattctttttttttttccaattgtatttttctttgacactcagtacttgtcccttgatagtggagaccatgtttatacattttcatggatcgaacagtatttttttttaacagactagctacttagtgaatacgcagttgaatctacttgtttggcaggttcaggcattgaacaagtactaagtgcctgtcctgtatcaggtactgtgtcagtctggggtaagagagccaggaacaacatagccaacaaaaggctctttgtgtctaatttatattcctgaggaccaccactggccatctgcttgggagaatggttatggcttgaataaacagtgtggaatgggtccagggaaccggctgaggaaaggggacatttactcaacctgatcttctttgttaagcagtggagagacccctggtggagccagcagtatcctttatctataatagcttgcttttcatcttttttatatcagtggctgcctgtggcctctcaccaaatctggtggactcattttctctgtgtatttagtttttctcctggaaatgactaacaactgcttaagtccttattcctttctccaggtttctggtgctgccataatttgttctatccacttgggatactgctgtagtgggaatattgtccctgttaccatcttcaggttacaaaccttttccccagcttgtggtaaaatcccgggggtctggtggatcccactcattttaggatgtatatgggaagctaacattataggcacagtgttttttttttttcactgtgtccgtctgttcttcagaggagcaaaggctagcatgacctttaagtcctcctttaagagtactgaatttctgccaggagcgtggcttgttcctcaagtgtcgctaggtgaattgttaatagcaaggagggatgaaattgcgaaatcttaaaaagtagagaattccttcagatttcattcttgagaggtagaaaacaggaaatagaattgctaaacagagaaggggagtgtttttaatagagatatttgtatgagaataagaggatggagccataatctgaggatgcctgtcttgtttgctctttggcttagttggatcttgggttggtttacttcctgtacaaactgtgagttagtagggactgaatttacagtaatatctaaactgattggaaccttcacttgaacagaattgagttttgcgtgttcacttttaagagaaagaaacaaaggcagccaacccagtatcaagagtttagtcaaaacaaacaactcccagatttgccttggtagtgaatagattcagcatgtttgtactttctatttcttcagtatcatatagtaatttattgtttcattggtgattttgcagcatcctaggttgcaaagaatatctcttgtggatgtgtaaagttaaaaaaaaatttttttttcttgtagcagggtctcagtgttactcaggatggtcttgaattcctgggctcaggtgattctcctgcctccgcctctcaggtagctgtgagtacaggcgtgcaccactgcgcctggctgtaaagcacttttttttttttttttttttttgagacagagtctcactcgttgcccaggctggagtgcagtggcgtaatctcggctcactgtaagctccgccacctgggttcacgccattctcctgcctcagcctcccgagtagctgggactacaggcgcccgccaccgcgcccgccaccacgcccggctaactttttgtatttttagtagagatggggtttcaccatgttagccaggatggtctcgatctcctgactttgtgatccgcccgcctcggcctcccaaagtgctggggttacaggtgtgagccactacgcctggcctgtaaagcactttcatatacttttttgtgaggtctatggtataggcaggatacgcattattcctttctttcagtaggaaaacttgtgctttgggtagtcgtgtttttagggttacattgctgattagttttagagctgtggttgaaatcaagtgtctcttgacagcttgagtgtttttcaattggaaacattactttttgaggatagactaatgcattttgaaaacatttgcatcattgaaatgagtggggtctagctttagaatttaatcaaatttttaattttttcacaatttcgtggtatgatttttaatactctattgaatattcttttttttttttttgagatggagtctcgctctgtcacccaggctggagtgcagtggcgcgatctcggctcactgccagctctgtctcctgggttcatgccattctcctgcctcagcctccccagtagctgggactacaggcacccgccaccatgcctggctaattttttttgcatgtttagtagagacagggtttcaccgtgttagccaggatggtcttgatctcctgacctcgtgatccgcccgccttggcttcccaaagtgctgggattacaggcgtgagccactgcgcctggcctgaatcttcttttttttttttttttgagacagggtctcactccgtcacccaggctggagtgcactggcatgatcttggctcactgcaatctctgcctcccaggttcaggcaattctcctgcctcagcctcccgagtagctgggatcacaggcgtgtgccaccaagcctggctaatttttgtatttttagtagagacagagtttagccatattggctaggttggtcttgaattcctggcctcaagtgatctacccgcctcagcctcccaaagcggtgcgattacaagtgtgagccactgcgcccagcctctattgaatattcttaccctttggtagttgagtgttttggaatggcggtgtgtaacaaacataccttatgtatgcttttatgatttataattttatgctgttatgaaattttataattataaaattatttataatttaaaaaatttatacattgtcctacaagctttgtggcagttttacgatttattttaaaattaaattgaactttttttgttgtgtttttttgagatacaaccttgctctgttgcccaggctggagtgcaatggcatgatcttggcttactgcaacctccgccgcctgggttcaagcgattctcctgcctcagccttttgagtaactgggattacaggcacctgccaccacatctggctaatttttgtatttttagtagcgatggggtttcaccatgttggccaggctggtcttgaactcctgacctcaggtgatcagcctgcctcagcctcccaaagtgctgggaatacaggtatgagccactgtgctaggcctaaattgaacacttttgaatagataatacattttctaatttaaactacaaagctacagaacaaacatgtattttcagaagcttgcttgcacctctgccactctgtccttttccttctcctactcctctggaaaattttttgtgtgtggttttttttttttatccttccagtgttcttttttgcaaatacaagcaaatatatatttattacacaaaagatagcatacagtatataccgttctgtaccttcttttttgtttttcccttaatagatcctcaggatctccccatattggaatatgtatatcttccttctttttatggctgcattgaattccactatcttggaagtatcattggttttccaaccagttccctttctggacttttggagtgtttccagtctttagatatgataaacagtgcttcaggggtaacgttatagctgtgggagagattcctaaaagtcggggcactgggtttaagggtacatgcgtttgtcatttctgttagtagatggattctacttggtagatagctaccattttgcgtatgtctgtgtgtatatatatgtgtatgtgtatatgtgtgtgtatgcatgtgtgtgcatatatatatatatatatttttttttttcttttttaagacagggtctggctctgttatgcaggctggagtgcagtggcatgacctcggctcactgcagcttcagtcctcggggctcaagtgatactcctgcctcagcctctctagtagctggaactataaatgtataccactatgcctggctgttttttgtattttttgtagagatggggttttgccatgttgcccaggctggtcttaaactcctgggctcaagtgcctccttggccttccagagtgttgggattataggcatgagccaccacacctggcctgtattaatatagagtaatagagatctatattggtagatatttccacattttcttccgtagacatcattctagtttacagtcccatcgctggtaatacagagattgccttcatccccaaagcctagctaagagagtgtattgtcaagctttgggactttttccaatctgatatctaagaaatagtattttagtatggttttaaatggtaggtcttctgtgagtgaggttgaacattgttttgttttgttttgttttttgagacgaagtttcgctcttgttgtccaggctggagtgcagtagtgtgatctcggccccaccgcaacctccgcctcctaggttcaagcaattcttctgcctcagcctcccaagtagctgggattacaggcatgtgccaccacacccagctaattttgtatttttagtagagacggggtttctccatgttggtcaggctggtctcaaacttccgacctcaggtgatctgcccacctcggcctcccaaagtgctgggattacaggcgtgagccactgtgcccggccggttgaacgtttttaacatgtttaggggagatacatacttatctttctgtgaaccatctcatcaggttctttgtgtggcagatatttaaataggaaactatgtagggcctagttgattgcctatatagaatccagtaccctgtctatgccccttcactgcccaagcatgtcacaaggaactgccctattccaagctccagaggacctgctgagtaggtgcttttcaggagcttgaaaagactgtttccaggtctacccccaggggttaatttaattggtctggggagaggcctaagtatcagtttttttgttttgttttagttttttagtaaggagagactttattgaaaaggatttttgcaaggaggggaaaacgactgttgaaatagggaggacactctgaccataaggaggtgtgcaggcatcttctttttcaaaaaatgttttcagttttaaaatttaaaaaaaaatttattttatttatgtatttattttgagatgaagtctcactctgtctcccaggctggagtgcagtggcgtcatctcagctcactgtaacctccacctcccgagtttaagtgattctcctgcctcagcctcccaaatagctgggactacacgtgtgcactaccacacccagctaatttttgtatcttttgtagagatgggggtttcaccatgttggccaggctggtctcgaactcctgacctcagatgatccacccgccttggcctcccaaagtgctaggattacaggtgtgagccaccacacccagccacctggacatgtttaaagaacccagtacctcaggtttaaggagcttttatgtttggtccagactacgtttcagggaagccacaagcagagtttaaagcctgctgagcaccgagctggttcttggtgctaacagggctgagactagtgaaaaagtcatgttgaggcatctgctcagttccagtgtcttccttggcatctgcttgtgcctactgtttgccccctttgcctgtgtgttaaaacagcctctgtctcagaacagtgtcttttttttttttttttgagacggagtctcactctgttgtctaggccggagtgcagtggcacaatctcggctcactgcaacctccacctcccaggttcaagatattctcctgcctcagcctaccaactagctgggattacagatgtgcaccgccacacccagctaattttttgcgtttttaatagagatagggtttcaccatattggttaggctggtctcaaactcctgacctcgtgatccgcccacctccacctcccaaagtgctgggattacaggcatgagccactgcagtgtcctttcttgaggaatggtggtctattaggagaaaaaccaaaagataagacctgagaccaaggaaattgtagtctcaatgcaaagatacaatcagaacattgcacaagggggaaagaaatgtcatgctagtgtttgtattttaattgtctttccttatttagaccaatagtagtaacaggtaacttgggttgcatgcttactaagttccaggcagtagtcgaataacttttaatatttaatattcagaacaataaggaagaaatgaaaactaagaacttactagcaatccggagtttatatttcttgaaaagctcattacaggtagttgctggaatgagatagtttgtgtgcatgaagaagaacacacaaaaatattaaaacatgacatgagtgatggtaatacagcaggtccccagataatggcctttcattcactattgtttcattatcatgttgatgagaaaaaaaaatcaattccctgctggagctactgtctatttggaatttacacattctccagtgtcctcgtggaacttaactcttgtttatatcaattaccttgccgattgatggacaaatcatggaaaattggttttgttatatgtcattttgctcaaagccccagtttccaagaacctatcaatgacattaagtgagaacttactgtagttattccctccccattcaaaacaaatttattgtttagaggatataaggagaaaacattttttccctcagatgtatccttctgtgtgttatgtgtctttttcttttgagacagggtcttgctctgtcgcccaggctggagtgcagtggtgcgatctcgattcacggcaacccccacctccctcgttcaaacaattctcctgtctcagcctccagagtagcggggagccacccgctacaggcgcgtgccaccatgcccggctaatttttgtattttttttagtagagacgtggtttcactatgttggccaggctggtcttgcactcctgacctcaagtgatccacctgcctcagcttcccaaagtgctgggattacaggcgtgaaacactgtgcctggcccgatatgtgtctttttaggcaagcagtgcttatgttgtttgttagtggtaagctgcctttgtagctctgtgttaccttgagtgagacatgatgtgatgtttagttcgtagcatcctcagcactgtcttattcacaatcattgtcaatctaaatgcatagtccttcctgattttttttttttgaaggctttttaaaaaagtttaattgagatatggttacaatggagaaaaaccttcaggaaatataaatgtaaaaaaaattttttaagctttattatttattataaaaacaacatacatttttgtaaattattcaatcaaggaaaattgattcagaaagccatttgaaattcaatcagcatgatcaatgatactttaacccctattcaaatgaaaattatcctaattaaaagtaggtgccctaagaccatttttcagggtgcatttgggttctattgcttccacatcaggaactcataattactgtatggattttataagttgatccaaccatggtatgacttctgtgggtactggtaagtccacatcattgctttgtaataatgtataatcatgactggatgcagtggctcacgctgcaatttcagcactttgggaggctgaggtgagaagattacttgagctcaggagtttgagaccagcctccaacatagggagaccccaacatagggagaccgcatctctacagaaaataaaaaataacaataaaaaatgtgtagtcacaatgttaaagtgaatcagaagagttgctaagttatgatcctttaattgaatcaaagttttttgtttaaattggcttgctgaggagtttccagtaaattaataatgaattatgtaattaatattatgttaatattaaatgttattttaatcaggtcactgccctgcatgccaacttccactgaagtgggaatgtttcacagtgattcagtggccaattagcaatgctcagattcgccatttattgagagattcacacacacacaatcaatcaaacattcacaatgtggttattaaaggctgtaattagggggacaatgaaccacagggatggctcagaaggtcagagcactgatggaccctcaagtgggttggaagtcccttggatgctagtaagtgaggagtggctgttcctctcctggagagccgctgggcggcaattgtcatgctaggaggaggcctcagagttctcatgggcaaagattccaaaggcgccccagacatcatcagctccttgctgtgtgtatgattctccaaaggtctgcccagtatcatggtctcagccagctcttggctccatttttccatcggtggtggtactatgccacagcaggtgttattatctcaccaccttattctattagacgtatgtttatcacttcgaagaaaaacaattttactatgatctcagttgccaggctagtacacatgtgcttatcattctttgtttgcttttcttttgagtcaaggtcttgctctgtcacccaggttgaattgcagtggcacgatcatcgctcacttcagcctgtaattcctaggctgaagggatcctcccacctcggtctcttgagtagataggactacaggtgtgcaccaccacacccagatttttttttttttttttttttttgtagagaaggatctcactatgttgaactcctggtggcctcaagggatcctcctacctcggcctcacaaagtattggaattacaggtgtgagtcactgcagctggccttcacttatcactgtgaggagtaaacagctgcatggtgggcttaatgccatctaacacgagtgactccatgttcagacagtaggatcacaaatgattattatatagcaatgaatggccacaggtacatagactaaggagccacatccctgctcctgggatatcctttagtcaaagggctagaagggtcctggaggtttgccacttctccgtgttgaggtacagagttcctagactaagggactggctgcattgttatgtgtgagtgctagtcatggtgctacctggcacccacaaatgccacagcagacccatggtcgagggagaggagcaggaataccagttaccatgccggagtaacagttacggcactgatgcaccagttaccatgccagagtaacagttacagcactggtataccagctaccatgccagagtaacagttaccacactgatataccagttaccatgccggagtaacagttaccgcactgatgcaccagttaccatgccagagtaacaattatagcactggtataccagctaccatgccagagtaacagtcaccacactgatatactagttaccatgccagagtaacagttaccgcactgatgcaccagttaccatgccagagtaacagttacagcactggtataccagttaccatgccggagtaacagttactgcactgataataccagttaccatgctggagtaacagttaccacactggtataccagttaccatgccggagtaacagttaccgcactggtataccagttaccatgccagagtgactgattttgaccaagacctttgggttgtacagaaggggtgagaccatacctgtcctcaagcatttccaacctagtgtagagaaaaacaggagcaagataagaacaatgtactgaaaaggaaattggatgagggcctggaaaaaggggtaaagtgagctggttgggattggtgagtgccacagcttcctgccccttaacagatcagtgccatggtggctgtggtgtccctggcccagaccttctcagacagggcctgggtgccctttacagagcagttgggaagagaagggaacctagccttgtgaccttttgctccacagacctagtcctttgttgtggtgcgaggctcagtcgtcagcccaccgagtcatgtatgttctctggttgcccctggttttggctgaactcaaaggatggctgtttgtgaggagtactggtactttttgccacttgtgtgccctaactgtggtggatgccattttggggattatgctcagcagtgagtcacgtgagatgcacacgtagcttttcggtgattaatccaggtcaatgcccttacccacatacttctgagatgtactgatgatgactacatttaaagctttttctccattggctagaagttgagacccatttcaacaaaagcacttccacctctcctgaagtgcattgggaaaactggaggccattactagatttacagatgatgggccgtgcttaaataacccatcttagccagactccaggtttcgtcacatattccctacctgttgctgccattgagggctttctctgtgctaggcactaccaaataatgctttggtaactttggtaatttggtaaacttggtaatttggtaaatttggtaataaagagcctttattctaaagtgcaaatctaaagtttggggttcagtagctcaaaactctctggtggttcccattatatagagtaacagtcttcattttaaaaaaggtcatgtacccttattagaattttgtgagcaaacaaatatgtgtgtatcgtatgtatgtttatatgtatatcagatgtacgcacattagtatgtgctattaagatactttatattatataatatatactgtataacaccgtatattataaagcattcataaaatgaaaatgaagatgaaataaattgcattgtaaatatttaaaactttaaaaaatgcgttactggtacaaaatttttttgtttctaaaaaattattattaatgagcaatgggactgaatttgcttcaccgtttttttaaaatcttgatttaacatttgtcatacagctattttaacatcttacactaaagttgattcttgttttttggagacagagtttcgctcttgttgcccaggctagagtgcagtggcgtgatatcggctcactgcaacttccatctcctgggttcaagtgattctcctgcctcagcctcccaagtagccaggattacaggcttgcgccaccacgcccggctaatttttgtattgttagtagagatggggttttgccatgttagccaggctggacttgaactcgtgacctcaggtgatccacccgtcttggcctcccagagtgctgggattacaggtgtgagccaccacgcccagcctagtttattcttttaatagtgcttgggggaggtagcctctaagatgactcccagtgattccccacctcctggtattcctggctcttttgcaaatgtcaattctaatttggtcctaaggtctctctcttgagagtggctatagattctagccctgcccaggaaaataggtttgaatgcattggtcaggtgagacacagagcagcacagcaagacacatgaaatagcagaagtatttttattacttactgatcccagagaggagagagagagaatcctgggccaaaacctttattgggagtccagggagtttcccaagtgggtttcctagggctattatgttaccgaagccaatagttctaattgatgggtttaaagggagcaggcacaagctttgtgggggtcacgctgtgattgagacatggtcactgtagcatattcatctagtacttgtggggtcggggaacaagaggggtgagccacataggccctatgtagctgtcctgtaaagaggtaggggaggtggccatcaagaggcatggtgttaggcagatgtctggagtggccacattgagggattggaagcgggtgtgtttctatgctcccttaaggatatttttggaaacaacatgcttgctgcatacaaatattcaaacattttatctttaaaacaaattttagtactggtaacatttattaacttttttttttttcctgttccctaatttgctacccagcttttacatcaaagctcctatcacaacccttcttgtttttttctttttttccctgagacggactcgctctctttcgctaggctggggtgcagtggccacaatctcggctcactgcaacctctgcctcccgggttcaagagattctcctgcctcagcctcccgagtaactgggactacaggcgcatgccaccatgcccagctaatttttgtatttttagtagagatggagtttcaccgtgttggccaggatggtctcgatctcttgacctcgtgatccacccgcctcggcctcccaaagtgctgggattacaggggtgagccaccacgcctggccccttcttgtttttgtagcttgtcacatgatgaatgctttttaccctgggggagaccaagactttgagtaatagtttgcttttataagccagaatttgttctacacatagaaggataaaactgtcttttctggccaggcgcagtggctcacgcctgtaatcccagcattttggggggccgaggcaggcggatcacgaggtcatgagatcgagaccatcctggctaatgtgatgaaatgccatctctactaaaaatacaaaaaaaaaaattagccgagcgtagtggtgggcgcctgtagttccagctactggggaggctgaggcaggagaatggcgtgaacccaggaggcggagcttgcagtgagccaagatcgcaccactgcactccagcctgggcgacagagtgagactccgtctcaaaaaaaaaaaaaaaaacaaaactatcttttctctctggtttctttgctgttccttttcaggagagaaattacaataggattggtggcctaatgatgtaagtgccaaagtttcattcgaggttttggggtagaatgtttttcaactgtttgcttttatctgagacaaagtgggcaaggaataaaggtagagtggtgagaagggtgttatcccttcctgggaacctttttttttttttttttgaggggggcagagttttgctcttgttgcccaggctggagggcaatggtgtgatctcggcttactgcaacctccacctcctgggttcaagcgattctcctgcttcagcctccctagtagctgggattacaggcatgcgccgccacacctggctaattttgtatttttagtagagacaggatttctccatgttggtcaagctagtcttgaactcccgacctcaggtgatctgcctgccttagcctcccaaagtgctgggattacaggcgtgagtcactgtgcccagccctgggaaccttttaattgtcaactgtgtaggtgttcatgctggcctgcataatagagcgcctgctgtttgattttcagttttctgtagaaggaaaaaaaaaaatcaaaccaacaatagcaaaactcatgatacctcctggtctctctctccctctcctctgcttgcatattctggtctataacaggaaatggaacctcctggagtgaggggaaaatgaccttcacatataggtttctcactctaaagttatttcttaaatattttagcctgagttcttttaataacagacctcagctctagttctttgaaatgcatgtgggaaaatgtttatcagtgttgaaatctgacatttttttaatctcatgaactccacaattgtctgattattaaagtcctgcttacttgactgtgactaaaattctactttcagaagagtagaatgtacccctaccaaattgaagatcaaataaataaagtggacctggaaaagtaaggcttgccattgtgtgtcaaaccagcccttcccagctgtgggctttgtacttacggactcagaacgtgaatggaagtacagactctggaacatgtaggagctgttatcccttgccagtttcatgcttcactgtccatctcctggccaaatagagagacaagggtgacattaaaatcatgggtttatctgaattcaaatctcagctgctcacttactaacagtatgaccgcagacaccaacaaaacgtcccactgctgcttatttccaagcctttccaaggtcttctggtcagggcagattcttctttcttgttcctaaatttaaagtttcaagaatttaatgcgttttttttttttaatgaatttaatgccttttggggggtaggttttcctaatttaactttatttttttaaattttatttttaaattagtgaacagtaaaattgactttttcaatgtatggttttatgaattttaagacatttatagatttgtataactaccattgccaccacaggacataaaatatttccataatcccaataactttcttcgtgctattctgctctcctgcctcctggcaaccactgatctgttctcatcactattgttttgtccttttgagactgtcacagaaatggaagcatctagtatgtaaccttttgagattggcttctttcactgagcgtaatgcctttgagatccatctaaatgttgcatgtgacaacagtttgttccttttcattgctgagtagtattccattgtatgaatatggcacagtttgcttattcattcatctgttgaggatgtgtttgggttgttgcttggtggggcattggtgattacgaatagagttttaagcatttctgtactgtttttatatgaacataattttttaattcacttagcatatactcttcctctgtctgctgtaataaggtaccacaaaactgggtggcttaaaacaacagaaaattattcttccactgttctggaggccagaaatctgaaattagtatcactgggccaaaatcagggggacagcagggccttgcttcctccagaaactccaggagagaaatacttcctggcctctctggcttctggaggccacctgcattgcttggtttgtgaccccttgtatcactctgaccccttgttccattgttttatttcctgttttgtaatcaagtctccctcaggctgggcacccctgagggagcatggctcatgcctgtaatcccagcactttgggaagccgaggagggcagattgcttgagctcaggagtttgagaccagcctgggcaacatggtgaaaccttgtctctacaaaaaatatttttaaaattagttgggcatggtggcatgcacctgtagtcccagctacatgggaggttgaggtgggaggatcacttaagcctgggaggtggaggttgcagtgagccaagattgcaccactgtgctccatcctgagcaagagtaagaccctgtctcaaaaaaccaaaacaaaatcaagtctccctcagtcttcctctttttttgtttgcgtggggacagagtgttgctctgtcgcccaggctggagtgcagtggcacaacctcagctcactgcaacctctgcctcctgggttcaagtgattctcctgcctcagtctcccaagtagctgagattacaagcatgcgccacaacaccctgctaatttttgtatttttgtagagacatggtttcaccatgttagccaggctggtctcgaactcctgacctcaggtaatccgcccacctcagcctcccaaagtgctgggattacaggcatgagccactgtacccagccccagtcttcctcttatagggacacttgtgattacatttatgcccactaggatgacggaggataatgcccccatctcaagattgttaatcacatctccaaagacccttttctcccatatagggtacattcataggttccagtaattaggactggcatatcttttggaggcccattttttagcctactacacttggctaaagacctaggaatgggtcactaggtcatatggttagtatgtgtttaatttcatgagaaattgccaaactgttttacagagtggcagtcatttcacgttcctaccagcacccttgaacgccagaattcctggtatcctcggctgaactggctagtgtcggtatttttaattttagccattctagtgagtatctcatcatggttttgcttttccctgacagctaatgaggtggattgagcatctttttgtgtgaaaacctcatatcttttaattttcctcctataacctgcataagtatgaggaagaaaagtgtgaactgaatcataactaaaggaaagaagaacattgctgtcttaagcagatcacgcctttgtcgttatacagtatggtacaataatccattacacatctctttgattcatcttgtctgttaaatttctttataaaatttgtttagttgatgacacacctgactctaatataagagttgaatgttgtatcacttttttttttcctttttctgagacagagtctccctctgtcacccaagctggagtgcagtggttccatcttggcttactgcagtctccacctcctgggctcaagtgatcctcccacctcatcctcctcaatagctgggactacaggcgtgagccaccatgcctagctaattttttttttttttgagacggagtcttgctctgtcgcccacactggagtgcagtggcgtgatcttggctcactgcaaccttcgcctcccgggttcaagcagttcttctacctcagcctcccaagtagctgggattacaggcatgcgccactgctgcccggctaatttttgtatttttagtggagacggggtttcgccatgttggccaggctggtctcgaactcctgacctcatgtgatccacctgccttggcttcccaaagtcttgggattgcaggcgtgagccactgcgcttggcctctatataagcttttaatgaataataaagactctaaattatgcttatttactaccaaataatctttttaaatgaaaaatttgttatccctcccagccctcagccatgacccgaagtatgaaataggcatatctttttgcctgctattaggctgtagttcatactggtttagtattgctgttgatcacttttagggacatttaatgatattttatactagatcttgagcaccagctatttattttctcttgaagcagtggtttatagtaatacattgtgctcagttcttttttggttctttgtcaagttcaacacagtagcttctgttgattgagttcttgtagttatgaggggaaattaatgctggtgaccagtatttgagaattaaaaacctctgttcagaaaggcaatgcagagtagaataatgaacggatactataaatgacatatcttgacactgggggtttagtataaataaacagtatttcaatctctggaaattgtaaagcccgttatttaacctaaaaacgttaatggctcagaaaacagaattacatggcatttccttgctaacctcccagagcctatcccctccaaagatgatagggctaaagcctggtccactaagttgttgtcagtcgtacgggctttagagtatgttgacttgatcaaacatttactgtttacaaatatttgcttctagctcatatcctgacacttaaagccacgtgatcttgtagaagtcacttagctgatgaggtaaaactgagtctgtttctccatctgttgaatgaggctggtgatagactctttctttgctctctcccaggtgggtaggagatcaggatgagctgatgtctgtgaaagaactttggatactataaagtgctttaggaatgtatggggttattattttatgaaattgttgattcgtcttcataatttgagatacaagatctccattccattgctaatgcttatggaagattttgtcactttcttaaaaaatattgccaaggccgggcacagtggctcacacctataatcccagcactttgggaggctgaggcgggaggatcacttgagcccaggagtttgagaccagcctgggcaacatggcaagactccatctctacaaaaattgaaaaaaaaataaattatccaggtgtggtggtgcacgcctgtgttcccagctacttgggaggttaaagaggaaagatcacttcagcccaggaggttgaggctgcattgagccatgattgtgccacggcactccagcctggacaacagagaccctgactcaagaaaaaaaaaaatacatatatatatatatatatatatatatccaagtataagtatatacttagaggtgggctggtaaaggctttttcattatggatttttcagtttatttcttctaagttttgtcagttgaacagtagggataaattaaagaggaggaaaaaaaatccccatcatccttccttccctccttccctccttcccttcctccctccctccctcccttcctccctcctttcctcactccctttcttttttgacagagtctcactgtgttgcccaggctagagtgcagtggcgtgatcttggcttactgcaacctccccatcctgggttcaaatgattctcaggccttggcctcctgaatagctgggattacagacatgagcacctgacctaacatggttctttttcttttttctttttctttctttttttttttttttttttttgagacagagtctcactctgttgcccaggctggagtgcaatggcacaatctcggctcactgcaacctctgcctcctgggttcaagtgattcttctgcctcagcctcccgagtagctgggattacaggtgctcgccaccatgcctggctaatttttatatttttattagacacagggtttcaccatgttagtcaggctggtctcgaactcctgacctcaggtgatctgcccctcagcctcccaaagtgctgggattccaggtgtgagccaccacgcccggcctacatggctctttttctattcagcttttttggtaggattgaggtagttgtagaggagtgttgataggatagtgaagaaattttaacctttgctaaaaacatgcaagacagtgtcataatgtttaagaatacataaatgttatcattttgtacatgtccttttgaaacttgttttttttattcagcttttttttttttttttttttttttgagatggagtctcactctgttgcccaggctggagtacagtggcgcgatctcggctcactgcaacctctgcctccccggttcaagtgattctcctgcctcaacctcccgagtagctgggactacaggcacgtgccacgacacccagctaaatttttgtatttttagtagagacagcatctcaccatgctggccaggctagtcttgaactcctgacctcaggtgatccacctgccttggcctcccaaagtgctgggattacaggcatgaaccaccgcgcctggccaaacctactatttttaatgggaaggggtttattatagatattatatagctaacagttatggggagggctgaaaaagcaggttcttggttgggcttcatgagtgattcccagatggaacggcctcatagacctgggccactgaggaagctgcagcctcttcaggaattgggaaggtgtcagctgtagaatctctgccacaatcaaagccttactgctcctggctccagagccaggtatggtcagccagcaaaattgatatcctgcactctgctcctcaacacccatgaagccagtgcctggacacaggactgctcgtcctgcctcagaaaaccaaatgctttccagccgggcttgcccacagcaacggcagaagcaacagatgtgtgctgggcctcccatctgctttccaaatctcatgtaattgtatccaacttgcagaccctaaatcacatttaaactgtaggtgcaggggaggtggtgatgtgtctgttagattttcagcctccgcactattagaaaagaagggaccctggaaggaggatggaatggctatggattatccatccaccatattcgctccaaattcttaacctgatatgaagatgtatgggtataatgtagggatgctttggaccctgtaattttatgcacacttgggaatgtgcaccagaacatttttctttcattagattctcaaaggggacgatgacccgacagaggctaagcaccattaaccagataagttaagtgatgaagtgcccagattctgaaggcaggcaggcctagatgtgaatcctgtctctgcttcatagctgttgtgagatcttgggcatgttatttcacttctgtaacccttaactttctcatctttaagatagggttctgaggatacttttatggaggtttcatggtaccagcatcctactgggaactgtaactcctgctgcctaccaaatatctataatatctttggcttggcactcaaggtcttctctgaagtagcccaaacatgctttcttgccctactgcagggttgctatgagggtgaagtatagaatgcctgtatggtgaatgcctggtatagtgcctggccccaaaaagcaaccaataagtagtcttctcttcccaaagctagtcactgcatgtatgtatgtattcattcattcctcagaagaacatggccaacatgaaaattagggtgtgctgctgccatctctgttaagaataccccttggtggctgggtgcagtggctcattcctgtaatcccagcactttgggaggctgaggcggacagatcactggaggccaggagtttgagaccagccatggccaacatatgaaaccccgtccctactaaaaatacaaaaaatagctgaacgtggtggcgaacacctgtaatcccagctactagggaggctgagactggagaatcacttgaacccgcgaggcggaggttgcagtgagccaagatcgcgccattgcactccagcctgggttacaaagcgagacttcgtctcaaaaaaaaaaaaaaagggctgggcgcagtggctcacgcctgtagtcccagcactttgggaggctgaggcgggtggatcacgaggtcaggagatcgagaccatcctggctaacacggtgaaaccccgtctctaccaaaaatacaaaaaaattagctgggcatggtggctggcacctgtagtcccagctactcgggaggctgaggcaggagaatggcgtgaacccgggaggcagagcttgcagtgagccaagatcgcgccaccgcactccagcctgggcgacagagcggactccatctcaaaaaaaaagaatacccttggtagctcctacttgtgctgcagaggtgaacttggctatcacttcctctgttcccactgcatgctgtgctattgctgtgctgtttatcacagtggtgtttactgtcttatacttgcctctctctcatctcttctttttttttcttttcttttttttttttttttttttgagatggagtctcactctgttgctcaggctggagtgcagtggtgcaatcttggctcacagcaacctctgtctcctaggttcaagcaattctcctgcctcagcctcccgagtagctgggattacaggcatgtgccaccacaaccggccaatttttgtatttttagtagagacgggtttttaccatgttggccaggctggtctcgaattcctgacctcaagttatccacccacttcagcctcccagagtgctgggattacaggcgtgagccaccatgccaggcctcatctcctcttaaatgtctttagagcaaagattgtgtcataaccccggcacctagtatcatgcctattacatagtagattttcaataaatgttaaatgcatgaatgaataatgagtaaagaaactgggtaatgtttttagcttggaggagagaagcctaagggaagatgtgtttgctgttttgaaaatatttattgtcgctgggcgcggtggctcacgcctgtaatcccagcactttgggaggctgaggcgggtgtatcacctgggtcaggagttcgagaccagtctggccaacatggtgaaaccccgtctctactaaaatataaaaaaaattagctgggggtagtggcgttgcctataatctcagctacttgggaggctgaggcaggagaatcgcttgaacccaggaggcggaggttgcagtgagccaagattgcaccactgcactccagtctgggcaacaagagtgggactctgtctcagaaaaaaaaaaaaaagagagaccaggcgtggtggctcacgcctgtaatcccagcactttgggaggccgaggcgggtggattacgaggtcaggagatcgagaccatcctggctaacatggtgaaaccccgtctctactaaaaatacaaaaaattagccaggcgtggtggcgggcacctgtagtcccagctactcgggaggctgaggcaggagaatggcgtgaacctgggaggcggagcttgcagtgagccgagatcgtgccactgcactccagcctgggcgacagagcgagactccgtctcaaaaaaaaaaaaaaaaaaaaaatttactatcatgtaaaggggagttggtctcaccctacactgctttggaaggcacaattaggagctgcggatggaagtcacaaaataaggcacatttggactcagtatgaaaagagctttcagataatgagagcaatcaagtaatggggggggccttggaagccagtgattattggtcattggaggtattaaaggagaggcaagataggaagatatagatggggtttgaataccgtgcggggcttctcagcactcttccttttctgagtgcttttaacaagcggactagggaatagatagggcctctgctctcagggagattattgtctgctcagggagagaagatatattcaggtgggaaagggcaaagggtgttaggaatggcttggctaggatagtcagaggagtacgtggagtaaggcaggaaagcatgtttgggcttcctcaaagatgaccttgagtaccaagccaaagattttggagatatttggtggacattgggcattatacatacccagtaagatattagcaccatgaaagctccacaaaagtgtcctgagcgcctagaacagtacttggcacatggtagatcttcaataaatagttgttgaaggaatttgttaaaatatcagagctatgatttaagaaaattattctgtaatctgaatttaggttgggagtggaaaggagtacccttaagtaggacatgagaagagcctgaagaaaggcagaggacaccagtaggcatcttggatgtgggattggtcagaggggagagaggtaaaaatgattccatgactgtgagtctggcgactagaaatgggggtgacattcacagagtagggtggttccctgtagttcctccttgtgcagaaggtgaggctttgcttgtcgacctgcttcagtagtagcattgacagaacagtctctgtgtactctgtcccctcagtgctttctgcatatgtgttgctcactcatcactatccgcatgttcgtggtctctggaaagaatcaactataatgatcagaataattgcctggtaggacgtatttcctttgagttcagcaagacgtgccccctcacatggtgttcctgttcattcataaggctgtaataatgtatgagttaggagacccttttgaccaattcccctctgttttccatcttggaaaaaccagaactctgttttcttgagcaaatgatgttgccaccagccctgaagctccttttcctgggtttgtaggggttggtggaatcctggcagtctgccgctcttcctggcctccagagatcagggctgtgaccttccatctgcagatggcagttctagctgcgaggttggtggccgaggaggacgaggacacagctcagggcctgtccttcaagggcttccgtgtgcagcagcagcactctgtaatatcatagatgaatttttgtcaaaacacagagaaaagttgattacacttctcatttattaaaaaaaaatgacttgatagcatagtagatggccccttatgtaagccacttagtattatttcaaaggaagcaagtctgtgagaaaaggggcaaccacttttctcatagagaagaacaggtttttaaatgaaaagatcaacaaatccaaatgctgtggtatttatactgatttagaaaggcagttgactttgggaggctttgttttctcatttcccttttctccttgacatttgacagacgtggttagcagagagctttctcattcggttttcctggagagagctctgcctcttgggcttcctgcatttgtatggaagttttaatttttttttttttgtcaaatgaaaggttgccatttcatttgttcagatttcccacacactgttgcagcaatctttagatttcaaattggctaattcagtgggtcacttaattcttaacttttacaacattttgagtctaaatacagcaaaattggtgcctttttcagctatttttcggcgttgctatattccaagccactgagctctgttttactctgacattttctcttcacttttgggattctgctcactgtgtttaaggcagctcgatagcattttgccaaaaaagagaagttagggctagtgtgagttgaggggaaggggatgtttctgttgttgctccttgctgagtatcttcagatatctaaaagaaacttgtaacacagcgtcagcctgacactggcctttgcagcatcagccttggttgactgtgttctaatagggatgcctgatctgtatcctctttaacttggctataagaaggttttggagaatgtatgtctgagggtgttttaaaagaaaatggaaacaaagctcctttttgccttgagctcatggtttggaatttgggcatttggaatccttcaagccctcctcctgggcagagctggagtccccttagggcactgcctgtcatcttcactacacagctgtgctccagagcagggagccgatggaaagggggacccagaacattccattctgcagaattcccttccagccgtctgtgagaaggcagtttgggacccttttagaagtttgctttataagtnaagaacctgaggccggctgtgttcatattctcagaacttggtgagaatgaggtactttaagataggctctaagatcagcagcatcagcccactcgggaagagctcctctgactcctggaggagaaagccagatgggggaagcattaagtcctgttttcctattgaaaactgaaattggccagccacagtggctcatgtctgtaatcccagccctttgggaggccaaggtgggaggattgtttgagcctaggagttcaagaccagcctgggcaacacgatgaaacctggtccctgtaaaaaatacaaaaattagctggggcatggtagcgcatgcttgtagtcccagctactagggaggctgaggtgggaggaccgcttgggcctgggaagcagaggttgcagtgaactaaggttgaaccactgtactccaggccttttttttttttttttttttgagacagagtcttgctctgtcacccaggctggagtgtagtggtgcgatctcagctcactgcaacctccgcctcctgggttcaagtgattcttctgcctcagcctcccgagtagctgggactacaggcacccaccaccaagcccggctaattttttttgtattttgttatagagatggggtttcactgtgttagccaggctagtctcgatctcctgaccttgtgatttacccgcctcggcctcccaaagtgctgggattacaggcatgagccaccgcgcccggccaggcattttttttatgtgtgtctcaaataaaaagaaagaaaaccaaaattttacctgaaagacgagaaagttgatgaagattttgagaaagtgaggaagcaatggcccctccagggcacacccaggtgctgtcccttcttttctcctcagttctcttagctataaaatggggcttataataatcccttccttgaagagatgttgttaatagtacttagatgatttgctaacttatatcaagcacttactctgacccaggtatcggactgggtgcttgacgtatattatctctattgtgttttgcagagtggctaagatttttttttttttcttttttgagacagagtctcgctctgtcacccaagttggagtgcagtggtgcgatcttggctcactgcaacctccacctcctgggttcaagccattttcctgcctcagcctcccgagtagctgggattacaggcgtgtactaccacgtctggctaatttttgtatttcagtagagatggggtttcaccatgttggccaggctgctctcggaactcctgactccggtgatccacccgccttggcctcccaaagtgctgggattacaggcatgagccaccagagacggagtctcactctgttgctcaggctggaatgcagtggcgcagtctcgactcactgtaacctccgcctcctgggttcaagcaattctcctgcctcagcctcccaagtagctgagattacaggcgtgcgccaccaagcccagataattttcatatttttagtagagacggggttttgccatgttggccaggctggtcttgaactcatgacctcaagtgatccatccacctcggcctcccaaagtgctgggattacaggtgtgagccaccgcatccggccccaatttattcaactttggaagcgttggttgtgagatgtgcagttgggtgttgtcatggagaagaattgggcccttcctgttgaccagtgccggctgcaggcattgcagttttcggtgcatctcatcgatttgctgagcatacttctcagatgtgatggtttcgccgggattcagaaggctgtagtggatcacacaggcagcagaccaccaagctgtgaccgtgacctttttttggtgctagtttggctttgggaagtgctttggaacctctttcggtccgaacactgagctggtcattgctgtttgtcgtataaaatccactttttgtcgcacatcacaatctgatcaagaaatggtttgttgttgcgtagaggaagagaagacgacacttaaacatgattttttaaaaatttttgctcagctgatgtgggacccgcttaacttcccaatttgcttcaaatgccaaatgatcatagaatggtcaacattgagtttttcagcaacttcttttatggttgtaagaggatcaacttctgtgattgatctcccagctggtcgttgtcaacttctgatggccggtcattgcactcctcatcttcaaggctctcgtctcctttgtaaaacttcttgaaccaccactgcactgtacgtttcattagcagctccttggccaaatgcgttgttgatgttgcgagttgtctccagtgctttacaatccattttgaccttgaataagaaaattgctcgaatttgctttttgtctaacatcattttcacagtctaaagtaaacataaacagcaaggaataagtcattagcaaaaaaatgtaaagcgagaaatgcccattaaaataatgtataacataaccacatttatttaagaatgtactcgaatatcaaatgacaaattccaacagtgtaaaaactgtgattccttttgcaccaacctcatactagccaggcatctttctactgaaactggctggagaccatgtctcagtggtggagccggtataggaggcttcacatttcttcccctaggacacgctgtcattgtttaggtttcttgttttgttttttcctgaaacagggtctcgctctgttgctcaggctggagtgcagtggcacagttacagctcactgtagctctaacctcttaggctcaagtgattgtcccatctcagcctctcaactagctgggactacatgcttgtgccacacatttaggtaatttaattttttttttttttttttttttttggagacggggtcccactacgttgtccaggctggcctctaactcctgggcttaggcaatcctcccacttcagcctcctaaactgctgggattacaggcatgagccaccacacccagccagttgtttagttttaaagatttaacctggttgaaatgtggctagtccccttatgcttgggtcacagaccaatttgggttaactttgccattgccttgcctgcagatcatggtgctgttgggatgtcattttgctgtaccaagggtaaacagtagctccctccttaacatcagtcctttagtgtaggacttctctattaagaactgggacgctgttggccattaggattcctgttccttttgggtttgtaatagaagctactgtccccctgatcattactgattgaaacaagaaatctgttgttcctggatttctttcagttatcttaacatagacccttccaagtcttacagatgtcaagggtttttgaaagtaggatgtattctgatctttttcaagtggctacatcactgaccctcataaaataacggaaaatattgggagatgacttttctgcttaaatgttaggaaactaaattctcagtatactgcttctctagttgttaaggaagaaaatttctcttgtaaactttttgggagactagatttatttcctcccccactttttttttttttgaaatggagtctcgctctgtcgccaggctggagtgcagtggcgcgatctcggctcactgcaacctccacctcccaggttcaagagattctcctgcctcagcctcccgagtagctgggactacaggcacgggccacaacacccagctaatttttgcattattttttggtagagacggggtttcaccatgttggccaggatggtctcaatctcttgacctcgtggtcagcccccgcaaagtgctatttcctcccccgcccctgcttttttttttttttttttttttgagacggagtctcgctctttcgcccaggctggagtgcagtggtgcaatctcggctcactgcaagctccgcctcccaggttcacaccattctcctgcctcagcctcccgagtagctgggactacaggcgcccaccaccacggctggctactaatattttgttttcggtatgtttttgtatttttagtagagacagggtttcactgtgttacccaggatggtctcgatctcctgacctcgtgatccacccgccttggcctcccaaagtgctgggattacaggcgtgagccactgcgcccggcctatttcctcccctttttatgaccattcacagcctttggcataccattaaaatctgatcattgacttctaggtgggagaatggcatctctcttttctcctcatgataaggacttagtctgtaaaccttccagtccctccctaccctgaagcctcccatggtcttttctctctcccttgtgaaggaaaggtccctcttttaaagcattattcagaccggaaggaggacaaaatcaagacatgctgaaaaacccctgttttaatcaactccccttttaattttttcaaaagtcattattaggcatcgaaagctgttgaccttcatcaaacaatgagcacaggatttcttttccgcatcacgcgtggtgccactccagtgctatggtgtgatcagaacacccacattaataagaacattacttctctgaagtaatttgaatcttcatttagtaagactaaccatttcttcaaattttgttttttagtatacaggaaagttacaggttttttttctcttttatttgacaaatgaaagtgattttatattcatcacattacaaaataaataaatgctcattatttaataagaaaattcacatctgggctcagtggctcacacctgtaatcccagcactttgggaggccgaggcgggtggatcacctgaggtcgggagttagagaccagcctgacgaacgtggggaaacccccgtctctactaaaaatacaaaattagctgggcttgctggcgcgtgcctgtaatcccagctacttgggaggctgaggcaggagaatcacttgaacctgggaggcgaagtttgcggggacccaagatcacgccattgcacttctgcctgggcaacaagagcgaaactcccagctcaaaaaaaaaaaaaaaaaaaaattcacaagtacagaaagagatgctgaagaaggtaacagttacctagaaccccacccccagagataaccaccttgtggtaacatttatttctctgccgtagccactcttgtctgaaggagggttcatagtagataggctgtttttgttcatttgcctttaaaaatatatatattgtaaatattcttctgtgccattgaatataaaacatggtaatttttaaatttgtgtggtgtgcatgtgtgtgcacttttgggaaacttgtttatagtgactttcaaactgagcatttacaaagaaattaacagttgttgggtgtgttgaatgtgcagggttttgctgaacactttacaggggtgtctgatcgagtccatcacttcctgtgggcttgtgcaatagcctccttactgatactcctgctttcagtcttcctcctctgctagttatttttcatatgaaaacctgaataatctggctgggcgtggtggctcacacctgtaatcccagcactttgggaggctgaggcaggtggatcacaaagtcaggagatcgagaccatcctggctaacacggtgaaaccccttctctactaaaaatacaaaaaattggccgggtgtggtagcgggtgcctgtagtcccagctactcgggaggctgaggcaggagagtggcatgaacccgggaggtgcagctttcagtgagccaagatggcgccactgcactccagcctggtgacagagcgagactccgtctcaaaaaaaaaaaaaaaaaaagaaaaggaaacctgaatagtctttcaggaatgcaaatgagatcatgttgctcctctgcttaaaacctaatagcttctccttccatgtcacaaaaaaagccaagcatataaccaagatctggcctaggtcccagcatcgcttcatgtatcattggcccatctttctgtttcttcagtatgacatttgtttcagcctcagggcctttgcacttctttctggttcccctgccctgggacatttggataattgctttttttttttttcatttcaggttctagttcaaattgaatccaagtgaagtgaccccataatacatgttaattgtggaaaaaaatttaaatttagcaaagtaaagaatagagcatgtcactctaccatccactcaacatttttgtggggtttttttcatttaattaattccatttattcattctcttaacacaatgcctacaatatgccaggtatattatattggtgttaggttgggctataatattaaaaaggacagtcatggttcttgcccttgaggtctgttagatcaggaattcagaagtgggttagctgagtggttctagcttgtggtctctcatgagattgtagacaagatttcagctgggacttcagagtcatctgaaggcttaactggggctggcaggcctgcctccaagatggctcactcacagggctggcgagcagtgctggcagttgacaggaggccacagttccttgccacacggacctctccacatgcttcttgcgtgtcctcacaacatgtcagcagctttccccagagcaagtaatccaagagatcacaaggcagaagtgacatgtctttataatcacagatgctaccctgctgttctgcagtatcctgttggttccccagtctaccctattcagtgagggagggcactcactcagcaaatgtgccgggaaatcagtgggggcattttggaggcttgccactcgctgcctgtaaaatgagcatcataatggcacgtgtaccgctaccaccccctgccagcacaaggggaacatgaacctaacataatgggggcagggaacgggcagaagaggcttcccagaggagacacttaggcagagactgggccgctgagtgggcgtttgggaggtgagggtgttccaggctgaggggaggtttgtaggaaggtcctgagtgggaaggcactgcctgcagtagcgcatggcctggaggagacagcaaggcgggccagggtcagagaggccaggacacacacatcactgtgtccttgagggagatctttcttctctaggaatatagctgagcttaccccagaaaccaggggagaaaataggagccgagttttctggagtgcgtttcttctgtgaagtgaggtttgtgtgtaggaggcatctgtccagagcttttcaagttttatttcattattgctggagggaactagctctggtcctgttggttgggactgaactgtattgctgaccctttcccatgttcaaagttcccgcttccattgggggactgtgctttgtgcttcttcttgtaacaatgtgtttagcttatttagcagcatcagattctccttctgatatatgcattcgataaacctggacacctgtgcagatttctttttcgtggtggcactgtgttttcttttgcttgttatgcgtaaggtcagatatgttgtgttttgggtccctgacaccttgggcttggatgaataatgtcacttaagaggaggcaagtaaaaggccaggcacagtggctcatgcctgtaatcccagcactttgggaggccagggcaggtggatcacgaggtcaggagttcgagatcagcctggctaacatggtgaaaccctgtctctactaaaaatacaaaaattagctgggcgtggtggcgcatgcctgtaatcccagctaattgggaggctgaggtgggagaatcacttgaacctgggaggtggaggttgcagtgagccaagattgtgccactgtactccagtctgggtgacagagcaagactgtctcaaaaaaaaaaaaaaagaggatacaagggatacaagtagaatttgtagtgtgctgattaaccaaagacaagttcctccacccttttctttttggccagagttgatcattttcagaattcatcattttgtcaagatgatttttttgttgttaaatatgaataatttgctttcctctggacttctaaggcttcctgaaattacatgcaaacatttgtgcagtctcatgtttggttattggtttttgggtttgctatttttgggcgaggaggtccatatccttcatcagcttctcaaggggttttttcagaggtacaaggggaggctttggtttggttatgacagtgctacagccagcaacccgggggccacctgggtgctgctcccccacttcaaaacgtgtagctagcaggatggaaatcctgtctacatggaaatccatgtggtgttggataggccatgattcatttccctaagcctcaaatgcttctattgtttgtagtttttctcccagaatcttcatgatccatttttgtacattcttatggccttacgataaattcctagaagtggaatttctacatcaaaagaatagaaacttttaaaggtttttgatacatattgccagttgcccttctggaaggtctactgggtacgtcagtgtacctgagtgttaacagtgacggatcagtattcatttctcttataaggaaggaaatgaaagtcatttggtaacgtagaggcacaattagacctgacagcctttgtgtttctcttctgttctttaggccccccagttccctttgctgctttcttctttatgccacagatttaatgcttgaacacatattgaaattttggaaagttactgtgaatctaatggggcataataggcaggttttcttaatcctggcaatgaccaaactaatcacttgtctgtggtggcttggtggaaaaacggtttgtcagcagaatttggtaaagaagcagtcacaaggacagggtgttggtctcatatttgagtgcttccctgaggaaagaaaagataaagggaagaattgggtgaattcatcagactgtatttggcagatggagatgaagtgggtgcaggtcatcgcccacgacctgtttcccaggcttgcagagaaactgctgctcaggagcttgtgactgtgagggccccgggccgtggcatgcgttggtgcgctctcaagaatgcggccatggcactcacagacacataccaagaagcctcggcccccagtgcccccgccagcctgctcaggggcatgcggatgactggagcctggaaggcgggtcttgctgggcaggacagatgccttactgtcaggacagatgccttactgtaggcccaggaagagatccatgaccgcagacagacttctgcgtagggccctgaggaaagagtggtaaacatgcagtgaagggcggccccaccactggtggcttctgacagggagctggagggtgcaggtactggatgtgtctcattgggatacaaatgagtgtgccccgtggttaggaagatgaggaagtgtaggcacttgcaggggccttttcttttgacttagtgagttcccaccaaacctggccttgtctgtttttgatgccttaggacttggggacaaggccacagcctgtgaccccagcatcatctccccccagggccttgccaccctctagctttcatccttgcctcctcctctgccctctctttcttgtccgatacagtcacaagtgcctagaataaacctcacaccacccactgctctgctgtcagggctaccaccccggccccaccctgccttgccccggctctgatctcaaagacttcccagcctcctgttgccatctgggtctgtcctcctcctgctagcagagagaccctcccttagaaacttacatcagatcttttcactacccagtttcctgtccctcgatgggtacccatctcagttagagtaatgttcagcttctctccacagcctgcgtggtctgggcctggtttccctctcgaatttccctcctgtcactccctttgtttactgccagtgctttttcctcttagggttccctgggccctgcccttcactcagcttctggtgcctggctctttcagacccatgcaggccccagctcacatgacatcttttcggaaagaccttccctgatggcccaggccacagtacccacaccagcatcagctctttgtcctcttccccttttcatttctttgcagctcatgccatctgaaactacctcattcaattattgatagatctgtttggaattccaggagtccctttgcgatcccattcttctaaagattcacatggcctcagaatgccatgttacagtggagagtctgacttcttgttttctgagacggagtctcactctgttgtccaggctggactgcagtgacacaatctctgctcactataacctccgcctcccgggttcaagcgattcttgtgcctcagcctcccgagtagctggaattacaggtgcctgccaccacgtctggctaatttttgtatttttagtagagatggggtttcaacatgttagccaggctggtctcgaactcctgacctcaggtgatccacccgcctgggccctccaaagtgctgggattacaggcaggagccactgtgcccggcctgacctcatatttgaataccgagttttagttctggaggagctgcaggttttatgaaaagggaacacatttgattcctcagagcagccacaggccagctctctgaagtaaagtgcacgtgtgcatgtgtgtgcacactcacacacacgtacacacacattcacaaataggacatctcttttaaacagaaatggccacctgcatttgagaaaataaagtttcatgcagaagaaaatgacatgttaaattcaatcatcaagatttagactggtgggaattctgcacaacaaatgacttggtttaattaacatggaaattgcgaggaaaaaaaatgaagtggaacctatggatttaaaaattaggaaattttaagatttccatcgtaatttttttaaaacaatatattttacttccaaaaccctgcgttttcacatggtagctatctgctggagctgagtagccgctgctctcttgaacagcatcacccagatgggagagcccccttccccccaacccccatacactcctatgtgtacaacttcctgaaccctgtaagcattagagcttgcagcctctgctttttctgtttccttcttgatgggaagactggcagcaggatttacttggttgctacatttgtgaatttgtaaaataattcatgctctgctaggtctgtaacttgggaggcttggtgtgcacgggcatttagcagcaactcagagcatatggaagactgtcactggcaagagcaaagtccccccaggacagagccagtgacgactagctgtgtatcctcagtctgatggcggtggaagtgaggcagcaccaaggagcagaaacaggaagtttccactgatgaccaccctgcccccagctaggctgaaaggcctccccagagcccttgcatcagcctggctttgcactggtctgggggatgttgcttgttagagccagtgaagaagaacggtagtaagttacctgatggccaaggctctgtctgaccctgtctgctgtcgtgttcctggcacagaatagtctttgttgaaggaacgaattagtgcatccttccaagccttggaggacctgtctataataggcccactctatagggtctttgtgagaattaaattaaaacccctatgagaaacctaactagagacaattggaagtaacttaaatatttgttcattgggaacagctacataattgtggctgtcattctgtacaacactctgtggctgttaaagagctagaggtagttttatgtggattgatgtgttcaatgtgttcaatggaaaagcaagggtaatataatcccatttatactacagagaaaaatcgggtctgtaaatatgttgagaaaggtctgtcgatagtggttatcttttgagagtggaatggatcggggtgggtatggcctggggacgtgagggggaatttttcactctttatttcacatacatctgtcattggcacagaaaattaagcagtaaacctaaagaaacagaatagtgcttgttgtatagttagatcaataacttgtaactattataaaaggtagttataaagttagtaagggccaaaggtctaactagagtaggtcggttatagaggaaaacagtttaatcagttgttgtttaacttttatggaatgcaacctctttagctttaatttggagagccaaactatggccctagtctttttttttttttttttttttttttttttttttttttttgagttggagtttcgctcttgtccaggctggagtgcaatggtgctatcttggcttactacagcctccacctcccgggttcaagcgattctcctgcctcagcctgccaggtagctgggattacaggtgtgcaccaccatgactggctaattttgtatatatatattttaagtacaaatggggtttcaccgtgttggccaggctggtctcaaactcctgacctcaggtgatctacccaccttggcctcccaaggtgctgggattacaggtgtgagccaccgtccccggcccctagtcttttattgtattgtattgtattattttttagtcaggtttattgaggtataatttacatatcataatattccccttctttattatacagttctatggactttgacaaatacatacacttgtgaaattgccaccccttttgagatacagaacagttctatcaccccctagaattcccttgtgcggcccttttgtagtcatcctttctctcttctcccagctgctggcaaccctgatctgtttttttgtccctgtagttttgccttttccagaatgtcatatcaatggaatagtacagtctgaagcctttgaatctggcttctttcattcaatataatgggtgaggagtcaaccacgttgttgcatgttatccacatttcctccttttgtgtctctgagtagtattctcttgcatagatgtaccacagtttgtttatccattcaccagctgaaggacagtgctccagggtcctagagcacagaactctggctttgttgtctttatttctaccagttgtctctctctctctcttttttttttaaaccctagaagattattaagatttataagactgggtatggtggctcatgccagtaatcccaatgctttgagaggccaaggcgggaggatcacttgaagctgggagttcaagaccagcttgggcaatgtagcaagaccccatctctacaaaaaattgaaaaattagccgggtgtggtggtgcacacctgtagtcccagctactcaagaggctgaggcaggaggatcacctgagcccaggagtttgaggtgatagtgagctatgactgcaccactgcactccagcctgggccacagcataagcacttgtctccaaaaatgtttaaaagattgacaatacagtcttcttcagagtctccataggaaaggagcggcacgaaatgcaaattatttggaggttttggaggtttcaaacttttaattatttggcacatatagtgcttactgtgtgcaggcactgttctaaatattgctttcaaatatttaaaagtgcttagaacagttacagcacatagtaaatgctatatatctgcttgttaaataaataaaaatttaagtttccaaataatctgtatttcacataaaagagaagagatgtgggacaatataaataggcaggagaccagggttgtagacccggtactatcacattcccagcctaccccttaacctagtcccttgggtgaattaccgactctgggtctcacttactaacatgaaaggaggttcataatctgaatcctcctgaaggaacagataatatctcaactcttaatagttgaactctaaaatttggtcagtataaaagtaatgttataaaatgtgtctatatctgtttattttacattgtattgggcctggataattggtttcttcctttttacatgtatataacatcctattgggatctgtattaaaagtgtactaaaaacattcaccacatggtggtgctcccttcaaaagccaaactgaaaattgtaggccagcattgagtattaggcatggagttgataggggcagctgtatgtatgtatgtatgtgtgtgtgtgtatgtatgtatgtatgtatgtatgtatgtagagatggggcctcactatgttgcccaggctggtcttgaactcttggcctcaagtgatcttcccacctcagccttctaagtagagtgccagtttatattctacatttgtgctttaagttttttttagggaagtagggtcctgtcattttattagcttgataacttatacagatgccaaaatacaggaacatttgttctttcttaggcattatgacatattcatgtacattaactgatgttatactttttaagtgttccaaatatcttcactcagaagtttatgtgcttgacaggaaaagaaaaaatacatctgtaaggaaagtatcataggtatttatccttcaaaagctgatgtttttatttatttatttatttttaacctaatgtgttcttaagtcatactgggatagcagcagtacccagcctaagagaagctgcagtatagtttccttggtcaaatgactttttctttctttctttctttctttctttctttcttttttttttttttttttgagacagagtcttactctgtcgcccaggctggagtgcagtggcagaatcttggctcactgcaacctcctcctcctgggctcaagcaatcctcccacctcagcctcctgagtagctgggactacaggcacgtgccaccacgcccagctaagttttgtattttcagtagagatggggtttcgccatgttgaccaggctggtctcaaactcctggcctcaggtgagccgccagccttggcctcccaaagtgctgggattacaggcatgagccactgcgcccagccaaaagttggtgtttttaaaaaatgcttcctggtaactgccttagggagaataatgttaacatttcagttgtgattctcttgaagcacagtatttccctgccttttagatttgaaatggatacttctaagcagttgtgactggctggatttcagtcatttacatcggaacactggtctggtcagctcacctgcatctttggtagagagatatctcccaaacatacactctccctgaaggattttcatccttcatatgcttatcaattcccttgccaagtatttactgtttgtccacatgagtacaaggcattgagcttgtgctactgtagactcacagatggtcatgattttcaggaattgaatagagaagatgaaacactgagacactggattcaaatgctagaccttactgggttgacgttagtaatagacatgtgaagaattatagcggttgagaggaaagagacatctcctcactagggtgactggtcagggaaaaagatgggagtggtttttggtgggagaagaggaggagacgggatctgggcatatgaagaggcctggggtactgaggtggaatttcaccacaccccaaatctgttgaaaagaggaaagtgtacaggcaggagacacagaatctggccagagtgaatgtcctgagcaagggcatgggaagaggaaaacgcagggcacagggattaggtgaggatccaactgaatgcttgcccaaggggcttcactgtcgaggattttgactgagatgggggcaaacatgatagacaaactttagggacaatttagcattgtcttcaaacacaggtatgagggagacttttgctggtgataggacagattatcctgaaaattgacctgacaaaaatacttagacctgatccctaaaatataataaacatctttttaatgaatagctgaacttgcaagaaaaaaggtaaatccccaaggcctataaaataaaagatgagctggccgggtgcagcggctcacacctgtaatcccagcactttgggaggccaaggcgggtggatcacctgaggtcaggagttcaagaccagcctgaccagcatggagaaaccccatctctactgaaaatacaaaattagccgggcatggtggcacatgcctgtaatcctgctactcgggaggctgaagcaggagaatcacttgaacctgggaagtggaggttgcagtgagctgagatcgtgccattgcactccagcctgggcaacaagagtgaaactccatctcgaatttaaaaaaaaatttaaaaaataaataaaaaataaaagatgagctgaaaataagaaagacaagccaaaactgtaaacgtcttggcattgtttgctaatttcagtaatcaagatgcttttttcccccaatgttttgtttttgttgctattgttttgaaatagggtcttgctctatcgtccaggctggagtgtagtggtgcaatcatggctcactgaagccttgacctcctgggctcaagtgatcctcccacctcagcctcctgagtaactgggactataggtgtgggccatcatgcctggctaactcttttttttttttttttttttcattttgtagagatggggttttggggttttaccatgttgcctaggctggtcttaaactcatgggctcaagtgtccttctgtttcagcctcccaaaatgctgggattacagacatgagccattgtgcccggctccccaatagttttattgaggtataactgacataaaataaactgcacatatataaagtatacaatttgataaattatatgtatatgcccacaaaacgatcaccacaattaagatagtgaaaagcccatcatcctcagaagtttccttatgattctttgtaattcttccctgatttacctccttcccggtccaatacttacctgttttctgtcaccataaattagttttcatttatataaaattttagaaaatacagtcatatactatgtactcttctttgcctgacataattatcttgagattcatccatgtttttggatcaataatttgttcctttttattgctgagtactattccattgtgtggatggaccataatttgtttattcatctgctgatgggcatttgtttccctttttgggctaatacaaataaagctgctagaacacatatgaacatatcttttttacttttattttttgcctttttcctgcagtatgagcaaagctttgtgtggacatttgctttcttttcctttgggtaaataggagcaggatcgctggtcatatggtagctgtcgatgacacttgagtcttaagggctgctgtttggggaactggagacataatcttgggcctatgagtagacagggacttggaattcagactgccctataaagctaagatcattgattggctacactttgagcaaaatgatagactagaaagaataagctgttggcagaatatttaaaaaagaaacttgccaggcacggtggctcatgcctgtgattctagcactttggaaggctgaggtgggcggattgcctgagctcaggagttcgtgaccagactgggcaacatggagaaacctcatctgttaaaaaaacaaaaacaaaaagcaaacaaacaaacaaaattagccaggcatggtggcgtgcatctatagtcccagctacttgaggggctgaggctgaagtatctcttgaacccaggaggttgaagccgaagctgagatggcaccactgcactccatcctgggtgacaaagtgagaccctatctcaaaaaagaaagaaagaaaggaagttagaaagtgggggagggagggaaggaggaagtgaggaaggaaagaaaggaaagaaaacaaagagaaagaaacttgtctgatttggtctgcactttgagtgagaggaaacaaaaacctcccgagataacttttattctaagcatgccttcttttaaactttgtttgaatttacctggcctctgtagtttgtgaaattccaagaagagacattattttagagagatactaggttgctagagttcctagattactacagttcctagttagctggcagaagtcaatgcatatcctcttggactatatctatctttttctcagtcttaacaccagattcccaaagataaagcttctccaaacatgatctcacaatccaaaactaagaacatgagaaaacaaacaaccttgcatcacagagcaggaaaatgaacagtagaactatagtactttatagctttagatataaaaactgtcagattcagaatataaaatactggtttaaaaacatttaaagaaataaaatgtgaaatagaaaacaagtaaggactaaaatcctatgaagaaaaatcaaataattgaaaaagaactaaaaaagaaatgaaaactacgatcagtgaaattaaaacttcagtggatgggtttaacaagttagacacaactgaagagagatttagtaaactgagggataaagctgaagaaattatacaaaacgcagcatagagagacagaagtctaaaatataagcctataaggagagagaaaagaagtcaatagagataacagatgagagacaatatttgaggagatattgctaaataatttccaagaatagtgaaaaacaagaatctttagattcaggaatcagagcaaatcccacgtggaattaaaaaaaaaaagtcttctccaaatataaggccaatagaacaccaaagacaaaaataagatcttaaaagcaatcagagagaaactgattacctcccaaggaaccctattaaactcaaaggagacttctctacagcaacgatggaaaccagaaagaagacagtggaacagtatcttaaaagcgctgagagaaaaattattgtcaacctagaattttaaacttagctaaaatataatttagtaatgagagcatgataatgacattttcagataaacaaaaactgatgtctccagcacggtctcacaaaggaacttttatactttcaaaaaagagaaaatgatccaaaaaggaagaatgtctgcaatgcaagaaagaatagtgagggaaaagaaaaagtggaatgaatagagaattagtcatgtggtatcacatggcagctcactcaggaatcataaagctggccttgggataacagagctaaactttagagtcctgagtcctgttaatactcaatcatctgtgaaattcaattaagtgagcttcaagttaacctaaaaagctgtggtgaggctgggcacggtggctcatgcctgtaatcccagcactttgggaggccaaggcaggcagatcacctgacgtcaggcattcgagaccagcctggccaacatggcgaaaccccgtctctactaaagatacaaaaattatctgggcgtggtggctacttgggaggctgaggcaggagaatcacctgaacctgggaggcggaggttgcagtgaccagagatcatgctactgtactctagcctgggcgacaaagtgagactctatctcaaaaaaaaaaaagcagcagctgtggtgactcttttcttgaggtctttgggggctgcctgttggtggacaggctggtgtgaagttggtagccctggaggagctggggggagttgcagggctagtgtagacaagctacagaagccacaagggaggtgctgcttagagggggctctttattctttgtttggttttaatttgagacgggttcttcctatgttgcccagcctggtcccaaacccctgggctcaagcgatccttctgtcgcggcctcccagagcgctggggatacaggtgtgagccaccatgcctggcctctttactcttattaatttaatgctggttttcctagatctttgtctttttttctggattttgggagatttctttccttgagtatttttcacttattttctattaattttttattttggcagtcatactttttaactaccacagctcttatttaaaaaatccttctcctagtatcacattcttgatttctgggcatataatctttatgggtctctctgaggatatgagttacggttttttgtagtttggattatctccagtttcctgaattatctgtttccttcaggataatctgttcatcttggtctttttctgtgatgctctaggctttcctcagcagtctggtaatcctggttgtccattcatgcttaagaacatgggaatggaaggggtgttgggagtcctatatatgtggatggggttgtctattggctggtttcagtattgcactaatgagtagaggaatcaaggaacctctcagggctttgtgttgggacgctgacacactgcattagtaccttctagactatgagcaggggaatcgaggaacctctcagggctttgtgttgggacactgactcactgcattagtaccttctagactatgagcaggggaatcgaggaacctctcagggctttgtgttgggacgctgacacactgcattagtactttctagactgtgagcaggggaatcgaggaacctctcagggctttgtgttgggacgctgacacactgcattagtactttgtagactgtgagcaggggaatcgaggaacctctcagggctttgtgttgggacgctgacacactgcattagtactttgtagactgtgagcaggggaatcgaggaacctctcagggctttgtgttgggacgctgacacactgcattagtactttctagactgtgagcagaggaatcgaggaacctctcagggctttgtgttgggacactgactcactgcattagtactttctagactgtgagcaggggaatcgaggaacctctcagggctttgtgttgggacgctgacacactgcattagtactttctagactgtgagcaggggaatcgaggaacctctcagggctttgtgttgggacgctgacacactgcattagtactttctagactgtgagcaggggaatcgaggaacctctcagggctttgtgttgggacgctgacacactgcattagtactttctagactgtgagcagaggaatcgaggaacctctcagggctttgtgttgggacactgactcactgcattagtactttctagactgtgagcaggggaatcgaggaacctctcagggctttgtgttgggacactgactcactgcattagtactttctagactgtgagcaggggaattgaggaacctctcagggctttgtgttgggacactgacacactgcattaatactttccaaactttatgttcttcagagaagacccctccttgctgggggtgaggaggtggagaagtgggtcaggcgtgtgccttggctggctgccgcttcatatacagacgtatgatccctggttttcccccgccctctgtgtctcactcccttcctccactgcacttgccatcttcatgtttggggctcttctgggcagatgggcttgatcctcacctgtgaattcctctgctctcctttgccaagcaatgcttgcccatccactttcagatcccccagtttgttgaaatatctagtatgatgacagcttctctgttctcaccattgtcgtggtttataccttttttactccttggctgtaatttaaaggggtcacaggcaggagggggatgagtgcatgtgctcagtccaccatcttgaccgggagccccagaggcatcatttcaattcctgtgatattatggattcctacgggtaggaaaaacacagcccattcaaccaaatatactttaacccctagagatttagctttaacttgtttagaattgtttaaaagtcccttgtattttgcagttttttcattttctccttgaaagtaaaaacatttgtggcaaatagggaagaaaaactttccagttaatcgagaattaggataagtgagatttaaatattatcagatactgataagaactatggcttttaaagaatgtcgtcttagaatcagtttctaattacttgtgtgcagaagagtcctgcagctgtgaggtgatcacagtctttggcctaagccgctgccaggtgagtgaaagccaatctggagtcacagagtggcagcgactgcaccggagatgtgtgtgccatttgttaagatgagtcaaatggtagttagggcaacgaagatccacagagggagaaagaaagatactggaaaagcagcagcacagtttaataacagtcatcgttcatgatggcaaggttgtttactataaaaattccatccttcttgcctctgtgctgccccccaccatttttttatttgacattagggcttgctgatttatggcataacgcagtacatttcacctctgaaacaaagtctgtaaaatcttgagatatattaaagtctttattccccaacgctaaagacctcatactgtttagtcctctatacatttagccctttatgcttggggagggggaggttataaatttctagagggaactggattggcaatggtatgtttgatggtgaaatgccttgactaaacaaacaaggctgctccagaaacgcacacacagcaaacctatatgccatataagtaacgtgttatgtggggagttactttaggtttaaaacaaatgtcatactcttgatgcttttaggtagctattatcttggtaaggataagacagaaatatggtgaagttgcatctgattttgagggatactgcgggcaaacctgacagctagcttggttactagaggtttaattagttacagctgctctgccattgtattaatagagccactctgctttcaggcaccatggatgccttttataatttggatgttcttaaaaagagcactgtgtgaaagtgagcagccctgggccgggcgcggtggctcacgcctgtaatcccagcactttgggaggccgaggtggctggatcacgaggtcaggagttcaagaccagcctggccaagatggtgaaaccccttctctactaaaaactacaaaaaaatactccgggcgcagtggcaggcacccgtaatcccagctactctggaggctgaggcaggagaatcgcttgaacccaggcagcagaggttgcagtgagccaaggtcacaccactgcactccagcctgggcgacagagtgagactcagtctcaaaaaagaaattgaacagcccattttgtgaaccacttcaaaaaaaagcaaacacattttcctctggcttttggctgttttaggaagaagccatacggtgaaccaggtgatgctgaggttatctggatccaggccatgcagatgaagccatatttacctttgtgatattggggctgatcttggagctgtctggatctgaccagtctccagatgaaaactcttgcaactttcgtttttggatagtgctcacctcgtatctgtactcgtacctgctatttctaggcgaattgtcccctttctcctccctcttccctcatctccctctctcctctgcctggctgacaccaggaaggaggagttttcttttatttagataaaaaaaagttgagaggagggagctccagaaatgtgggatactcagcactggagacatttgggctggaattcttgtttccattcttttcttaccatatgaccaagtaagtccaagaaagtagattggattctgagtgggcagtgaaggtggaaatgtggtcctaaagagaacgggcaaattaagaaaagattgttttaagacagtcaaattgttttgcctgttgaagaaggtgatcagaccctaatgaaactgaaaatgaggagagtgttcccatctcctgcctggtcctagcgactctgcaaatgggtgcctgattggtctgttggctctgaagccagcctttgctggatatattcagcctgttttgaagttgtgcagagaacctcacttgcgtcattctgaagacgcagtgagtcaacgcagtcccaagagagcagtaatggccccaaacagaaacttggaatgaaaaatagccatggatttaaagacatagcacattcttcctatgacttcatttggtaatggtaagattaattcacagaaaacccttcttgagtggcgtaccttaaacacatgtagaatgatttttttctttgcttttcccatttagccttttgaaacaggatacacagtagggtgattggtttgggagggcactggtacagtaattctccacctctcacttgcccgtgtgggtgccccatccccaccctcaggcacacacgcactcttagctgcttttggactcctcccgcaatgtcacaatagttttctttgaacattcttgaccctcagtcatgttgacatgcgtttggattttcagtggagaagaattgccagagaagaatcttcctctgattttaaccattgaccatatttatatatgcagtttcagcttgacttttaaattgataatcttttaatagaattccagataacatcttactgtaacaaacaccaaggggattatccaaattcctatttgaaaatatgtcttttatattaccagatttgccagctgcattattatctattagtgtgtactaaaagtatattattttggcttattttgagattagataattcccagtggaattctccccttaaccatctaaatctgtattttttttttccccatttagtttcctaaacagtgaggcttctgggcaggaaatgagagaagaggaggaggtaatatagaataatgcagtggctttcaagtattgtgacccgtatgaggaatacatattcagttatgacttagcattcacatatgcacacatacatgtacgtatatatatcacattcacacatatgcatatatgtacatatacagctgaagaaggtctggattagtacttttccttattgtggagcacagtgagtgatattttctttttctttttctttttttttttgagacagtcttactctgttgcccaggctggagtgcagtggtgtgatctcggcttactgcaacctccaccttccaggttcaagcagttctcctgtctcagcctcccaagtagctgggactacaggcgtgcgccaccatgcctggccaatttttttgtatttttagtagagacggggttttgctatgttggtcaggctggtctcaaactcctgacctcaagtgatccgcctgccttggcctcccaaagtgctgggattacaggcgtgagccactgtacctggccgatattttctattttatttcattttgaaaaagataggctgtgactcattagtagtggatctcatgactaagaatggatcctgacccaagtttgaagagactggtaggggtaaatttagagcctggggctccaaagtttgtctacccagttttaaatcctggctttccccttaacttgggtgggatcacaccattaaccgtgttacccctctgaagctttggctcccacacctgtgagatgtgaatgttgataacacacacccacctcataggattaatgagaacatgccaagatataatgcgctgaaggtcttagcatgcctgcgcagagccccagcatctgttagctgctgctgctgccgctgtggtggtgactgtccttgctaagatgctgcagctggattggcttcgtgggaagttgtggaattctgttccctgaggatgttgggaaggacagattgtacttaccaagagcatttattgttgtttttattttcttaaacatttccaatgaaaatcatcaaacctataaagttgaaagaacaatgcacctagattcatcaactcttaacacttgctatctctcttacatagaaacatttcccttttaccagtccacttggaaattggctatatactcacgatagccaagaacaagaacactctcttacaccatcacatcattgccacacttaaggaaatccacactgatccaggaacattatttgatatacagtccatattcagaatcctccaggtatcagtaatattttaattatgacccatttggtgaatttaagatggattagatggcctgtggagttattcatggagctgaagacttctgtgaagtaaaaaataaccacccagtgttaagtgtaactctcgtgtggaatattaaatcaattgtgtgttttttttggcatccttgatgtgaactctggagacctgatgagatggaggctgtgattgtttactctgtgttagcttggacacttagcttggcagtaatcacaagagctttagggagtgcatcctttgctagttcataaagatgtattctgataacgggggaccaaaaggatatatcctgaattgcaaagtcgagcagtagattacatttggatttgaatgtaagtggctgtgaattagaaatatttgttggaattagaaagtgtctaggtaggaatgtaaggtctcccctcaaattgagaatgacaaggctgtcttctaaggacagaatttaaggtgaacactgtggaagtttgtgcatgtgttttttgtttgtttgtttgtttgttttttgttttttttgtgacagagtctcgctctgtcgcccaggctggagtgcagtggcgcaatctccactcactgcaacctctgcctcctgggttcaagcgattctcctgcctcagcctcccgagtagctgggatgacaggcgggcatcaccacgcccagctaatttttgtatttttagtagagacggggtttcaccatgttggccaggctggtctcgaactcctgagctcaggtgatctgcccacctcggcctcccaaagtgctgggattgcagggattagccacagcacccagcttgtgcatgtgtgtttttaagaaaacgtccacaaggtaaggaaattcaagcaaccaagaaaagacgcttgataaacagtaagtcccatcttgctagtttcttctgtatttctccagggccactttaattgattctaaaatgtacattatttctcatttttaaaaaaaaatctctaaaatcagggtacatcttaaaagcaatataatgccatggtttaattggcacatgatttagtgatacataaaataaaggcacctcttgcagtggcatcttcgatttgaagaagtataatattctacgaatatacaaatttctgtgtttttttgtccccccaacccctgcccttttaaagacatatagtaatatagtggggttataggtttatatactgctacttagctgtgcagagaaattacagcatttaaaaaaatcaccaatctgtcttcctcataagtcatcatctagaaatggggagaagcaaagagtggtattttggccagttaataaggtcttatattcttttggcttaaacagtatcttttgggtaaattctggattttttcatatatcctgccatcccccattaaaaaccagcatctggtcttgggggattgtgagatttttgtggaggtgagggaggccctggcctatgcttgctgcctttgctcatctagtctggtctggtctggtccctgggcctttcgcaggtatcccctgaagtgtggttggtggtcttgaatttttttcttttgtctccatcagggccagggaactgtccttgcttccttttggtacattcaccctgcagcagatgtcatggcttccaagtggaacttcactctctttcttactagttaagctacaggaggcttagagtgctaaaaccgagatgcttcccctgcataaggccatgcaacacggccattttattctgtagccatccgtgttgggatgagtggaaggttgcatctgcgaggtggtcttctcctagagtttcaattaggaagtggggcaaaagccccagtgccttcccttcaacctgacgaccagtctaccctctccccacctgtgctagttatcaatttcttgcttgttatctccaaatccattctgctttgccatgtttcgtgacatgggaactggactctgtcaacagttttcctttgcctgctggcgaggtgttaggctttgtcaacagagtgctggagggacatggcaaggtcatggtgggaggagggcgtcctttcccagtgtgctgattttcactggtgagtgagtatcagtggactggcgtgcaagatgcccagaaacacatatcagccatcatagacagcccagtgggtggtaccgtgcaccagctccaaccacacacaccctgcagggagtttctccaccacgtggtgggctgctgccctgggccagctctggatcacgccctctgacaagcatgtttgccaccggcatgctgtgtgttcctgtggagctgtgccctttctgaagagtctgaatctcagctttggggttgggggaggctctcctaagttcttagttcctccctcttcactctacctgccctttttaagacacatagtaatatagtgggctctaagtagtagacactttgttcatttgctacttctgtacccctgggtcctcttttactcttctgtcatttgttaaaaatctcggccgggcgtggtggctcacacctgtaatcccagcacttcaggaggccaaggcgggcagatcacttgaggtcaggagttcgagagcaacctggccaacatggtgaaaccccgtctctactaaaaatacaaaaattagctgggcatggtggtgcatgcctgtaatcccacctactcaggaggctgaggcacaagaatcgcttgaacccgggagatggtggctgcagtgagctgagatcgtgccactgcactccagtctgggcgacattctggaactctgtctcaaaactaaaaaaaaaaaaaaaaaaaaaaaaaaaatctcctgtgggacttcagtctgtggaggttattgagtgatggcacagaaaggccaatcccaataaaagaaaatggaaaatgtttattacttccatttccaagaggggagcatgccacgccacaccacacaggcacatggggaagcaccatccacagggcagaaaggagctgggggaacgcccaggccagagcctttgttgggcttctgtgggaaaggccagacagggccagggaaacatctgaggattggctattttggataattctggggggccctggggcagagggccgtccctcgttgtctggttcctagctctgggtgatttagggtaggagaaatattggctctgtgtgtgagagttagataaggaggtggttcagagaatgggctctgggtggcaggggagacggaaacagctttggctgtgtgtgagtttgaccctgtgattagactaatggatgccaaatagatgaatacagaatctcagaaaacacagaacgctctcttagcagtatctactttttgttaataattcttttattaaattttccctattgaaatgactggtgtggtttctgtctcctgactggtacatcacctcttcctcggaatttgcgggcagggaagtgatgatacatgtttgactgcctcctactctttgcaccctgatgtgagggaagggctggacccttctacatctttctgtctggatgaagctcctctgctgtcatttcctcctccttccctagtgcggcaagcagctctgccagcttgtcatagaagggcatttaagtgactttgccaacacaaacagtactgcaatgaagatatgccacactttgcaattagttattcactttaaagttctgttatgatatagtaacttaataagtgaaaaaaacatcttggaccaataaggatggaagaaaagtatcggaaaactagtcagaattaaaataaggactaaatcacgacttttatttctgtgatttctttttgtatttttgaagctcttttcttaggtcagggccaccatggctttttgttgcattgatctctttatcattatatgctgtttctccttaggctctgcaatattccttgctctgagtctactttgtctgataggcacttcagctttcttttgatcacgcttgcataatacaccttttcccatccttttactcgtagcctgcccgtgtcattgccccagtggggaactgctgttgctctttacttggagccaggctcatggtaagaggatggggactttcttggttctcttagtctgactccatcttaggcaggtactgtgtgcctggacttcaggatagggctttcttagcattgtgtgctttcaccctccatgccacctggactctgccttctgtgtgtgtgtttgtgtgtgtgtgtggtgtgagctcccgtgtgagagagaatttcccacgtttccccccaaccccacccgaagctgacttttgcattgtatcagtgcagaatccagcagacgatcatatttgctggtacctcacccccaggagcagcagatctttgcctgggtcccggggacagggaaggtttcttgcccttcccccagtggattacggcttttgcattaggtctgagagacgggctcaggaaggaggcaagattttacccgagtccggtattgaggggtgctctctccagcctcgtgctctgctcccagtcgtcgtcacgagcacctggtagtggcccatggaaaagggtttgcaagtgagttcagacaggaattctagtgttacaccagcccatgctcagctccataagaattcattaaaaattgagatgttttcccgtcacctgttgacatggcagcctcatcttcctcctgtgctctgtgaagggtcacagggtttgcgtgtcccatttctccttggagggatttgtcactgattagaattcagttcacctgatggccttgtggcctcagctctctgattagctcaagaaaagttaggattttgttgattatctggctttttctttttgttgggttgaaagttctcttatggctttctgcatcttaagcaaggggagtagaactctatttcttcacctgtccctcagcagaattatgtaagtaaaataaaatttaggttcctcacagatcagtgcagtttgctaatacaaatactgtatgtatagttactctgttttccacatccaccattggtttaagtttgaacacccctgttttactttgtattttgaaataatttcaaacttacagaaaatttacaagaatagtacagagaattcctacatgtcctttacttagttcgagtcatcaatttttaacgtattgctacattacatttgctttaccatttccccccttctatatgtgtatgggtataaaatttgtttttcggaatcatttgggagtaggtcacaacattttgtccttttatcccttaatatttcaagtgtatgttgtaagaacaaggatcttctcttatgtaactatagtataattattaactttaggaaatttaactttgatagaatatttttatttaacctaaaatccgtattccaatttcctcaattctcccagtaatgtcctttctagcaattacccccttgggtgtaggatccagtcctggatcatggattgcattaatttgtcatgatctttaatatcctgtaagctggaacagttcctcagtctctctgccttgcatgacattggtatttttcaaggacatggagcagttattgtatagaatgtttttcaattttggctggaacatttcagtttcagtttgtttgatgtttccttactattagattcaagttacacatttctgttttagaatattacagaagtaatgctgtatctttctcatggtgttacatccatttgcataccttgtctttctgcctgtcgttaatgatattaattttgattatttagtcaaggtactgtctggttccttcattggatagttgctagttttcctcttgcatctatttgcttttcggtttttgttttttcccttaactttttctccctgtgatttcctgaaacctcttgcatctaaaaagcaatctgtggggagacattttgtgaccatataagtaacctgctcctcatgaaacataaaatacaaaccttgggttctcttagagtggagaaagggatcagtgatccaagaccgtttctcataaagctaatacctcagagaggctacaccatcagagagaaaatgtacgggggagaagcacattacacagtatcaatcagaaaggaatatttctgtctgagctttcactttgagtggagggcaaagaaaaaaaatcacatgagaacttgtggctgctgaccagctgctcccacatgggtgtagaaactggttttatcctatctgtgtgacctccaatagctgcaagttggaaatcttgatttagagtggacctaggtttttaccatccctgggtgcttgacaaaagcaagtttaagtcttccctaactcagagtttccatagatcattgcagccaatatgaacacaccaaaaaaggacatacacacacacacacacacacaccctgaaacaagatatcatgcgcaagagtcagtagaaacaatagttgttcctgacaatttcagatattggaaatattgaatatagactataagttaatttactacctttggggaagcaaaagaaggaattgaaaatatgaggaaagagagagatacatcaaaaacaaccaggcagttttatttttaaaaatcaaatataatgttcagaagtaaaaagcataatcattgagataaaaaatttatggattggttaaatgttagaatagaaacagcagaaaccagaattagtgaactagaagataagtctgaagaaataacacagactgaagctaatagaaacaaagggatgtaaaccacgagaggctcagagatatagtgagaaggtccaacttatgtctaattggagttccagaagaagatactacagggaatggcaaagagagaatattgaaacagataatgagtgagaatcttcacaattgatgaacaacaggcctttgtctgtcatttgtggaagctagcacaacagtttaaacggaggcccataggccatgtctaaatatttaaaagttacaaatgtgacagactgtgaaataaaatatgtctatactcctaccttgacaaatatgtctctctgatactctagaagatgaggtttaaatgtagagttcttgaactccacagagctctatgctggcacatagcagcacagagtgagccagaccttcgcctgtggcccccacccttttgtctttcttcccgcagctttatccatgctgtgaggggcctcatgcacacatgtgtacatacttcagcctgcatatctaagctgtgttcacgctcctcacaagcatgcttgtaggtggcaactctggcctatgcccgtatgctggtgcattctactttctttcatttttattttatttatttatttatttatttatttatttatttatttagagacagggtttcattctgttggccaggctggagtgcagtggtctgatcatagctcattacagccttgaacttctggactcatgcagtcctcctgagtagctgggactacattaattaccacacctagtattttatttttatttttattttttgtagcaacagggtctcgctgtgctgcccaggctgggtttgaactcatggcctcaaacactctttctgcctcagcgtcccaaagtgctgggattacaagcatgagccactgtgtcgggccagcattccactttgataatagacctgtggaaaaggcccatgcaagtcctgaatgtgggcatggattcaattaagtagggaattcnnnnnnnnnnnnnnnnnnnnnnnnnnnnnnnnnnnnnnnnnnnnnnnnnnnnnnnnnnnnnnnnnnnnnnnnnnnnnnnnnnnnnnnnnnnnnnnnnnnngatccgccctcctcagcctcccaaagtgctgagattacaagtcaccacgcctggcttccgtatttaagtattaggtggtgactccatacaaaatatttaacagcttgctggttaacatttaaatctttgttgctaagaccttttctatgtttgacagttattccaaacacgttccatataggaatagtttgccaaatagaagaacacgggatattcttctcccatggctgatgtgttgtgattctaggtgcatatttctgtttccaagaacacggacctgttctcaagttcaaacactgcatcaagagactgtgccccatgtcttttcacttttttccctctctctttctctccccttcccctccttgatttaatttcttcagcaggtcagaattgatacagcttccagaagaaatagtagaagtaggcaaaagattagtttttaattcttgttctgtcaaatactttttgattgaaattgtttttattacaaaggtagcatttgctttttgaaaaacaaaataagaaaaatctttttaatcacttcactattaagtttgttgaatattccctcataactttttctcctggctttttgagtatttgagacatttctttccacattgcagttttgaaacattctaccccacactcatacatgaaagtgaaggctctgcttctcagagtacagtttaatttactttgtggacatcattaacaaaaggcagagaaagacattggaccatactaattgtgggacttagaaaagctatattagtgatggttattaagtatcgcttgcagtggagtctgtaacatattcctatgaagttaatctaactactgagatagtgggagtgcagaggaggcatgctgtgagatggagtggtattttccagcatggcttttctgtttcttgaaaaccctacagcactttgccatggtttctcatctggatgaaataaagcacctgtaccttagtatgtcctgccatgcctttgtatggcatacttggctttgttctccaggcctcttcccacagtaacaacggattctttaggaattggaagggggggccgggcatggtgactcacgcctgtaatcctgggactttgggaggctgaggcgggtggatcacgaggtcaggagtttgagaccaacctggccaatatggtgaaaccctgtctctactaaaaatacaaaaaagaattagctgggtgtggtggggcatgcctgtagtcccagctactcgggaggctgaggcagaagaattgcttgaacccaggaggcggaggttgcagtgagctaagatcgtgccactgcactccagcctgggtggcagagactccgtctcaaaaaaaaaaaaaaaaaagaattggaagggaatggaggaagcaaggtggttaaacaaaaatcatctttacacacaccacccactctatgatgtatatgagttcagaagagcactttgctttatccttaatagaaatatctgtaaagccaggggagtcataaagctgtaggctaagtaaggtgccatgagaaaaggaggcttcacttacgccagtatttggagcagcgtttggcctcttggaggtgtttgcacccatcggagatgctccatagtgagatttaggataagtgcaaggtgagctttgcttttgtaaaatgcatgaagtgtgaccacgaaagggccatgggaaagaattattgatgggttacaggtgcatcgtttcaggcagattgacactaggaaagagcaaagagcaggtagaggtttgacagtttactcctttaaagtaatccatgtccaataacccatggaaagtcttcatgtacttctaaggggtagacataccctagtctaggtgctaatctaggttctatcatgtgttagctgtgaccctgggcaaataactttatcctatggcctcaatttcatcttgcaaaaaaatacggattagataatggcacttccttaaaaggtttgatgggatttcaatggaatattgcatagaaagtgcttgaggcattgtaagtacacagtaagtgaagtgttgaccattattaatatcatgatgataaagtgtgtaacttattttataagtaccatataattgaaatttgccaatagtaactcctcggagacttccagggaactctgtcaatcaaaaaaagctttgtgtaataatggacgctaccttgacagagtgtgttagtcaagagaggatacttatttataaattttgggatatttatacttttttttttttctttagagatggagtcttgctctgtcgccaaggctagagtgcagtggcgcaatctcggctcactgcaacctctgcctccccagttcaagtgattctcctgcctcagccttccaagtagctaggactacaggcacctgtcaccaggcctggctaatttttgtattttttaggagagacggggtttcaccatcttggtcaggctggtctcgaactcctgacctcgtgatccacacgcctcagccttccaaagtgctgggattacagacgtgagccaccgcacccaactataaaatgtatttttatagatacttattgaattttaggatgtgggctgggtgattattttttaaagtacttttaaaaaaattaaggtattatttacatataatatccacccatttttaagtatacattttggtgaattactgtgtgtcaatcatgtaacctcaaacacagccaagattataaaacagttctctacgctgctttggtgatggatacaccaaaatctcagaaaccaccactacagaacttattcatgtaaccaaacaccatgtgttccccaaaaacctattgaaaaaaaaaaagaacccaaaaccaaaaaacagttctctcaacattaaaagttttcctgtgcctttttccagtggattccttccctcagcctctggccccagacaaacacttatccactttctgtgtctgtagttttgtcttttcaagaaattcctatgaatggaaccatataaaagttatataaaaatcatagacttttgtatttgatttcttttactcttagcatcatttttttgagatttactcctgttgtatgtatttacatttcctctttttcttggtgagtaatattgcattatatgaatatctcacaatttatccattttactagtggataacattagattgcttccaacttgaggctattatagtacagctgctatgaacatttgtgtattcaccattgtgtgagcatatgattttccctaccttcttttctatttcactttcttttcctttttctttccttttttttttttcttttttttgagacagtctctctgtgtcgcccaggctggagtgcagaggcacgatctcggctcactgcaacctctgcctgctgggttcaagcaattctcagcgtcagcctcccaagtagctgggattacaggggcccgccaccacacccagctaatttttgtatttttagtagagacggggtttcaccctgttgaccaggctggtcttgaatgcctggcctcagtgacccacctacctcagcctcccaaagtgctgggattataggcctgagccacagtgcccggccctttttcctttctttttttgagataggatcttgctcaatcatgcaggctggagtgcagtggcacacttggctcactgcaacctccacctcctgggttcaagcgagtctcctgcctcagcctcccgagcagctgggactacaggtgcgtgccaccacgcccagttaatttctgtgtttttagtagagacggggtttcaccatgttggccaggatggtctcgatctcttgacctcgtgatctgcctgcttcagcctcccaaagtgctgggatgacaggcgtgagccaccaagcccagctgacaatggattttctttgttttctccttcatctgaagatgtcttccctttgccttcatttttaaaggatattttctctgggtatagaattataatccgagagtatagaggttgacaagttttttggtattggttttagttttgggttgtgtctttttgttgttggcttttgttttgtttttgccccttatagatgtttcactgtcttttggctcatgtgttccgatgagaagtcagcccttcattgggtccttgttctcatctgtttaatacctgttcccatacctgccctttctctctcactgcttttaagatttgctctttatctttggttttggagtatttgactatgaagtgcaagctgctttgtttcttcttggtgtacattcagcatcttgcatcttcaagtatctgcgtatcattaagtttgggcagtttttggctcttgtttcttctaaattttttctaccccattctccctgtccctctccttttggtattgtagttacccactggaacacgtgacattatgtagcaagtctctgagtctgttcatttttttccttcagtcttttttttttttttttgaaatggtctctctctgttgcccaggctggatggtacagcggtgtgatcacgactcactgcaactttggcctcctgggtttaagccatcctcctgcctcagcctctttgagtagctgggaccacaggcacgtgccaccacgcctggctaattttttgatttttactagaaacagagtcttgccatgttgcccaggctggtcttgaactcctgggctcaagcaatccacctgccctggtctcccaaaatgctaggattacaggtgtcagccactatgccagccttttcaattttttatctctcttcttcatcttggttaatttctactcatcttttttgaaatgcacatactgtccttttctttgtccattcagctgagtatatccagtgaattttttatttcaaaaagttaatttttttcagttctagaattgccatttaattattttttgttgttcctatttcccccattgagatttcctacttcttagctgagattttcattcattggaaacatgccttatactgcttcattgagatgattataatagctgcttaaaatctttgtctattccagcattttgttgatctgcaggttagactggcagttgaactaatttgtcccactgtcttgcttctttgtatggtgggtagttctggattgtttactggactgtatgaatgtcaaattctggatattctggattctgttacttttctctaatacttgtttggttttatcaggtggttttcttggctgggtttgaacacaaatgtgtttctctctgagatctttagtctgtagctgagctgctttgtgtctgtcccatgcatgagtggctcaagggtcagtcagggatgtgattgtacggggattggagatcttcccctgcctttttcccttctaggattacttcagtctatttatttatttgtttatttatttagagacagaagtcttcctctgtcacccaggctggagtgcaatggcgcgatctcagctcactgcaacccctacctcccgggttcaagcgattctcctgcctcagcctcctgagtagctgggattacaggcccgcaccaccacgcccggctaatttttgtattcttagtagagaaggggttttgccatgttggccaggctggtcacgaactcgtgaactcatgctctacccgcctcagcctccccaagtgctgggattacaagcgagagccactgcgcccagccggctctctttgttattcatagtttcctggcttctcttttctgagccacccagccaaaaatgctttgactttttctatgcatgtttctgtcatgtctgtgcatgacataaatcataatatcctaagacacaaaattgttaaaggcaataatttggaaacatacaacaataaataaaatggttatagagatgtaactttaaaaagttgaacattttgttaaaacgattcctgaatatgctggaaaattcagatagttaacaaaatattttgaggataaaaaggaaaggaatctgttatctggaggtagaataacttggccattttacagaaaggaaacaaattctgatttcactttttgtatatcatccatttgacaattttcaataaaaggtttattgaaaacggaatacataaggctggtgtttggacctttttcctaattagaaattgtccatgtctccaaagattattaactcagtttattatcagctaaagagatcttaaagttgactaaacacctggaaattaaaacttaggccaacacatcaaagtctttatgacttgaagtgttttaagaattaatgaggcaaagcacacacctgtggtcccagctacccaggagactgaggcaggagaactgtttgagcccaggagtttgaagctgcagtgagctatgatcatgccactgttcttcagcccaagagactgagtgagacctcttaagaaaaaaaaaaaaatgaccggacacagttgctcacgcctgtaatctcagcactttgggaggctgaggcgggtggatcacgagatcaggagatcgagacaatcctggctaacacggtgaaaccctgtctctactaaaaaaatacaaaaaaattagcagggcgtggtggtgggcgcctgtagtaccagctacctgggagcctgaggcagaaaaacggcgtgaacccaggaggcggatctcggcagtgagctcacaccagtggctcacacttgtaatcccagcactttgggaggccgaggtgggcagatcacctgaggtcaggagttcgagacaagcctgaccaacatggagaaaccccgtctctactaaaaatacaaaattagtgggcgtgtggcgcatgcctgtaatcccagctacttaggaggctgaggcaggagaatcgcttgaacccgggaggtggaggttgcagtgagccaggatcgcgccattgcactccagcctgggcaacaagagccaaactccgtctcgaaaagaaaaaattcatgagactaaatcattttaaaaagatgtcttttattacaatttctttcaattaaacagttttatatttttgaaattttaaacaatttgtgcaaacgagatcctactggacctataaaactaatgtagttaatttagaaggtttaaatcacgagaagttaagcccaaatcttgggttgatttaattgttgtgttaacattgtttttatatcataataaaatcagaaggatgcatagacttgtttttaagctaatattaacttctatttctagcccaaagagtcatctatcaaaagccagctcatattaagtagggggaccaagagggaggtctctcagttaaacaaagttattgacttgtctttagacaggcaagacagagtatctcctcataaggttttcttttaacctttttgttctgaagttaatatgtcttttaagtgaataatcttgtttataacaacattttcttttctgttttgtttgtttgtttgtttgagacagagtctcgcactgtcacccaggctggagtgcagtggcacagtcttggctcactgcaacctctgcctcctgggttcaagtgattctcctgcctcagcctcccgagtagctgggactacaggcacatgccaccactcccatctaatttgttttgtgtttttagtagagacggggtttcacaatattggtcaggctggtctcgaactcctgacctcgtgattcacccacctcggcctcccaaagtgctgggataacaggcatgagccactgcacccagctataacaacattttcaaagtggcacattttaatatgaataaaccttctacaatcacaggcctagaaagtttttctttttcttacggaatttcttgactgtttacttgtactagatatttcttcggtatattcataatgacagaacaattgtttatgattgattgatctccaaagtttcccaagaaaagagaaaaagtaggaggggaaggaagaaagaagtgagcagaagttggcttcagagagataggaagggccagttcccttctctgtttaaggaggggagaagacttagatgcagggaaactcattttgacatgccaactcaaaccacagaagccagagtcagttcagctggtttcagtagtaactcaggaccttgacaattctgttaagccatgtcctttaaaagccagctcttattaagtagggggatgaagggggaagcccttcagttaaacaaagttactgacctgtcttttagacaggcaggacagaggatctcctcatgaggtttttttaacctttttgttctgaagttaatgtgtgttttaaatgaataatcttatttataacaacattttcagcgtggcaactgcagtttcagaatggtggaattataccagtcagagagagatgcaaatgatttaaaataggaagaaagcaggtgtctggcccagaggaccagattaagaagaccccatgagagttacaatagttagtgaaaatggtgcttctgcaaacctcatgtctacagaagctggtcaaagaccagatgccaccaggtagaatcccagcaaactcttcaatggtagatatctgtcaccatccttaggaggtaggtctgtggaagctcactataataccatttgcttaacagatatacaaacatggatcagatataatttcaacccacaaggagctcacagtctggctcttcttttgaggcaaaaagactaaagctgttgcctttatggtaagataaatctgccttggagtcaatccaaggtgatttaattactgtaggtagttgtaccaataaggcttgtatcccagagaactccatattgcatttaagcttgttagtaagccaggccagctctatttcctgtgaggactttaaaaaaaattgcattcacacatttaaaaattagcataagcagggtgcagtgatgcacgcctgtagtcccagctacttggtaggcagaggtgggaggatcacttgagccccagaagttcaagaccagcctggacaacaaagtgaagtgaagactgtctcaaaaaaattaattatgacataaaatgttatatgtcttaatttacacaaatataagtatatacttttaaatcccattcttacacacaaaagctagcatactgtgtaaagtattctggacctacacacctttatttttttaacataacaatatgtcttggatacattttcctatttgtctatagaaagtttcatcattattttaaaaaatttgtttttggctgggcacagtggctcatgcctgtaattccagcactttgggaggccgcggcaggcgaatcaggaggtcaggagtccgagactagcctggccaacatggtgaaaccccatctctactaaaaatacaaaaacttagctgggcgtagtggcgggcgcctgtaatcccagctacccgagaggctgaggcaggagaatcgcttgaacccgggaggcagaggttgcagtgagccgagatcctgccacagcactccagctggggcgacagagtgagactccatcttaaaaaaaaaagtttgcttttatatttcatacctgcatggtattctattgtgtgagtaggccatcatccagtggtcttcaaactttcctgtgtactccgtaacagaatttgttgttttgacatgcagtctcactctgttgaccaggctagagtgcagtgccacaatctcagctcactgcagcctccacctcctgggttcaagagattctcatgcctcagcctcttgagtagctggcgcatgccaccatgcttgactaatttttgtatttttagtagagacgggatttcaccgtgttggccaggctggtcttgaactcctgacttcaagtgatctgcccgccgtggcctcccaaagtgctgggattacaggcttaagctaccacgcctggtcttctaatagaatttttaaaaactgtatttacccccttgcacatttaaattgacatctaagatttttattataagtttaaatagttgtaaaggatgtattttccattatattttatacattccttaattttatatatatatatatatatatatagttttttttttttttttttttgagatggagtctcactctgtcacccaggctggagtgcaatggtgcgatctcggctcaccgcagtcactgcctctagggttcaagagattctcctgcctcagcctcccgagtagctgggatcacaggcacccgccaccatgcccggctaatttttgtatttttagttgagatggggtttcaccatgttggtcaggctggtctcgaactcctgacctcaggtgatcccccccacctcagcttttcaaagtgttgggattacaggcgtgagccactgtgcctgccctcccttaattataatttaaaaaatttttgcagatgtagatttatataaattggcaagccagttctctttatcaaattaactgatcaaaaaaaaaaaaacagattaactggtcaaacatagatttactttctgtcagtaaaattttgacttcatttttttaaatcaaataagcatgttaacccggtattgctgtgacaacctttatcctaatttcttttcttcttcttcttcttcttcttcttcttcttcttcttttttttttttgaaatggagtcgtgctctgtcacccaggctggagtgcagtggcacaatctcggctcactgcaacctccacctcccaggttcaagcaattcttctgcctcagcctcccgagtaactgggactacaggcatgcaccaccacgcctggctaatttttgtatttttagtagagatggggtttcaccgtgttggccaggctggtctcgaactcctgacctcaggtgattcgcccaccttggcctcccaaagtgctgggattacaggcatgagccatcgcacccagcttttttatcccaatttcaagatgggtgggcaggtaggtaggtaggcaggtgggtagatagatagggccttcagacttgcctcgcattcatcttttacataaaataagacagtttcaccttgaacacttctgtggtgagactgtttagtcttgtagctctaaactccagccatactctgatgactcccacatttataaatcccagatttgtatactcaactacttatctaacaggtcaaaactgaactcttaaaattcttacatttgtgtccacacatgattggctaagctaatggggctcagatttaccctgtcacctgaaacaactgtaaaactggagaaaatatgtcaaactctgaagttattaggtctaaggtgattaagaacagcgaatcctgagacctgagaaatagagccctatgattgctctgatttaatgctcggagaaagtttccagaccgcggtgcggggagaaggaacatcagcaggccccagcagtctctcctcattgaagaggtaaaatgaaaatccagggcagctggggcagctagagttcacaggcagagaaacaaagaggcaagagatgcacagagaagagaacactggcctgcagatgcccagggagcccactcgagtattcggttgagtactgatcagtgcacccatgtgaggaaaccccttagttcagggaaggagccactcaaaaggattagagagaaccatttacggagttcacacagggccagaaatagttcctgttcccagtagcagagtagaacatttcatgattcaggggtattgattggagtactaagaagagttgtattagtgaaggttcttgagagagagagagagagagagagagagagagagagtgtgtgtgtgtgtgtgtgtgtgtgcacgtgtgaagaaatttattgtaaggaattgccacgtgattatggaggctgataagtcccaaaaatctgcagggcgagtcagcaagatggagacttaggagagccaatgatgtggctatagtccaaaggctgacaggctcaagacccaggcagagccaatgtttcagttcaagtccaaaggcaggaaaaaagttgatgtcccagttcgaaggcagttaggctggaagaattctcttttactcaggaaagggtcagattttttgttcaattcaggcctttaacagattgaatggggctcacccacattagggaggccaagctgctttacgcattttgccagactaacgtttgaccaaagatctgagcacgtatggcccagtcaagttgacacataatgttaatcatcacaaaagtcttgcctcaatagttgggaaaaattaatcctagaataaatgctattctggtcttgcttagcaaaggttaagagcaagaccaaaaagatcaaaccttttccaaacaaaagctgaagaatatttttagggatacaaaaccatctaggaccgagtgtggtaaaatgcacaatgtttaccagccattccagaattactaggtatgagcagaagtagtaacatacaaccaataactgaccagaaatgagacagattatataagtagtacattacagacattagtcattataattgtattccatgtgttcagtaagctaaagaaaagatttaatatgttaagtaaagacatgaaagatgatggctgggcatggtgcctcacgcctgtaatgccagcactttgggaggccaaggtaggtggatcacctgaggtcaggagttcaagaccagcctagccaacatggtgaaaccccacctctactaaaaatacaaaaattagctgggtgtggtagcgtgcacctataatcccaactatacgggaggctgaggcaggagaatcacttgaacctgggaggcagaggttgcagtaagccaagatcgtaccactgcactccaacctgggcgagagagcaagattccgtctccacaaaaaagaaagatacagagatgaaaaatacactgaagactgtcagaataaacattgcacaagtaaagatttgtgattttgaagacttaaccatagaaactatccaaaatgaagcagaaaaaaaaaagaaaccctgaaaaaaatacatgaacacaacatcagtaaagtgagggacaacatcaggtagccaaatgtgtgtggaattggagtccctgaaggaagggagggtatgagggaccaaaaaatatatatagagagagaaaaaaaaatggctgaaaaatttccaagtgtaatgaaagcagtaaacacacagatccaagaatttcaaggaactccaagcacaggaaacatgaagaaaaactatatactaaggcacatcttaagcaaattgcttaaaaccatggtttaaaatggccaaagaaaaagatacattatatacttaagatcagggtgacaccagatttctcattggaaacaatgtaagccaggttaacagtggaacaatacatttaaagcaaagaaagaaaacagttgtctacctagaattcttttctcagtgaaaatacctttcaaaaatgaaggcaaaataaggtctctttcagactttaaaaaaaaaaaggaagaatttattaccagtagatatgcagtacaagaaatatcaaaggatgtaattaaagcagaaagagaatgataactggtagaaaactggagccaccaggagtcccaggctgcagtgagctatgatcgcaccactgcattccagcctgggtgacagagtgagaccctctgtctaaataaacaaacaaataaaagaaaactggagctataaaaataaatgaagacaatgcaaagggtaactaagtggataaatacataagatattttttctttttgtttcagtctcattaaaagatatgtcttagaggtaattacacattgtagcatttgtaacttacatagaagtaaagtttatgacaatagcagcacaaagactgggagtgggagaacaaatatactcttgtaagctttttacactacatgtgaagttgtataatgtcaattgaaggtagactgtgataagttaaagatgcatatgataaaatctatagtagcagagttatagctaatgagccaacaacaataaaaagttgggatataatcccaacactttgggaggccgaggtgggtggatcatgaggtcaggagttcgagaccagcctgaccaacagggtgaaactttgtctctactaaaaatacaaaaattagccgggcatggtggtggcacctgcccgtaatctcagctactcgggaggctgaggcaggagaatcacttgaacccaggaggcagaggttgcagtgagcggagatagtgctactgcactgtagtctgagcgacagagtgagactccgtctcaaaaaaaaaaaaaaaaaaaaaaaaaagttgggataaatatctttaaataatccaaaagatggcagaaaaaaaaactaaacaggaaaagcaaacagagcagatgggacaaatatgaaacaaagagcaagatggtaggttaaaattcatatcaataattaattcaccattaagggccaggcagagtggctcatgcctgtaatcccagcattttgggaggtggattaggaggatcacttgaagccaggagtttgagaccagctttggaagccaagtgagactccatctctacaaaaaaaaaaaaaaaaaaaaaaattagccaggtgtggtggtgtagttccactcaggaggctacggtgggaggatcacttgagcccaggagtttgaggctacagtgagctctgatcacaccactgcactcctccagcctgggtgacagcgagattccatcttaaaaaaaaaaaatcctcattaaaagcagacattgtgagattggataaaaaagcaagacctatttatatttatatgctgtctacagttatcccactttgaatataaaaatacaaatacgttaaaagcaaaagagtggaaaaagatgttaatatgttaacattaatgaaaagaaaaccttagtggcatattaaacaaactatattttaaaatgaatgtcaccaaggataaaggagaattatttcataataataaagagatacattcatcaagacataattctaaatgtttatgcatgtattaacagagattcaaaatacaaacttttcaaggagaaataaatctgtaattatagttgaaggtttaacaactctctcacaaaaactgatagaacaagtagacaaaaatcagtgaggatatagaagatttggacaatataatcaactgacttgacttaattgatgttcagtagaacattcgacccctaaacagcagaatacacgttcttttcaagtgcatatggaactgtttccaagacaaatcattttctgggccattttaaaagcctcagtagacccggcggggtggctcacgcctgtaatcccagcactttgggaggccaaggcgggcggatcacctgaggtcaggagttcgagacaagcctggccaacgtggtgaaaccccgtctctacgaaaaataccaaaaattagctgtgtgtagtggtggatacctgtaatcccagctactcaggaggctgaggcaggagaatcacttgaacccgggaggcagaggttgcagtgagccgagattgcactactgcactccagctgggcaacagtgagactccgtctcgaaaaaaacaaacaaacaaaagcctcagtgaatgtaagctgattcaatttgtagaaagtatgatctctggccaggtgcggtggctcacgcctgtaatcccagcactttgggaggctgaggcgggcggatcacgaggtcaggagatcaagaccatcctggctaacatggtgaaaccccttctctactaaaaatacaaaaaatcagctgggcatggtggcgctcacctgtagtctcagctactcaggaggctgaggcaggagaatcacttgaacccgggaggatgaggttgcagtgagccgagatggtgtcactgcactccagcctggctgagagagcgagactccatctccaaaaaaaaaaaaaaaaaaaaaaaagaaagtatgatctctggccacaaggaattaaatgaggaattaataacagaaaggtatctggaagatctttcaaatatttggaaaataacataattttaagtaaatcatgggtcaaagaaaatcaacagcgaagtaagtaagtatctggaactgaatgaaggtgaaagtgccacataaaatttgtgtgatggagctaaagggaaatttatatagtgcagatggtccctgacttatgacgtctcaacttacatttttcaattttatgatgggtttttcaggatgtaacccaattttaagttgagcatctgtatcagaaaagaacaaaggtcccaaatcaatgaccttggggtcccacttttagaaattagaaaaaatgaagactagtgaaaccccaattaagcagaagaaaaagccagtgtggccaggcagggaggcccatgcctgtaatcccagcactttgggaggctgaggcgggcagatcacaaggtcaggagattgagatcatcccggccaacatggtgaaaccccgtctctactaaccatacaaaaattagctgggcgtggtggcgcttgcctgtgtaatcccagctactcaggaggctgaggcaggagaatcgctttaaccagggagtcggaggttgcagtgaaccgagatcgcgccattgcactccaccctagcgacagaacgagactccgtctcaaaaaaaaaagaaagaaagaaagaaaaagaaaaggccagtctggaaatcaatgaaacagaaaaccagtacagaaatcatgaaaccaaaagctagttatttgagagagcaatgaaactcataaacctctacccagactgatcaggggaaaaaagggaagacaataactgtaatatcagcagtgaaagagatgacatcacacagattctaaagatattgaaagtgtaataactgaatattgatcagcaatctagaagaaacagattccttgaatgacacaaactaccaaagttcactcaagaagtaaccatctgccgggcgcagtggcttacgcctgtaatcccagcactttggtaggccgaggtgggcggatcacgaggtcaggagaccgagaccatccttgctaacacggtgaaaccccgtctccactaaaaatacaaaaaattctccgggcgtggtggcgggcgcctgtagtcccagctactcaggaggctgaggcaggagaatggcttgaacctgggaggcggagcttgcagtgagccgagattgcaccactgcactccagcctgggtgacagagccagactctgtctcaaaaaaataaaataaaataaaaataaagtttagtaaaataaaaaaaatcagtaaaatacaaataaaatttagtaaaaataaagctgattctaaaatgcatgtgcaacagaggatctagagtagccaaaataagctcctctgtctgacttaaagtcttaattaaaataatcagacaggccgggcatggtggctcacgcctgtaatcccagcactttgggaggctgaggcaggtggatcacctgaggtcaggagttacaaaccagcctggccaacatggtgaaaccccatctctactaaaagtacaaaaattagtcaggcgtgatagcacacgcctgtaatcccagctactcaggaggctgaggcaggagaatcgcttgaacccgggaggcggaggttgcagtgagctgagatcatgccaccgcactccagcctgggcgacagagtgagactctcaaaataatgaaataaaaataaaaaactgaacttcatatcttgtccccagatctgatatagtcacttcttcctttgttcagttaaacccagcttcatgtttctgcttgcccagggccaataactttgggatcttccttgactcttctttttctgtcaaaccccgtaccagtctttcaggtaaccgtaacttcagagtctatccaggtcacctctgcttgtccaagcccctgtcatctctcacttggatgatttcattagcctcttggccaggatccctgcttctgctggtatttccttagtttcttctccctacagcagccagagctaatcattttaaatgtcatatttctgtctcgcctcagctgcaaaccttccagtaccttcccagctccttctaaataaacaccagaggccgggtgcagtggcttatgcctgtaatcccagcactttgggaggccaaggtgggcagatcacctgaggtcaggagttcgagaccagcctggccaacatggtgaaaccccctccctactaaaaatacaaaaattagctgggcgtgatggcgcctgtaatcccagctacttgggaggctgaggcaagagaatcgcctgaacccaggaggtggaggttgcagtgagccaagactgcgccactgcactccagcctgggcaacaagagtgagactctgtctcaaaaaatataaataaataaacaaacaagcaccagagccctggcagtcacctgtgaggcttcaccccgtctccccacccactataacctctgacttacctccttttacactccttcttgctgactctgttccttccacattggcctctttgctcttgcttgaatgatccccagtcatcctccctgcccagggcctttgcacttgctgttctctgccaggaaggtgcttcctccgtagttcactcttcacctcctttgggtctttgctcagttgtcatcttcagtgatggctcttctgatcaccttatttaatttttattttttaattaaaaattttttttgtggagatgtcttgctatgttgcccaggcttatctcaaactcctggactcaaacgatcctcctgcctcagcttcccaaagtgctgggattacaggtgtgagctaccacacccggccccgatcaccttatttaaaattgcagctcccagcccccaaccccagcatacccattcctcttttttttttttgagacagaatcttgctctgtctcaaattccctccagccatgagccctgaaatgaaacaagttatctatttccaaaacacaacagtggggcaggcataggatagacattcccattccaaaagggagcaataggcaagaagaaaggggtagctggtcccaagtaagtccaaaacctgagacagagtcttgctctatcgcccaggctggactgcagagtggtgcgatctcagctcactacaacctccgcctcccgggttcaagcgattctcctgcctcagcctcccaagtagctgggattagaggcatgcaccaccacacctggctaatttttgtagttttagtagaggcagggattcaccatcttggccaggctggtctcaaactcctgaacctcaggtgattccccccgccttggcctcccaaagtgctgggattacaggcgtgagccaccgcctggtctccctcattccttttgttatcagtcatccctcccagccctggcaactgctgctcactttcctgaccttagaattttgcttattacagaatgtcatataagtagaattataaagtatctaagcttttaagtcctaatgcatttaagatctgtaaaaagtaaagtagaggttcctcttcaaagactttcctccccatctaattaggaataaatagtaacttctcttagaagaaaaatttattcaaagacctgtgctaacattcttaaatatctgctagccataataaagaaatcaatgtactttatattcttagctctcacaatttagcctaaatatttgccctggcatgcttatactggtccaagcaagcattaggtcatggcctgttcctcttccttatttgaaggtgtttttacctttctcagcactccacaagttacttcctccttcctttgttctcctctgcctttgcctcttttaaaaagttctaagttcctagccaatcaggacaaatacagaatgtgaggtcctgttccagccaatggaaactggacacagcagtagggtggacgcgtcaggttgtaaatgaccctgtctcctttgttcagtgtactctcatggcaaaactgctggtgagtgtaccctttctgcagaaagtaaaaaatggccttgctgaggaaattaaatttatgttcaagtgctttttcttcagggcaccagggaacaagcatttctaacagatccatatgtgtcgctgcatgtaatcagtggttcattcctttctattgctgagtagtgttccattgtatggatgtacccgtgtattgatccatccatccactgaaggatatttgagttgtttccagtttttttgtgattatgaataaagccactgtaagcattcacatagaggctttggtgtggacataagttttcatttctcttcggtaaataattaggagtagaattgctaggtcgtaggataagtatatgcttaacttaggagaccctgccacagtattttacaaagtaagggtgctattttgcattactaccagcagttcacaccatatgtattcacaccagttgctccatttggtcttcgttctgtgacttgtctctattctcttaacagtatctttagaacagcagaagtttttgattttgatgaaattcagtttatcgggccaggctgggtggcttatgcctataatcccagcactttgagagaccgaggagggtggatcacttgaggccaggagattgagaccagcttggccaacatggcgaaaccctgtctctactaaaaatataaaaattagccatacatcgtggcgcatgcctgtagttccagctactcaggagtctgaggcaggagaatcacttgaaccctggaggaagaggttgcagtgagctgagatcatactgctgcactccagcctgggcaacagagcaaaactccatttcaaaaaaaaataaaataaaatttcagtttatcagtgatttctcttaagtttcatgcattgggtattgtagctaagaaatcttcacctaactcaagtttacaaagattcttctgttttttttctagaagatttataagttttaatttaacttttaggcttataattcatttcacattaaatggtgtatgtggtgccaggtattgctcgagagtcatcatcttgcataggggtttcggatgttctagcaccatttgttcaacagatagcctcttttcattaaattgccctttcacctttgtggaagatcaattcagcatgcatgtatgggtcacttgtatgtttttaattgatttctaaattctgaaaggaaaatgataaaaaggaagattctttcactatatctgcatttccaatttctcccccaagaacgctttcctaacacctgcaggcagaactaaccactctgggcccctgtagctgttgtgcgtatgtttattattgagtttttctggcctttgcagttctttcagtgtctgattctccctctctctcagcttctttctcaagactgtgcatccttggaggtcagaaattgtctcatcctgccgggcgcgatggctcatgcctctaatcccagcactttgggaggccgaggcggttagatcacaaggtcaggagttcgagaccagcctggccaacatagtgaaaccctgtctctattaaaaatacaaaaattagctgagcgtggtggcacatgcctgtagtcccagctactcgggaggctgaggcaggagaatcgcttgaacccaggaggcggggaggttgtagtgagctgagattgtgccactgcactccagcctgggcaacagagcgagactccatctcaaaaataaataaataaataaaagacaaaataaattttctcatccttttttgtcatcttcatcacagctggctctctaatgttcgttgaatgaaagggccattcccaaatctctgataagtcaagcatttttaggagagctaaaccagccaaatgagaccaggaagtgaagaaaaatacctttttttttttttttttttttttggagacggagcctcactttgtcacccaggccggagtgcagtggcacgatctgagctcactgcaacctccgcctcccaggttcaagcaattctattgcctcagcctccccagtagctgggactacgggcacacaccaccatgcccggctactttttttttgtatttttagtagagatggagtttcaccgtgctggccaggctggtgtcaaactcctgacctcgtgatccgcccgcctcagccttccaaagtgctgggattacacgcgtgagccaccgcgcccagctgaaaaatacctactttttttttttttttacagcaggaggtgtttctgcttctactttgctgtgacttctgtttctccaggcattcctggtatggacatttataccaggtgttttggtcattggtgggctctcagcttcagaggacacttggcttctctataccctatctttggtgacttctgcttgttggacttcagtcactgcagttcacaagtttcacactcatgaaatatttattgttaattaattccaatatttaattgattgcttctctttctcagcactttggaaacatgtttactacctagacattttcctacagtagatttttaattcttaacattttgatcttaagcaatttaccatgatacttggtttccatgagagatttaacagttggaactgtactgcccataagatgcaggtggggtcatggtatgtagttgggaactctacaaatggcagcccttcatgcctttgcaaaggctgcaggttggaaagctgccattacttgtgagggcgtccaaatgcttcctgtgaatggaagatgtgtttctgtgcctcactgtcttcactgtgctggattgctggctttctcagatgtctttatttgagtcaacctgtattccatctccccactcccacccagtcttgatcatctcatttgtgtgtatacaaccttcccctcacacacacctctttgcagagtttcgttgcactgggcgttgggaggagaggcgtcagagttgggtggaatcatttcaggctgactgtccagacatagctctcattagaagcatcagtaaataagctgaaaaccaacaacacgtacagcacagtctttctgtgtttgcagcttggaactgagcagccctcactgggtgcatttctaatcctttgtctcatcatttatatgacatccacttagaaaaaggtgttaaaatcatataacatattgctttttccccttttttattagcagttttactgaggtgtaatttatatgccataaaatttaccatttgaatgttcaattcaatgatttctactaaatttatagagtgtgcaccataaccacaatccagttttattttttatttttttttcgagacagagtctcactctgtcactcaagctggagtgcagtggtgcaatctcggctcactgcagcctccacctcccgggttcaagcgattctcctgcctcagcctcccgagtatctgggactacaggcacgtgccaccatgcccagctaagttttttgtattcttagtagagatagggtttcaccatgttagccaggatggtctcgatctcctgacctcatgatccgccagcctcagcctcccaaagtgctgggattacaggcgtgagccaccgcacctggccccacaatccagttttagaacatttccagcatccccaaaagatcccttttgtccctttgcagcagtcctacccccacttccagccccaggcgaccattcatttgctttttctatagatttgtcttttccgtacgtttcatgtaaatgaagttttatacaatatatgaccttttgtgactgttttttttcccagcatgtttttgaggtttatctgtattatagcacgtctcagtactttgttccctttttatcactgagtattattccattgtacggacatacatttttctctattcactagttggtgaacatttggattgtttccagttttggtcatcattaacaatgctactatatatatccatgtataagtctttgtgtggatatacattttcatttctctagggtagatttctagaagtaaaattgctgagtctttttttttttttttgagatggagttttgctcttgttgcctgggctggagtgcaatggcataatcttggctcactgcaacttccgcctccctggttcaagtgattctcctgcctcagcctcccgggtagctgggattacaggcatgtgctaccacacctggctattattattattattattttttttttttttgagacagagtctcgctctgtcacccaggctggagtgcagtgcgcgatctcagctcactgcaagctctgcctcccgggttcatgccattctcccgcctcagcctcccaagtactgggactacaggcacccgccaccacccccggctaattttttgtatttttagtagagacgaggtttcactgtgttagccgggatgctctcactctcctgacctcgtgatctgcctgcctcggcctcccaaagtgctggcattacaggcgtgagccaccatgcctggcaaattttgtatttttagtagagacgaggtttcaccatgttgatcaggctggtctcaaactcctgacctcaggtgatccacccaccttggcctcccaaagtgttgggattacaggcgtgagccaccacgaccggtcaaattgctgtcttatagtaagtttatgtttaactttttaagaaactgccaaactatttcctaaagtgactgtaccatttacattcccaccagcaatgtgtgagtgttccagtttttccatgtccttgccaatagttggttttgtctgcctacctatccccgcccctgcttttttttttttttttttttttttaagagacagggtcttgctgtgttgttcaggctggcctcaaactcctgggctcaagtgctcctccctagtagctgggactataggcacacaccagtgtaccaggggttgtctgtcttttgattatagctattggaatgggtgtgaagcagcatctcgtgattttagtttccatttcttgaatgactaatgatactgaacatctttttatgtgcttattagccatttgtatttcatctttggtgacctgtcaattcaaatcttttgcctatttttttttattaagtttgtgcactgtcttattatcgagtggtaagagttctctgtattgtgggtacaagttcttttttttttcgagatggagtctcgctctgtcacccagggtggagtacagtggcacgatctcagctcactacaacctctgcctcctgggttcaagcgattcttctgcctcagcatcccaagtagctgggactacaggcttgcaccaccacacccagctaatttttgaatttttagtagagacgggatttcaccatcttggccagacgggtctcaaactactgacctcgtgatcctcccacctcggcctcccaaagtgctgggattacaggtgtgagccaccgtgcccggccttccaagttctttatcaggtatatgatagcacatgtagctttttatcttccttacaccagtgcaagtttatagaaaggaaaagggatagttaatagtaatcataataatgtttaatatttgaatgttttttaggagctggacactgggctgcatgtttcacggggatgatttgggtcactcttcaattttctaaaggttacaggactgtttcaaacacctctccttctattaacagttttcaatggagaaagaaaacaaaagattgatttggggaattcttaggttaatgcgagttagaactgaccttttaacattattaccataaggactaaatggctgttacagacccaaaataggagcaattcaaacaagcgagatgcttctctctgtaacaggctgacagtcgcggtcctggaggggcacgatggctcctcagggtcagacacctcctgtcccttactctgtaaggcacagcttctacctcaggatccaaaatgcccacgccagctgccatggcccctcacaggcagtggacaccagaaagaggagagggagtgcgtgcctgttgctttgaagaacctgacccagaagtcttacacagcacttttgcccacataccatcacttagtcatgtggtagtgcctggccacaagagagactgggaaatggagtctttattctggggtgatgtgtcccatctgcaactgaggggttaaggcctaaaacttagggattgaaggcaggagaaaaaacagatgtcgagagccagtgttgggattgcagggtcctgtgtgggattcctgttcattttcatcaaagaaagtctagttgatatgcaattgttggcctaagtgttattgaggagttaattttactgttgaattacaccagaacatttgtcatgtgaaataactataaatacgactgattattgcctagtgtattacagttctctccagagacacaggaaacaatagggtctgtctatcggaatagatatcctaaaagtgtatcttttgaagagattgattataaggtattggctcatgagatgatggagcttaagaagtcccacagtctgctctctgccagatggagacccaggaaagctgctggtgtagtttgaaggcctgagagctgagggccagtgatgtggattccagtctgaaggtctgagaacccagagggctgagggcaggagaagatccatgtcccagctcaagcaggcagagggagggtaaatccaaccttcctttttctgtttttttgttctaatcaggccctcaacggactggaggatgcccagccaaagtggggagggccatctgcttaggcagttcaccaattcaaatgctagtctcttctagaaacaccctcacagacacacctggaaataatgtttaagatctgggcatcctgggggtctagtcaagctgacacatacatttaaccaccacacttagggaatatgaaaataacttagacattaaatttgattttggtgttgctgtaaagaatacagatcttaggcaccagctcgtaggaggggtggtaaacaaggaggacagcttttaccaggttgcctttggaagcaaaactctgctttgctgttttgttttcaagcggctgcatggccactgagcgagccctttcctgccatcaccacagtgccacttagtgaacagtttctccaaggttaactgtagctgctcttgttcagttaatatgtagttctggattaatatgccacatctgtcactttaaggaagaaaaagagcagttccgtttagagatcccattgctcctctaaggacagcagtcatttctaacaagcagagggaagaaatcttctggttccatttgtcctttgtgtgtgttgaaaaccttgacaacaaaacaaattggtactgaatggtttgaagaaataaacattaactcccctttagtatttcatttctagggtttccagccttggtaacaattaccaagaactttgctgtcatggggtacagctctaggctgctgacaggatcttcatactggaggagactatacttttatagccaattccaactgccccagagataacttggataaacactggctcctccactacctcctaatccctgctgggttttacactgtggggaggtttagacaacttgttttctttcccttttagcccttctctctacactcccctccagctgccttcttcccccacccccaaatgtaacgtgatctcctaggcctgctctgctgcttttgcagattcttttagtcttagagaaagagaggaaaacattaaccattggtttaccaattcaaagttaacaacattttaaacaaaaggagcttgtcaataaccagggcttgggcttttcttttatcagttcctcctacttggctgagtttacctcatcataaatcttatcacacagataataatttgacagctttagggtttttgcagcattgctattttctattgcaacaaagctgtaacattgctatttttgatgtatttgttttatagatatcttaatcttcaatattcagattaaaaacaaacaagacttagtgatttaaaattatttggtaaaaaggtaaagggacagagacatctcatgaaaacatggcaaaatctctttaagtttaattcaagcacttagagtttaataagaatatcccaaaccatttttgcttaataatatttctgtttataattaaaccttaaggtacagtgttgtaactggatttaagaatttagagttttgttgtttcttcgccatcagcgaaattaagatttaaaacctatagtttgcaacaaattttagtttttcagcctagtgtcctaaaacttgtctgtcatgggtacctagtaggtgtcatgtcacaggaaagggatctaacaagggagtttgaagataggggttttccttgctctgccactaacttgctatgtgacctagggcaagttatataacctatctgtgtcacagttgtctgaaatgcaatatggggaaaataaattcttaaaatgacaataaaaagatttctttttttttttgagacagagtcggcgcaatttcggctcactgcaacctccacctcctgggttcaggcgattctcctgtctgagcctcctgagtagctgggattacaggcacacaccaccacgcccagcaaatttttgtgtattttgtagagatggggtttcgccatgttggccaggctggtctcaaactcttgagctcaaacgatctacctgccttggcctcccaaagtgctgggattacaggcatgagccaccacgcctggccaaaatatatatatacatattttaagtgaagatgtgtaaggactaaaggagcccaaaggagacagtaggggataagaaaggcaaagagagtggtaatagatttagcagaatcaaggatgccaaaacctcttctgagagagaccttgattaagagtgagctggtttgcctgtaagaatctgcggaaaggtcagaaattagagacattagtaccacagaaagcaggggatgaggcctgaagctgaaatcaaggggatcaattgagagcctataaaaggagggtttagattcttcaaacccctcccaaccccacagagtcagatgaccacctctcctaaccacctacaggagaccagaggcattatattgagaaatgcccggccgggcgcggtggctcacgcctgtaatcccagcactttgggaggccgaggcgggcggatcacaaggtcaggagatcgagaccatcctggctaatgtggtgaaacaccatctctactaaaaatacaaaaaattagccgggcgtggtggcgggcgcctgtagtcccagctactcaggaggctgaggcaggagaatggcgtgaaccctgaaggcggagcttgcagtgagccgagatggcgccactgcactccagcctgggcaacagagcaagactccgcctcagaaaaaaaaaagaaaagaaatgccccgtagaggctctgcactcagaagcctgacccccagcatgggtccgggtaggccattggccgaaaatagtggagtgggcaaagagcagattttttaaaagtctgcatactgaatagtaagattcccagccctcttctaatacctgctagccaggggcctaataaggaagagattgaaatattcttttctagggggaaaaagttgaatgaccctagagaaaagccctacagataccaacatttagggattctcttgaaaaagcgagtttaccatctcctttcactgaagcttaccagtggctgtgccccttccacgcatacaaaactaacagtcatcttttagttgctcattcatagagagtgagtggcctgccaaatctctctaggcattagaggaaggtctctaacctgatattaatagataaagggtaaaacaaatagcagaaaacaggaacttggtggaaataaagacaatgcagtcaacagaggaagagtttaaaagaactattcagcttgggcaccatgactcacgcctgtaatcccaacactttgggaggctgaggtggacagttcacctgcggtcaggagtttgagaccagcttggccaacatagtgaaaccccatctccactaaaaatacaaaaattaactgaacatggtggcaggcacctgtaatcccagctattgggaggctgaggcaggagaattgcttgaacctgggaggcatagcttgcagtgagccaagattgcaccactgcattccagcctgggtgacagagtgagactctgtctcaaaaataataaataaataaataaataaataaataaataaataaagctatgcatttcccacaaatactgcttaaaaaaaaaaagaactattctttgctatccttggagagagagattgcaaatgtcagaaaacaggatgcttttaaaaacaataacaatcagaataagaataaaaatgaattatttttcttttatttatttatttatttatttttgatacatggtctctgtcacccaggctggagtgcagtggcaagatcacagctcactgcagccccaacctgcctcagccccccaagcaactgggactacaggcacgcaccaccacacctggctaatttttaaattttttgtagagagatggggtctcactatgttgcccaggctggtcttgaactcctgggctcaagtgatcctcctgcctcagcctcccaaagggctgggattatgggcatgagccaccacaacccagcaagaatgaattgtttaatattaaaaacattatagcccaaatttaaaatccaacagaagatgtggaaaattgtctcagaatgtattgggttggtacaaaagtaattggggcttttgccattttaatgacaaaaacgttgattacttttacaccaacctaatagaacataaagacaaagacatggactgttgagagaacaataagagagaacaggtaagaaaattagaaactctcgggaggctgagacaggataatcgcttgaacccaggaggcagaagttgtagtgagccgagactgtgccattgcactcctgcctgggcaagcaacaagagtgaaactgcgtctcaaaaaaaaagaaaagaaaattagaaactcaatcccagggctttaatatcctttttgtaggaattccagaaagaaaacaaaaaaataatgataataacgaagaaacaaatggaggagaagttaggagacgttaaatgtaaggaaaaatttcagagtttagtgaagtgagtattttccaaaacagaattatataaatctctggatttatgagtgcccagaataatatatgaaaggccatatcattgtgaaagttcagaacaccaagaatattagaagatcctaaaagtttccaaagagaaaaaaagcaagtcattttaaggggtcaggaaccagaatgggattgcatctctaaacaatacttactggaaactagatagtagcagataaataaatgccttcaaagttcatttgggaaaattattttcaacctagaattctatacccagacaaactgtcaagatagaagaaaggtatttttttagacatgcaccctccctccccacctctgtgaagctactggatgatgaattccagcaaaatgaagaagtcagtcaataagtagaactgagcccgggcacggtggctcacacctgtaatcgcagcactttgggaggccgaggcgggcagatcacgaggtcaggagattgagaccatcctggtgtaacacagtgaaaccccgtctctactaaaaatacaaaaaaattagcagggcgtggtggcgggcccctgtagtccgagctactcgggaggctgaggcaggagaatggcgtggtgaacccgggaggcggagcttgcagtgggcggagatcgcgccactgcactcccgcctgggtgacagagcgagactacgtctcaaaaaaaaaaaaaaaaaaaagtacaactgagaatatttgaaatgttttagtgattggaaaaaatatcactagatgtttgacagatctttgaagtatttgagggaaaatggtgataggtatatagaagactaaatgaaaacaaggcaatatctctaggataaacaaagatgtataataaaggaaacattcatagtatattattggctaagcagtgaagaatatttatatcatcctaataatgtaaacactaactattgatttatcccccaaattgtgattttattgttttggggggttatggatggtgatagtataatactgctgtcataagttaatagataatggataaatctaatgaattcagaaagagcaagatgatgttactagctaaaaatctgaaggaggctgtctctgcggaaacatacaggggaaagggattgctgttttttattaccagatttttacaagactatttttagccttttttacaagacttttagtactgcttgagttttaaccatgttatgtatattactttgattaaaaagaaaaattaatttaaaaaaatgagcatactaataccattaattttctccttctagagaaaaatgtttaacagttaggtttagacttgttaattataaaaatatagtagtcttactgtaatgagattttctagaaagcggatttactctaaggcagttcagatttggtccccagctgagaattatagcctggaaataccaacagaaaaatcagtgtcatttgaaggacagtcatctgtgcagcctgtgcatgaaatcatgggtctgaattaggcccccattcaagatgcgggggtgtggggtttgtgttttgctgaagctgtggttgcaaatctttgctttaggatgaaaggtggggctctctgttacatttgaaccttagttgctactcctacctcacagctagtgtttctttctcttcataaaataaattgatttcctggtcccttggaaaacctccagactgctttctggaatcattttcatatagcatgtttgttaatttgagctcttgactgagtcccagtgagatgtaggcaggaacacagacctgatacagaaatagtcctcttttggaaataacaatagctactgtttatcgagcaccttctgtgctttgggcactctccctacatgattcctaatcttcataataaccctgtgagataactactcttatgactacctcccatttttcagatgagaaaattgaggctctgagaggtgaagtcgttgcccatggccccccagtgagtggcagatctgagactcagcgctagcctttgtgacacataactcgtgaccagcaggtagtgctacccgattgaaaaaatgtgagacttaaagggatgcatgtgtccctatacagtggcaaaaactggtatgacagaaatgatgttttaagctatgttatcctttagttggacatacactggacccacagagctagagtacctggcaggctcttgctggacaatgtttgctgaatcagagaaagtgggctttgttggcatttgcatgtgaaatactgtgcacatacctcaagatctttgctgttccccccctaaagctactagctatgctggaaacagtgaaggggtcagccagacctggggtcaccttgtcctggggtcccaagccaggcctcctgtcaggttcatctgtctctgttccacctgcactcacacccagtcttgctgctgagagatggagcatccacatcctgaatcctgcctccttcccttgacacacttctatggtgggtgcctgcccaactttttcttaataggactaaattccaaattaaaaaaaaaattcagtctctctcctctaatcatccaagaagagtcctcttttggtaacttgttctagaactatgcctatcttaaattcagaaattgctttcaaatgaattaaattttagaaatatccattcctgttcgtcctattcccagtgaaaataagcaactcttccctcttccaaaacagtggatttcttttctttttttctttttttgaaatgtagtcttgctctgctgcccaggctggagtgcagtggtgcaatcttggcacactgcaacctccacctcccaggttcaagcgattctcctgcctcagcctctcgagtagctgggattacaggtgtgtaccaccatgcctggctaatttttgtatttttagtagagacaggatttccccatgttggccaggctggtctttaactcctgacctcaggtgatcgcccaccttagcctcccaaagtgctgggattacaggcgtgagctactgtgtctggcccccaaacagtggatttccatcttacatatgcatacagatcatctgggagcttcagatccagcccattgcacatattctgattctagactagaaaccaagactccgcattttaagcaagccccacattattcaaaatagattgtccatggattatgcttttagaaacattgttcagatcccatgctttaatgttggggagtttatcctttccttctaaatattttttttttttttgagatggagtctcgctctgttgcccaggctggagtgtggtggtgcgatcactgctcactgcatcctccacctcccaggttcaagcaattctctgcctcagcctcccgagtagctgggattacagatgcccgctaccacgcccagctaatttttttgtacttttagtagagatggggtttcaccatctcaaaaaaaaaaaaaaaatcttaaatagctctagttccctgaattattttctcctaagacatgttttcccaacagttaatgttacttatttcatcttctgatcttactcatattatccacctttcacttaaattggaaattttctgccattttacaaagttcaagactttcctaccttcctacctcctggctgtgtgaacttggacagaatacttccccctctcccttcagtcagttttcttacttgtgaaatggaattaaactatacaaaatcattaggttactgtgaggcttaagagtgcctggcacatattacatgcacattaaaaatgtatttcttcccaaactaatgcaacatagcaaacaagttagttcacagtctttaatttctttccttttccctttctttttagctaatagcttttgggtcttaggctgattagaaggaatccttcttggggtgttcttctggtaagaagattgaagctctcctttatttgcttgtaacagaatgctcttcgtatctttcaaaagcgtcaaaagctggatatggaaagtataggccaggtttgatacagaagtgtagtttggcagttttttcagtatccattgccactaattcagtattttgttagatctgttgatgtacggttttataactaaaattaaaaagatttgggtacagtttataagcattattcattttaagaggatttaagaggataagaccattttagactcgagcagaatattagtaataataattagcttaaaaaaataaacatataccaatataaagaacagcacaaggcaagcaaatatctgggcctatattaacagacggtattcaaggatatggctagaatttccaaaatgcctaataatgtgtaattcttggcattaagccgccaatttgaatatggccctttaatatgaaatgctatataatgacagactttattatagtctgatccaaggcccctgaactttccaaaagggcaacaaaacagacagatactgtattttttcactagttggtactggtggcacccttttgagtgttatttttggcattacgtgtagaggttgacagattcaagacaacactaaacatgttagcagtcaccacacgcaggctgtccagcagaatgacagcgcctcccagatcctagaaagcatccagagtcactgcacccatcccctgggggccctgtagtcctgcatctccagatgatgggagctgcaaacttccctgatggtgccctcttggatgctcatgaggcctgatctggtaccacgactctagcagtaggtccattcaatggcagtaaaaatacatgttgtatgttgatcagaatttggcaggacacatgtggaaagttaatgacatcctggccgagaacccctgtgatatacactggttacatcctgtccaactggagtttttatgtgctgtttttggcagagccaagtgaagatcttgttacttagccattcctgaggtactgaagatacccgggtttttgtcattacaggataggctagaaagtagccagggtctcataaccaaggctttctctgaaacatataatgacaatgctagttatttgaccaaagatatccaatgctttaatccacttggaatttattcttgatgtgaagggtcagcatcatccactggtcgggagcctgatccttggagccaggcagacctgggttgagtccatctccgcctgtttccagctgtgggcaaggtgtctgacttctctgagcatctgtggggtttgtttgtttttaaacctgaagaattgggataatctgtttcctcacagaatcattacgcagatgcaatacagttaatgaaggtaacatggcacataggaagagcacaatacacgtcagctcttactcttcatggctagaagatgtggactaaacttccccctttacagttttgtgattaacaccatttatgaaagaaataaatgaaataaattccttttcctgtcatgaggggaacttacctgattttattgaattatttggtgccattgagttccttattgtttccctctgacctagatttctgggtgtgcgccagtaacacgactgtgattgttgctgctttataacattgtctgtggtcagtccaaacaagagtttaaaataattgaatgaaatggattttaaacaatggtccccccaccctcaccccgtggcactcggccaaaggaagaggaaaagttctctgttaaagaaaatgaatcagagaagaggcccagaccgtgcctccgaaaattctcattgtagggactaagtcctctcactctgaactcacacccgtctgttcgcagcctcacctcatatcctggtctggatgtgcggcctcaccggggtgtcgtgcgcacgtgtggttgtcctgtgggtgccagctctgacttcctccccagacacccactgcctcagccttaatcacaggacgcgcgttgagtagaaatgagaccagttagtattggtaactgcagaggaatttgcattttcaccagcgttctcgggtcagagggtttgcctggcaccgcgtactgggaaactcgccaaaagcggtgcaggttggagacgccccaggccgcggtggagttgcgcgcggcttctaaagtggagtggagcaggcctgcaccctccccgccggggctgggacggcgcttccaggcggagaaagacctccgcgggccgcgcgcggccttccccctgcgaggatcgccattggcccgggttggctttggaaagcggcggtggctttgggccgggctcggcctcgggaacgccaggggcccctgggtgcggacgggcgcggccaggagggggttaaggcgcaggcggcggcggggcgggggcgggcctggcgggcgccctctccgggccctttgttaacaggcgcgtcccggccaggcggagacgcggccgcggccatgggcgggcgcgggcgcgcggggcggcggtgagggcggctggcggggccgggggcgccgggggggcgcgcgggccgagccgggcctgagccgggcccgcggaccgagctgggagaggggttccggcccccgacgtgctggcgcgggaaaatgttggagatctgcctgaagctggtgggctgcaaatccaagaaggggctgtcctcgtcctccagctgttatctggaaggtaagcccgggccgcacgggttgggctgagtagccgcgcgccctcccgctgctgctgggcccttcctaggcctcgccgcccgcgcgctcccgcctgcgccctccccgggtcttgtcttttttttctttcttccctcttctcttctcttctcttcagttctcttatattctgtctctctttctttctctctgtgtctgtctcttttctcttctcttgtctctctctttttctctctctctgtctctttctctttctcgcgatggcccctaggcgccgccggcggagcgtggcccccagccccggcaccagccccggtagagccacgccggatggtgacggcggcgtccgggaccccacagtgcgggctcccccgaaaaagtttgagaaagccaactcgccaggccttaacatccctgggatcccacgttgtggaatttccaccgttaattgggactgtgtgttaaaaagatcgacccgtgtttgtgaaaacatgcgatttccattaagcatcatgtacacaaggagcaccactctaccatttatggatacagaatttcaagtgatctttccatctcccccacccccatcttatctacagaccacgaagaggtcttaggaattcgctctcttttcaggggaggggagcccatttaagaaggcgtttccaaggagtcccccagagtactggggtgtcatgttcgtttccttaagtgaagctcagggccaggagggcttcacttttgcgttctttctacctactctccttctctaattacatctgttttattttatttttctttcctgttgtagtctttagttttataaatggaaaaaaagtaaattaagggttatgggtcttcactttcgtagcttctaggtgggtatgaaattgatctgatttgagactggtgctcccagaccattgccttcagcagaaaggctatctgtgcttcagagatggagttgcacttggacttctctgttgttttcaactaagaatataagagtaaaaatgtggccgggcgcggtggctcaagcctgtaatcccaacactttgggaggccgagacgggtggattatttgaggtcaggatttcgagaccagcctggccaacatggtgaaaccctatttctactaaaaatacaaaaaattagccgggcgtggtggtacacgcctgtaatcccagctactcgggaggctgaggcaggagaattgcttgaacccggcagggggaggttgcagtgagccaagatcgcgccactgcactccagcctgggcgacacagcaagactcggtctcaaaaaaaaaaaaaaaaaaaaaagagtagaaagaaatgtgaagctcactttagatcaagtaggatttctgctagaatgccatgtttttctttttaaaaaagcaggagaaataaacaggcctcatttattttctaacctatttttctttccttaacctctgactctaccctgaaggcctgcttggagtcacatatgcagatcgcactagtgatgtgggtgaaacctgtttgcccttcttgccacagtttgtgtacctcactcctcttctgtctctgggattccagggggctgaatggcccagagaaggctcatctaggtggagtgggctcacagagcctagcatttggagggtggagattgtttatttgtccctaaaagttgatgtctgagcattccaaatcatcttcaattaatacatcgcttattttttccaagttgctcaaaattctgagcacattctcatttacatctgtatcgagttagtgttaggcatcatcatctccactttgcagatgggtgcctaaggcggggatgaatggacttttgtaagtgcagagctggagcaaagtttaggtcacagctttgccaagtcattgttttgttttcctgggagtaaaccggagatttagtatggacctggctggtttaattattgttttgggaaaaaaatctaaaactcattccaacatgtcttgaaatgaattataatgttgactctaaagtctcaaaaaaaaaaaaaagttctagtacagcagactgccttgggttaaaccttcttctaggaaggtgtcactctaggaattctttcttactgagttttcttcttttcgttgttatagttaattagagaaagtaaatggaattatcattttgtagttggtagactttaacaagcctcagcgatagtcttttaaagactggaagtgctatttgtcttttgggaaaaatagttcctaacatctggatgagtaatccaggctttccactttcactgacagcctaaatcagtcaatcagtgtcgatcagtcagtcagtgtttattgacgcccactcagggtcccaggcattccctgtcagggagagaattgaatgagatcaagtttttcattgttctatcaaagaagcttccaccataaatgtggtttgatggtgcatgctacctgctactcagcctagctgtcaaagcaacactggtaaacataaagatggctagcaattattaaatgcttactatgtgccaaatactgttttattactctatgtgatctgatatagttatatttcatgatagcactatgattatttccattttatagatgaggaaactgagtcaccaaaaggttaggtaacttgtctagggtcacagagccagtgagtgggggtactggaatttgaactcatgctatctggcttgggagagcccacttttagccactggatgctctactgatgtctcttttggaattcactgtgattttcaaaatggtatctccagaaactcctccaattaatccctgaaatgtaagggtagtctctttttcttttctagaaacctgatcctggcaaaatgattagctttaacagtaggattaattttttttaaatgtatataaaaatacttgtatgtaagaaatcctaaaagggtatttagtgaaaagtaattccctctcctattcattttccccacctagaggcaatcaccctggagttttatgtgtgtccttctagaaatactgtgtgcacatataagcatttattataacatgtgaattttgctctccagctttttgtgaatatgcatgtttatagcagtatctattcaccaggaccgcatttagctttgcaatattcggtctactttgaacactgaattttctgattatttctttcccctggagacgtcaaagaaaacatgaacactagccttttgaattcagggttttcttttcattttattttcatttgttcatgtgtttgtatttacatacattgtgcctgaatattgtacatgtatgtgacagttgtgtactgtagaatcaaaaactaatgtctgtgaactgaactcttcttgaactttttgttgttgttgttattgttgcttttggagatagggtcttgctctgtcacccaggctggactgcagtggcacaatcacagctcactgcagccttgagctcctggtctcaagcaaccctcccacctcagcctcccaagtagctggggctgcaggcatatgctacctgactaattaaaattttttttttttttttgtagagacagggtctcactatttttactagtttgcccgggccaagccagtgttgaactactggcctcaagtgatcctcccaccttggcctccccaaagtgcatccctacaggcatgagccactgcactcagcctgaactttcgaaatttattttaagggcccacttttaaatgcttcttttcagcagctaactttccagcggatgcttcatgtggtgccagccatacagatacgcttttagaacttgagctttggagaagcttatgcttgctttctgctctctcctgaggtcatcagatacttcccttgttcagtaacaaagaaagtgagactctttctgttacctaataaaaggccagtctgtccatttcattttgggtgctattaacattgttgaccatttacaatgtcacaggccctggcactgagcacatcatgtgcagcctcacttaattttcacaccagtgccctgaggtttctagaaaagaggaagggccccagtttaggtggcagtacttttcaatttggaggcaggagatcccagttttcctctgacctctctgagcttccgtgtttttacctctaagacagagagaccaatctctgttcagccaccttagaggattgttttgagggtctataagatgattgagggaaagctctgaaactggtaagagttaaatgtatgtttgtgttatgttgatacgagattcctctgagatgctctttagtccaggcaggtttatggctcacacagcgttcctagggtctcattcttctgcacaggcaggcagctcccgagccagccagtctggacccaaatgccacctgtgctcttggctggtcttgcgcattcaccgaggctcactgtaccttggtgttcccatttctaaaataaggcctgtagtaatccctacctcactgagttgttgagagacttcatgtaaattgtttagcagggagcctggcacagaacaagagcctagcagaaaagtaagctgttgttactttaagcaaatatttagcagcctaaaatggtggctttaccagtttctgtaatggttgaagtgatgacagaattcagccaatcccacccatagtttttcttgctaataaagcagtttgtttctaagtgtgttttgatgcgtataattaatacttcctgtccttgatttttggctgaaaaatgtcttctcttcctcgcaccctctgttattcccgtagtgaatattttcattgtggaagagaaattcccattggctcatggttggcattttatttctcctgtccagagacaatatttccacagcctcaaacgtgaaaactgaaaatctggtgccacttaccaccttgtaaaatcaagtcattgtaattgtgccagtataatcattgatctgaaataaaagcagaaaataaatcaatgggtagctttcttaaatacataagaactaaagatcaaatgggatattggaagactttaacttttcctccataatggtggatcttaattaaacacacagaagaacaatttataaaataaattcataggtttgtttgttcttttttagtgtcaatttttaaaactatctcttttttaattaaaaaaaatagagatgggtctcactatgtcgcccaggctggtctcaaactcctgggctcaagcaatcctcccacctcagcctcccaaagtgctgggattacaggcatgagccactgcacccagcctaaaactgtctcaaaagtagacagcataatgaactcccatgtacttatgatgtggctttaacaattatcagcttatagtcagtcttgttttcttacataataaagttacagtttcaaagccattaggaagaatagcttgctaattataattacttagttttgatagtgtaactttgtcctcagatgggtagaatcgttactctggaacaggggtgtccaatcttggcttccctgggccacattgggagaaaaattgtcttgggccacacgtaaaacatactaacgatagctgatgagctaaaccaacaaaacaaatcccacaaaaatctcatttctttttttttttgagacaagagtctcactctgtcgcccagactggagtgcagttgcacgatctcagctcactgcaagctccgcctcctgggttcacgccattctcctgcctcagcctccctagtagagggtactacaggcgcccgggggtttcaccatgttagccaggatggtctccatctcctgacctcgtgatccgcccacctcggcctcccaaagccctgggattacaggcgtgagccactgcaccgggccaaaaatcttataatgtttttaagaaagtttgcaaatttgttaggccacattcaaagccgtcctgggccatatgcagcccgtgggccatgggttgaacaagcttgctctagaaattggttttcaggccgggcgcggtggctgacgcctgtaatcccagcactttgggaggccgaggcaggtggtcacctgaggtcaggagttcgagaccagcctggccaacatgctgaaaccctgtctctactaaaaatataaaaaattagccaggcgtagtggggagtgcctgtaatcccagcactttgggaggctgaggtgagtagatcacttgagaccaggagttcaagaccagcctggccaacatggcaaaaccccgtctctactgaaaatgaaaaaaaaaaaaaaaaaaaaaacttagccaggcgcagtggctcacatctgtaatcccagctactcaggaggctgaggcaggagaatcacgtgaacctgggagctggaggttgcagtgagcctagatcgcaccactgcacttcagcctgggcgatggagtgagactccaactcaaaaaaaaaaaaaaaaaaatttcaattggcttctattaaagcttttttatgtttgtcattgttttctagtaataacaacaatccacattttttgtgagaaatataccataatatagagaagtataaagaaaatgtaaggccagacacggtggctcacgccgataatcccagcactttgggaggctgaggcaggcttatcacctgaggtcaggagttcgaaaccagcctggccaacatggtgaaaccccatctctactaaaaatacaaaaaaagtagccgagtgtggtggcgggcacctgtaatcccagctactcaggaggctgaggcaggagaattgcttgaacccggaaggtgaaggttgcagtgagcagagatcacgccattgcactccagcctgagtgtcaagaacgagactccgtctcgagaaaaaaaaaaaagaaaagtaaatttaaagcacttaaaatcccaccaccctgagttaactactgttcacagtttggtgaaattcctcctcgtcttctattttttcatagttgggaccatgcctatatactggaatgtaatataaacacttaatatattattgcgagtatattctcaaacttaaatattttttccaaaaatattttgagtggcttttaaaatatatcctattttatgcatgcagcataaactaacttatcctgtgttgatagatattttgtacttgcccttttctgtgctgttgtttaaaattagtgtatagaaataattgtgttgatcacttaggataaattcctagaggtaaatcagatattaaattctttatagacttctggttcatattccagttgccctcaatttatacacctactactagcattgtatgagagtgcccgtttctctgaaatcttacccacactggctgtcagcgtcaaaaagatgtatctgcagatttggcaaggaatttgcatttcagtgattattatcaagcgttcacacactttccatgtttaatggtaattttttttgtttttttttgagacgatgtctcactctgttgcccaggcagagtgcagtgccgcgaccttggctcactgcaacctctgcctcccaggttcaggtgattctcctgcctcaactccttagcagcttggattacaggcatgcgccaccatgcccggctaatttgtgtatttttagtagagacggggtttcaccatattggccaggttagtctcaaactcctgacctcaagtgattgcccgccttggcctcccgaagtggtgggattacaggtgtgagccaccgcacctggcctttaatgataatgtaaattttttgtgaattgtttattcgtggctttgccccattttttccatagtggagggatttttctttttcttgttggtatgtaaagtccttgtgtgtcaagaatgctctgcctcacagtttttctaatataatgacagtggaagctcgtaactggcttccacttgactgacttgctaaattgaccggcactcttcacttccttataaaacatgcctccatagtccctgtgccccatggcacatgggatggggtagccacactaccactgtctgctgctgcatatgttcctgtccacaagagccagtcatgtttgtttccaagcctggttctttcagatatagctgttgttgtaattacttggttgatatgaaaccaatgaaatgcaagtgtgaaaagagaattgtttctaggaaaattaagatgaatgctttagaaagactcagtaaaggaagataaatttaacaaattactacagaattaggtgtaagacaacagtaaatgattggaatgaattacagaaatctagaaagctttgacagtgggaatgcgtagtgaatggctctaagttctccctccatctgtaggaaattgaagctggaagtgagatgatatattcattatagggaggacttacagaagaaaacatcaagctctaatcacatgtccacatttcgttttgtttacttattttttgaaatggagtctcactctgttgcccaggctggagtgcagtggcatgatctcagcttactacaacctctgcctcctgtgttcaagcgattctcgtgcctcagcatcctgagtagttggggctacaggtgtgcaccaccacgcccaactaatttttatatttttagtagagacggggtttcgctatgttggccagcatggtcttaaactcctgacctcaggtgatctgcctgcctcggcctcccaaagtgctgggataacaggcatgagccaccgcacccagccccacatacctacatttcaaaggacagtctttggccctacagtcaagactaccaaaccaatgtacactaaatgggggtggggatcacgttgttgttttttgtttgtttttgtttgtttgtttgtttgtttgtttttttgagagagtctcgctctgtcacccaggctggagtatagtggcgtgatctcggctccctgcaagctccgcctcccgggttcacgccattctcctgcctcagcctcccgagtagctgggactacaggtgcccgccaccacgcccagctaatttttttgtatttttagtagagacggggcttcaccgtgttagtcaggatggtctcgatctcctgacctcggggatcacatattttaataaaattgataatccctaatagtgatggcgctaggtgtacttttagagccaatgtaaatagtcgagaaagggggccaaacatatgactaagcttcttctacactctaggagatgtcagtattgcaagatcctgttccttgaaattatctttgccccccgccattcagaaaaattaccaaatattgtaataatgtaatttaggacttaccctttcagagaaacagttcctgaaggttgacttcagttagtagtacagaagcgagacttgaagctcttcatggtttatgttctgttggtttatcccaaagagatgttttagagcacattcatttctgaaagttctcggtcatgtttccggaagtttgatcaggtgggttctttttctttttttaaaagataattttttttttaaagataattcagaatcagtcccacccctgagatggtattattacccaggaaagaatgcgtgaggatcctctaaatccatagagaaggaaaactaaaacaattttgttaccatttgtttggctcaagcatctggtagatccttcagttcttttcaaattagaattttcctctctttttcttttttttttttttttttgagatggagtcttactccatttcccaggctggagtacagtggcacaatctcggctcactgcagcctcacctcccgggttcaggcaattctccggcctcagtctcctgagtagctgggattacaggtacccgccactaattttcatatttttgcctggctaatttttgtgtttttagtagagatggggttttgccatgttggccaggctggtctcgaactcctgacctcaggtgatctgcccacctcagcctcccaaaatgctgggattacaggggtgagcctccacgccgggcctctctttttaagataataaaaattactaaacatcataatgacatgatttgggattactctttcagagaaacagttcctaaaggtttacttcagttagtgatttttatttttattatttatttattttttgagatggagtctcactctgtctgccaggctagagtgcagagacgagatctcagctcactgcaacctccgcctcccagactcaagcgattctcctacctcagcctcctgagtagctgggactagtagctggaactacaggcgcccgccaccatgcccggctagttttttctattttagtagtgacggggtttcaccgtgttgcccaggttggttttgaactcctgagctcaggctcaggcaatctgcctgcctcagcctcccaatgttctagggttacaggcatgagctactgtgcctggcccagttagtgatttttaaattgtagttccttaaatgagtattttggatttcactccacaatgttcttcaactgtaagatctacttgaggttatttgatttgctggtttgcaagaactcgtctacacgttgtctttatcacaaagaaattctggagcatttgagccctgttcaaaaaaaaaaggcaagaagaaacttcaggaacaaataacctatttgaccctgtaatgaataatattcacacattttctaatttaagagctgttgattgatttccaacttttagaatctgtttcagacaaaacatggaagtttagtaacagttttttctattctgtaataataattgccacaaggttaaaaaaaaaaatttacagaagaacatatttgagggtggtcgtgggggcaagaaagctggaaggacgggtggggtgtgttaatagccttgtcttgtgaagtaagtcctcagagacgctgtcctagttggaagaacaggcagtgaaggtgtgcgtctgttacggagaataggactccagtgatctagctggtacttagagaggtgggggtgatcaccaaaaaaacagctctgcctctgggagcggagaggactgggatagaaagtatttgtctttcattttaagcccttctgtacgatttgacttttcttttttttttttttttttttttttgagatggagtctcactctgtcacccaggctggagtacagtggcacgatcttggctcactgcaacctccgcctcccaggttcaagcaattctcctgcctcagcctcccaagtagctgggactacaggcacctgccaccatgcccggctgatttttgtatttgtagtaaagacaggatttcactgtgttggtcaggttggtcttgaactcctgacctcatgatccacccccggcttttttttttgacacggagtttctcgttacccaggctggagtgcagtggcgcaatctctgctcactgagacctccacctcctgggttcaagcgattctcctgcctcagcctcctgagtagctgggactacaggtgtgcgtcaccatgcccggctaatttttgtatgtctaatggagacagggtttcaccatgttggtcaagttggtctcaaactcctgaactcaggtgatccacccaccttggcctcccaaagtgctgggattacgggcgtgagccaccatgcccggctaaagcaagaaattttcattgcatattttaagcaaaggcaaatgcatatgtggatagactgttttaatttgactaaagtcatattgaatccatgaattttagaagctcaaactattggggaacaataattaccaccttggagtgaaaatacttaatttccacaagatttagtaaaggaagagttttttaaaaaccaccttaatgataatagtatgtacagatgttaagaaatgaaataggaatgtgtaatgttggaaacacaaatatttttgcttctgagaataaaactaattttttctcccaattttctcttcctttttcttttttctgttcccccctttctcttccagaagcccttcagcggccagtagcatctgactttgagcctcagggtctgagtgaagccgctcgttggaactccaaggaaaaccttctcgctggacccagtgaaaatgaccccaaccttttcgttgcactgtatgattttgtggccagtggagataacactctaagcataactaaaggtaaaagggttgtgggcagctagtggtggttgcaggagatagaaatctgggaattgcggtttgacctaccaccctttgctcgttaaaggagcagctttgaaatctggactgcagggatatccaaaacaacaactgcatgtttctaagggagtcgactctccttagaggagttcttgtacaatagccctgggcaaaaacagaacttgccctattttttatactgaaaaggacagctggacaaaatactgaacgcaatttttcccctaagaaaaagcattatttccctaaaatgtcttatattaggaacagagcacttgaataaacataattgatttataaaaactgaggctatacacttacctatctgttcagtacaaacaggaagcttcaaatgtaaacgtgaattctcatacacttataaatgcatatctttatgtggacttgttaaaatgaaattggtatttaggaatttggagatttttagtagttacacaagaatcaatgaaaaagaacgaagctggtttccaaagctgatatgtctgatttggttcctttcttctcaggtgaaaagctccgggtcttaggctataatcacaatggggaatggtgtgaagcccaaaccaaaaatggccaaggctgggtcccaagcaactacatcacgccagtcaacagtctggagaaacactcctggtaccatgggcctgtgtcccgcaatgccgctgagtatctgctgagcagcgggatcaatggcagcttcttggtgcgtgagagtgagagcagtcctggccagaggtccatctcgctgagatacgaagggagggtgtaccattacaggatcaacactgcttctgatggcaaggtaggggacccttggcagggggcgctgatgggcccagggcaggggaaccagaggtcctgctgtcggattgataaattattgcaagaaagctcaaccaagaagatgtttaaagaatctttcaggtgggagtcattccattagccttatgaagaccctttattgaggatccgttctgtgatattacaagttcctgggactggtatgattctcttattgtcttgctagagttttgttgttagcaagttacttaaaataggaggaatatctgttgggttttggacacattttttacaataagattcttcctttaaaaaaaatattttataatgatagaaatcatccccaacgagaaaaattcaaataatagataacctttcttagagcgaaagaccactttactatcccctcccccacagacgcctggcacgtgggcttcttcctgcggatgaacacattcatggagaggtgtgtggacatacgtgcatacacgcatgcagttttcagtgaaaaccgggatcaaacccacagcttaccaaacccaaagtgtggtgttgtaagggaggtggcctatatgattttgtggtcttcatataaataatccttaagagtccataaagagaagggaggagttaacattgactgaggtattgctataatacctgcatctttgcattaaagaaagggaggcataaagagatcttgcccgatgtcaacctagtgagtcactgatggaataggcttggatcccacagtttattctactgcaccaggctgtagttgaggtacagtgttgataggtggtcccgatggtgtatgtttgtttgtttgtttgtttttgagatggagtcttgccctgtcacccaggctggagtacagtggtgcgatcttggctcactgcaacctctgcttcccatgctcaagtgatcctcccaccttagccttccgagtagttgggaccacaggcgcacaccaccatgcccagctgttttttgtttgtttatttgttttgagatggcattttcgctctcattgcccaagctggagtgcaatggtgcgttctcggcttactgcaacctccacctcccgggttcaagcatttctcctgcctcagccttccaggtagctgggattacaggcatgcaccaccacacccagctaattttgtatttttagtagagacagggtttcaccatgttggtcaggctggtctcaaactcctgacctcaggtgatccacctgcctcagcatcccaaagtgctgggattacaggcgtgagccaccacgcctggccgtttttgtatttccagtagagacagggtctcgccatgtcgcccaggctagtctcaaactattgagctcaagcaatctgccctcctcggcctcccaaaatgctgggattacaggcacgagccactgtgcccagcctatattttttaaatagtatgtaatgcatgcatatggttaaaaaaaatcaaaagaacaaaatgaattacagtaaaaagtaatcgtctcctaattcacttttcctgcccagaggcaagcactggtactagttccttctagagttacctggacacagatggatggtatatagatgtttatgtggatgtttatattcaaaaaggcacgcaaatgatacatgcacgcgaatgcatcatgcttctcccgtgtgataatacaccttcgagattgttttatggcaacaggtttagagctgcctcattcttaccagtgactgtgtaccgtggatggactgtcacttatttcagtagtcccctgctggttgacttttaggttgtttccaatctttagttattgtaaataatgctgatatgaggtggctttcaaaccttttcaaaaatctggttctgctgtaagaaaaactcattttacaccaccacccagccctcacaatataacaaaagtttcatgaagtcttacctacccttactgtatgtaacgcactctgatagtttgtatttcattctgttctatttcattttttaaaaattctggttgtaatccactaaatttatttcatagactgactagtggcccatggcctggtttgaaaatgcgttgcacgtgcttctttatgtgggtgtaagtgtgtgcagataagttgccagaactgactgaaggttatgtgcatcaccaggtcaccctctatagaaattgtacaaatttgttctcccacaaacaatccatgaaagggcttgtttccccttaacccacaccaacagtttattattagacatgtaaaaacacctttgtcactctgactggtaaagaatggcatctcattatgttgaatatccatgtggcatattttgggtcatctttatgccatttagtaaattcatctttttcctacatgttagaaatataccaagtgtatatgtgtatctaggcctgttgacctctctgttctcttccattggtctgtctatccgtatgccagtaccaaacttgtaattgctatggcttcataccatgttgtggtatctgataggctagtccccacttacctttttaactttttttttttttggctgtcttcacacattcacttgtaccatatgaacatacatatacttcctttttaatgttcttatttttcttcacatcccaaagtcttctggctgaaatcctattgcccatatctgatgctttccaccactgcagaattctttagtaccaacactgcagtgtgcgtgacggacaaaagagcctgttatccctgtgtgactagacgtgggcctgtcagcttgctttttgggttattgttcttatcccagaggtggagctgcgttcttccattctgagggacgtacttcaggacattgggccctttgaaagagccttcagaccacaagggtacctttctagtgaatcagaacaccagggtgcaccgcccatggggggtgattttctggagcagacagcttgcttcccatgtgtgctatttatccaaggcaagtcatgctgcaccgagatagtcacttgaggtttgcaccgaacaggataatggtttcttttccctagagctgtttaatcagcaaccttggaacagatgcaggcaggcatgatctagtgtgacagctcattagctaggggttgatctaaaatactgttcaaatgggcaaggaaaggcctgcgtatgggatatgtgatttgcagaatttgagattcatccaaagagggagaatctgcctaagatgcctctgtctaaaagctagtatgtgccaggtgggtttgtttcattccaggtagagcacagggagcttatgtgaccaggcagtgtccaccattgggcaacacatcacacttcccttggcgtcttgcctcctccctccccgtctggcacagactctcccatcagccgtttgggcacctggggacttctgagcccacagcgtcatccagcagaccgtctgcggaggttccttcctgtgagggccgcactcgagggggtgtattgggtgggatcgtatcactggaatgagtgaacatcgttagagggagctcccacagctatgcgtgtgaccgtgtggctcgccgctgaaaaatgctgctcacatagcagaacttcgatgcaatcctttttggatttctaaggggaaattttaagaccgataggaggaataggctggggttgaataagtttggttcttatttttaaattagctcatctttagaaaacaactgaatttagaagattcttctgtaaggccccaaaggatttctttctgcctccccgctcttggctcttatttgtgtctctcctcgtgttctgagcttttcagcagcccttgtgggtcatcagccgaggaccatcagctcggggcccagagctggggactgggagttatgagctggactcttgaaggggccaatactaaaccgagccgttgccatttcctaggagccttgacaggctcaaacatctctgggtacccggggatttgactgtcattgttctgatcctttcccaaagttgtaaccctctgttgacatagcggaattgaagattgatttttcttcaccaccttctgcctaaagttcttagttctgaatgtgtccacacctcattgacttctatgagatgcccctgtcacgttcctcgattccttctagtccttaatagagtctttccttttcttgaaagaaatttgcccagttgacatttattttcatcgtctgctgaagtgacagatccaaggccctaagcttcagcagagttgcaggaagggaccatttacacagcctcttagatgtttaaggtttacccgccctgacagtggctcagcaggcgtaggcctcctggtgaaaagccgagcacatggctaacctgctctggtggaggggctttggaccgttcttgtgtactgcgaggcttgccttcctgctggtgtgtgagcagctctcgggggaacttgcttcctggctgagcaacctgtaaacagtatgtctgaggtgggactcccgggcccaaagcagccaaaggttgcacaagtctaagctccgttaggcctgtcagtgtggctgtcaaaagaaacgctgtttcttttctttctttcctttttttttttttttttttttttttttttgagacaggctgtcacccaggctggagtacagtggcacaatctcggctcattgcaacctgcgcctcccgggttcgagcgattctcctgcatcagcctctcaagtagctgagactacaggtgcccaccagcatgcccggctaatttttgtatttttagtagagatggggtttcaccatgttggccaggctggtttcgaacgcctgacctcgtgatctgccctccttggcctcccaaagtgctgggattacaggcgtgagccactgctcctggcaaaatgctgtttctaagcgtttctttgacaagtcccatccttcaggttcatgcatgattagggagaggcagcagccctgactgagcacctgagtgttcatggaaccaggtgcatagcgtaatgacatgccattcatgacactactttcttccctgaacatgccatgaattcctgatgattacacagttccccaacaagtgctgctcaaaacctggaactaatcagaaggaagcaccagccttgactgttagtgggacacggggaagatggctgtgaaccgaatatgcggtgcctttgggggagaatggttttagtatttagtaagtgtcagtatgtaagttttatgttgaaaaatgaactaagtcacaacaaggtctataaatttaattattgaaaaggataaagttgggccattcagtgaaacctcctgtaactgaagtctctaacacagtagccaatgggggaatcaaatgagcccaagaagaaattctgcgtaaactaggacttaggggagcccttagcattccactttggagtgaaggaacccgatccgccagttggggaacgctcctttgaggcccatgtgcttcctgctccgacgggagagagggataatgagacttgctcccaggtgccctgccctggagcccagcaggccacacgggctctttgactctgtactgtgccagtgatttccaagatgggagtggtgctctgattgcaggaatgtcttcttggaatggcttttctcacttctctagagtccttggtagggagcacatcatcagctgagctaacgtgagaacaggggttggagcacttgccaccggcagtgaagtaatcggacagctgacagtcttttccagagggtcggggattgggagctgaccccaggtcccgctccgttttctttgtgtgcagcacttgtgttggtgaccagcagtgaagagagtgcgtggacgtcaccgtgtggttatgaagctaacggcagccctcagcggtgccgacttccgctccccgacacattcctgtgtgcacgttcgtgggtctgagcgtgactcatggtgtgtgtccctagagcagttcactcagaggcttctcttccgtgctctcaagaataaaagcagggccgccacatcctgataagtcttgccattcagcggtcctgtcttgcagagggataagccagtgtccccaggccacagtccttacaccttgagcaagttccccagagtgaagcaatctttctagacaagttttgcgtttctcagaattttattttagtgatattgttaccaaaagattgtaaccccaaaatgtgtgcctttggcttgcctgttttaggaattcacttgtgttatctccccaagcaaaacaaaagaaagagaaaccttcctgttgacgaatcctttttaccttcttgagagttgtcaatgggactaacttgtatatttctttgctaccttcttttaaaaacatttttcttatttactattacagacgtatagtaatggtgcctgacataacccacagccaaaggccttggccttgctgtgtgtatttcaggctttttcttcccttttctttttttttaagtaataagatattacagttatagctgaagcctgatcctgttcccttttctccctctcgtcccaagcatcaccactgtcccaaatctgctccttcttcccacatctttgcagtttgggcaagtcttctgaatgcctagtcatgattttaagtcttctttccaccttcagtgatggttggctaccctgagcaagccagtagattcagttatgtgcctggagtccagatgttttatgtggatttttcatgtggaattgtttttggtaaggaagtattcccttgccacaccaatgaaaagagaagaaaacaggtagctggcacccactgcattgttgctttctgccagcctgctccttctccttcctctccagctctgttgtgtccagatgcaaactctacatgcagggtttgaccctaggtcctcacctgctgtagctctcacacggggaccgaatgctcttgtgtcgtaaatccttccttttgcttcctcgtgttggatgtgtttagtggttttcatcttctggtcactatttcattctaggtttatcccctttaaattataaattaaatgaattcttcgcttttcctaccagcaactacccaccaagttctaccatgtgttaatttaatcaacagttatttattgagtacttattacatgttgatttcctgttctcaacattggaatgaagacagcttagggttctgctttcatgaagcttgcatgctcttaggtggagacagacagtaattaagcagataaacaggaaattatgagctagtagtgggtccattgctgagaagtaagacaggtggtaggatgacccgtgccgtgtgatgactttagattgggtggttggggaagacttcacggaccttaaaactggccttggaacgggaagcgagaactgggcacggaagatgagggagtgggagatttcaggcagagggagcagcagcaggtacagaggccctgaggccttttattgtgtctttttgcttgagcgagtaacttagagcacacgtagagaaagacagcagaagtgatcttctaaacactctgtcctgtgtggagagctccttatgtgagattttgctgtgtagtgaattaaggctcagccaaactggctcacgtgagctctttgagcttgcctgtctctgtgggctgaaggctgttccctgtttccttcagctctacgtctcctccgagagccgcttcaacaccctggccgagttggttcatcatcattcaacggtggccgacgggctcatcaccacgctccattatccagccccaaagcgcaacaagcccactgtctatggtgtgtcccccaactacgacaagtgggagatggaacgcacggacatcaccatgaagcacaagctgggcgggggccagtacggggaggtgtacgagggcgtgtggaagaaatacagcctgacggtggccgtgaagaccttgaaggtaggctgggactgccgggggtgcccagggtacgtggggcaaggcgtctgctggcattaggcgatgcatctgcctggaagtctacctcctgcctgctgtccgagggcttcattggcgccacggaattgacttttccgtcttatatcattcctgtgtctttgtaggagtggaatcattctcatagtccgagtgtgtttccacatatggtgagagctgacaagcatggaggggttttggtgtaaaaagattagtcatttggagaggttttctcattttatggcaaggttcttttaaagccgtggatttccatgctgttcgtgcggcatggagatcacttcctaccgagagttaaggaggaaaaaaagatctctgagttttgaaagaagatttaaccaaaatgcatttgactcttctgtggatttttgttggctgatttggaaggcaggtgccctgggcatccccagtgggttccaattctgcagctgcccagactcctgcaggcagaggtggaagtgtccccgctagaaaggcatccaggaaactcgcttttgaccaactcagatacagtctggtctttcttgttaactgggactttaccctctccactaatgaatagtgtttgtagtttccaggcaggtttttttcttcttttgaagttctttgaaacccttaggacgccaagggaaggaagttttcattttcagccctttgcattcttcaaaatgtgatccaggcttttccctgtggcgagggtgtcccctagtgttgacttacattatttccacttgttttaaatgaactttgattaccttgacctgtgcacagaaatcaagagaggcagcccctttttagagctgttagaaaagaactgaaacatccacctctgggaaaaatagagtttagtttgtgcatgtgtctcagaagtcaggtgcacacattgagactggtgcagccacatgcctgccttttagggactccttgactgacctgatgccttcacccaaaggcatagtgaaatgggaagtatgatttctgactggtatgaagtggctgctttagagaaaagatcacattctttagtcctagaaaccaaaggtggcttcctgatgctcttattcagcacgtgcctgtctttgaggcaggactggcactggggtgggggcatggtttggggttaccttaaggaccctggatatttctcagataggactttttcttttctttttttgagacggagtcttactctgttgcctaggctggagtgcagtggcatgatctcagctcactgcaacctccgcctccccaaattggcgattctccttcctcagcctcacgagtagctgggattacaggcacccgccaccacacccagctaatttttgtatttttagtagagatggggtttcgctgtgttggcctggctggtctcaaactcctgacctcaagtgatctgcctacctcagcctcccagagtgctgggattataggcatgagccaccacacccggccctggactttttcttaattgaataaatatttatcaagttcttcacttctatttgacggttcctgggctcaacactggattagaaaatgaatgggacagagttcttcatctgagacatagggtggtccaggtagtaggaggaagaaggattgcagcgcagcagtcctcgggacaccaccagggggtgaacgaaggagggacgggggagctgtgcaggtgccccagctccttgggttgcacagggttgaagaccagacccaagaaatggggccttgaccagctcagcaaactgagaatggcctagatttcagcacactttcaccaggatttgtcaaatgaaggaagattccaagcgcaaaataccctagatttcaaccagtaaaagcttgtctgaaaacttccaagatcgggttgtacaacttgacatttgaggaaacgctacttcagtagatggtgctgtggcattgttttctgaacaactgaaggaggagactccagagaagggtacctgctggagacctgtgtggtttgtggggtgggtttcttatatcactgaatctaaagtgggtgcctttcagaatgtgctttactaataatgtgttactctgcttttaattatacttctaataattttccccaagagcctaattaacttacgatctcacagttggtaaagaattacaggatgtcattgcgtggatttctgtgggcagtcacccggagtggtatctaattagggaaaaggcagtatgtccctttctggaagtgtgttaactgaaaatacggtactaagcaactgctaaataaattagccctccttcctcctggccgtgcgcagaaacatccctgcagtatgttgcctatttgtcaaataagattagtgtaaatatggggcatttacctttgctatagaagctgaaattgccaggcacggtggcttacgcctgtaatcccagcactttggaaggccaaggctggtggattgcttgagcccaggagttaaagaccagcctgggcaacatggcaaaactctgcctctacaaaaaataccaaaaatcagccaggcgtggtggtgcgtgtgtattcctagctacttgggaggctgacatgggaggattacctgagcccgggaggttgaggctgcagtgagccgtaatcgtgccactgcactcctacctggggagcagagtgagaccctgtctccaaaaaaaaaaaaaaaaaaaaaagctgaaatccttgagtggattctaaatcatggcagtggctaacattcagcttcatcgtgcccttgctgtgtgcctggcagagacctctgtgcttactacatgtcgcatctcattgaatcctcacaaccttaagatccttccaggttgagcatcccggaccctaaaatcccaaatcctaaatgctcccaaatccaaaactttttgagcaccggcatgcagctcagaggaaatgcatactggaacatttcagattttggattttctaatttggagtgctcatctggtaatatagtgtggatattccccaatctgcaaagatctgagctccgaaacacttgtagccccaagcctttcagttaagggacattcaccctgtatcaacattttaatgctgagaaaatggaagagagagaggttaagtgactgacctggcatcacacagccaggagtggcagcatcaggatttgaactggggcactcagctccaaagctcagctcttcttttttaaaattgaacccagattcttatttctcaaataccataaaatatttacataagccacagttatgccttttaaaaaaaaatcaccttttccccccactctcccatttacttcctttgcagtttgtggctacgatctaccttcctcttcaaaacccttgaaaaatccttgcagccttgcccaagcgtccttccctcagccgatttttgggcctcagtttcctcccatccagcctgtttcctatcgctggcttctccaagggcagagccagagtcctcttttgccagcagggggagcaagggcctacttttaaccgcaactccatagtgaacaagtcaagcaaccttgggtcattcatataccttccaggcagaaggaagacagaagagaacaggaaaaaagcaggacactaggctgacccctgcagatgggaagctggaattacagcaaaggctcattgattgggaactgcacccttgaattttgatagtattgggcaggacatagtcttgctatctgtgttaaagggaggacgtgcttaagaaaaccaacagtcaagtacaagaagctctaattttttttgaggtgggggaacggggtctcactgtgttgcccagctggcctcaaactcctggctcaagcagtcctcccacctcagcctcctgagtagcagggatcacaggcttgtgccactgtgcccagctaagaggctgcaattttttaatgaactgtattcagagtttgtacatcagtgtcttttttttctatgaatcagttctctaagtaatagaatttggaaaagaccgctggtgatctagctgtggcatttagattgactcatgagctaactgacaaatttactacttaaacagtggaaaataatgtgcaggatatatttttttgaataggttgtcccaccctcgagttctgtgtctttcctgagtccgcatatgtgaaccttgttttaaccaggtgacagcatcccataggcacggatctctgtcttctgttgtccacatcatgtgtcttggcagttgttccttattgatatacataaggttgtcttgtttttgtatggatatattttaacatgtaccagtgttcagtgggcctttctcttatttccaatattttgctgttctaaacagcagcacagtgattcccctcatttgcatgtatgtgaaactatcctggtgggtccgcttccagaaactactggatcagggaccatgtgcatttatggccttgaccatactgccagagtaccttccaaggagtttgtgtcatcaatttgcactccccagtggtgttgagagagtgcctgtttcctccacccagcacagtgtgtttcggttttatttctcccaggaaatgggtgttagttggggagctccagaaagaagccgagaagaagggcagtcgtacccttggcagttgtacgcagtggctctctggccgcacaaggagggctcggagcctgctgttgccaggttgcacttgctcttgcaagacaggcattccttgcagtgggttctcctctggccagggagatgagttctgggggctcctctacgaggtggtctctcctgggctttcctctcgagcttcaagtcccacctctggagtgtgaatcgccttcctcagtctaactctatccctccagtggtttttttttttttgctttttgtttttgtttttgtttttttgagacagagtctcactctgtcacccaggctggagtacagtggcgtgatctcggctcaccgcaagctccacctcccgggttcaagcaattctcctgcctcagcctcccgagtagctgggactacaggtgcctgcgaccacgccggctaattttttgtatttttagtagagacagggtttcaccatgttagccaggatggtctcgatctcctgacttcatgatctgccctcctcggcctcccaaagtgctgggattacaggcgtgagccaccacacccagcagtctcttcagtgtatttagctgtgttgatcctgattcatctgatgggtgaaggaatattggaaataaggataatccctgtggtgtttcactgtgcctgtaacctctctcacctagcatttggttaaccagaaacagatgtggaaactgatctatctgtagataatggccctgctcagggagggggtccctgctgagagcgagacattgaaagcctgctacacagaaactgctggaaggccaagccatttcttttttctttttctttttttttttttttttttttcagacagagttttgcccagtagttcaggctggagtgcagtggcatgatctcagttcactgcaacggcctcccaggttcaagcaattcttctgcctcagcctcctgagtagctggcattacagactcctgccaccacgcccggctaatttttgcatttttagtagagacacggtttcaccatgtggccaggctggtctcgaactcctggcctcaagttatctgcctgtctcggccccccagagaggccaagccatttttaaaaacagtgttctttttcatgctgtagaatacctgtgcttgggggtgagcaaaaaggaggaaactgattagaaaatacctatgagggccgggtgcagtggttcatgcctgtaatcccagcactctgggaggccgaggagggcagatcacaaggtcaggagatcaagaccatcctggttgacatggtgaaaccccgtctctactaataatacagaaaattagctgggcgtggtggcaggtgcctgtagtcccagctactcgggaggctgaggcaggagaatggtgtgaacctgggaggcggagcttgcagtgagccgagatcgcgccactgcactctagcctgggcgacagagcaagactccgtctcaaaaaaaaaaagaaaatacctgtgagatgttgagtctgggagaatgtatctgtgagaagacaaacaaccctagtattcattaaagaaccagcctttgttttctacaagctatctgttcggtctactcaggaatagagataaactgccttaatagtaataaaagcaagcaccgctgagtgagtgctggcctcatgccaggaactgctcttggcactctgtgcacaagggagatactgacattctttctgttgtgcagatgagaaaacaggctcagagaaggtgagtaacttaccatggtcacacagcagcagagctaggtcagtataatccacaagtcattctcttaaccgctccgccgtaccgcccagaatgttcatctgcatctgggccagcctcgtcagtccgtgcaaagaggccagttgacccatctccctccctaacaagcacagaagagaccaggctgaaaattcatagctttcactcaaagtgtttccttcacctcattcatctgagttagctttattttactatataaagagaattttcttcagcaaaatgataggaatttttttaatgaaagtaaaggaatgtcacagaattgcgtcagggatatttccagtttaacacaactacaaacgtaggctgttttgttgttgttgttttggttttctattttgagatgaagtctcactctgtcgcccaggctgaagtgcagtggtgcgatcttggctcactgcaacctcctgctcccgaattcaagtgattctcctgcctcagcctcctgagtagctggaactacaggcatgcgctaccacgcctggctaatttttgtatttttagtagagatggggtttcaccatgttgaccaggttgttccggaactcaggtgatccaccttggcctcccaaagtgttgggattacaggcatgagccaccacactcggccagctgttgttaatagttaaaattataaattggacaaggtctgattccagcagggggagacaaattcacattgatttttctataagaaaaggaattatttgtactttcctcccttgtgtgtttgtgtgtatgtaagagagacagatgagaagagggctgcctttgagagccatgttccttttgcatgtacatacctctcaagattattacatgggtcttttagaagagggtcagtagctataaaagcaaatgatatttatgaaatgatttcattgtatgtggtttattatgtagtcttcaaaacagaaaaaccccacttgcttcgaaagcttcctttgagagctactttttaaccatattgttgatcaagcaagattcttaaagccccagtcctatacgtgagcagcattgaatccccggatactggcaggcgttcactgtccagcctttgacattagcatgtcaccctggtaaatcagagcactccatgccaaaaaacagcatggtctgctgagcacattaaggagcagagagggctcagaagaattaaacggccaatggggtggtgacagaggtgagctctttccccctcggacagcttggcatggtgactaccaatgaggtttaattgacattaagagcagctcaccatttttaaagagcgataaattgtttccaagtttcagcctcacggagccctgagctaagagataatgggctgacacatagcctcattggtcacgcttcacttgtaaacaggattggccaaagcaagaaggctgtaagtaaaggttggcccgtcctctggaagcctcccccacagcagggtggggaactggggcagccatagcaagcaggaccatcaggacacggtgtctcccaaacgggccggaacatacaaggttctacgtttaatagaaagttgatcaagccttcctctttggggagcctaatttttaagccattcactctctgttcccctgcagtcttttctctccaaactctgttgaaacttggaggcatctcgcttcctcctttggcctttgtagccaggttttcgcagcaaacagaccatatcatttaacacccacctgcttcttgttctgatagtcagttcagtagacagtagcattttttaagtcaaaaagaggcttagtgatgtaggccaaggtcaaggctctgtgtcatggggctctccccagggctcagtgccacggcacttcagacttgaccccagactgaaaagatgagaggacctgtagaagtcacggcctgtctgtcccgggcccatgctcctatctttttctcccccttggcatttagataccatggacttgttaaaatgtgacatgtactgatgatccttatgaatttgttggtaggggagctgctggtgaggattattttagactgtgagtaattgacctgacagacagtgatgactgcttcattaagagcccacgaccacgtgccagaatagttcagcatcctctgttgctactgtactttgagacatcgttcttctttgtgatgcaatacctctttcttgtcatgagggtctcttcccttaaatcaggtacatttcagattcttcaggtgatgttttttaggctgagtgtgttagcaccccttggaaaccaggttccctggggaaagtgtgtcacgtttgtggtgtttgcccgtatagctctcccacacccccacgagctccaagaggtggggaagcacatgtggcctgcctagcaggcaccagaagcaggttgtcggcacatgcaagccagctttgccctgttgcctgggggagaattgaaaagtttggccccaaaggggaaaattctttctgccatcaagttgctggtcagctgtcatggaacctgtctgcagcaatgtggctgtcacaaaacgcagcccaggacgagtatgcgctgaagctccattttgcattaactagtcaagtacttacccactgaaaagcacttcctgaaataatttcaccttcgtttttttccttctgcaggaggacaccatggaggtggaagagttcttgaaagaagctgcagtcatgaaagagatcaaacaccctaacctggtgcagctccttggtgagtaagcccggggctctgaagagagggtctcgcgccgcacccccagggtgacacaggcgctggggaagacgcacgggcggctcactgcacaaaacctcgttggaatatttgtgctctgccgacgttcagccgcgggtaaaatgaggcctgtatgggatgggtgtgtgcgtgtgtgcacatatgcacatgtatgtatgagagggagaatgtgattattttaagtggatacctaaaagcagtcaaatgcaaatctgaaattagtttctgaaacttgggcattttccagagttttctcactgaagtgattctgtaagtagacacataaccatcagacctaaccattcaggggtaaactgacggtggtgaaggtcatttgaggtggggccaggtctgcgtctgaattctgtggcagcctctccctgcgtaaattcaagttcactggcttgagaagaagaaaagagcctggccatgtccctcccacacgagcacagtctcaggatgcaggtgcttgggaccatgttggaagttgggcccaggactgaggagcagagtcagaatccttcagaaggctttttctttagacagttgtttgttcagttgggagcggagccacgtgttgaagtcctcgttgtcttgttggcaggggtctgcacccgggagcccccgttctatatcatcactgagttcatgacctacgggaacctcctggactacctgagggagtgcaaccggcaggaggtgaacgccgtggtgctgctgtacatggccactcagatctcgtcagccatggagtacctggagaagaaaaacttcatccacaggtaggggcctggccaggcagcctgcgccatggagtcacagggcgtggagccgggcagccttttacaaaaagccccagcctaggaggtctcagggcgcagcttctaacctcagtgctggcaacacattggaccttggaacaaaggcaaacactaggctcctggcaaagccagctttgggcatgcatccagggctaaattcagccaggcctagactctggaccagtggagcagctaatccccggagtaaggaatatttcatttttgaaccattttgggctaagtggaatattaaatgaagttcataaaaggcgtccttcctaataatcacagtcccctctgaaagagagtactcattgttcctccggggccagcgcccagcagtaatggcctcttcctgggagccgctggcattgcttttacgcaaactcatgggaacaaccagtacatggcttttgttttttagtgtgtgtgtctttttttcctgctttctctttattatcttttcattctccacttaacttgctgtcctctgattcagggatgtttccacaattgtcagaattgtgtatgtggaggtctaaattaagtgtctttgctgttttaaaccctgaagtgttttgaccttcaaatgtgccacaattatcttggtcttcaaattctttgctggtggaaatggcttcccagcaaagcgacggcctgtgcaggacagagcctgatgggctttgctggcgtcttttatacgagatgttctccacaccaccactgtgacctttcctacccaattagctcaagtatgaaacctctacatgagatttcatagcaaggaataagggtagcatgtgtgaaatgctggcggctccttgtaagacagattttctatgctccatgagagcctgatccagatactcctggctttcaggaaagtgaatcctctgatgctgcaaattgagattgcttgacttctggtttgcctggcacggccgggtccgttccttcttcattcaagcgaacttaaaatgctttatcaaaatcctcttaggcacaactcttctgtatttaatttcactcttgttgctgacgatcaggctatctcacgcagccatcacctcaagctgctgccccctctcattccgctcttcccgtttgccttgtgatttcatggttaatgttcatgaaccaaagattagactcctacctccctgggagaatcaggaagtgagaggaagcagattatacaggagagagttttttaggatacatttgggtacacctcaggaagaaagagggaagtaggaaacacagtttgggtaaagaatgccatgggctttgttttattttgtcccatcaagtctgaataggacaagtggagatgcactctgatagaagtttcttgcaatcaaggactgggctcagtgtttgtctccgtgcctggcatagagtagcaataactgcacttactattctcgacacttcaatcaaagcacttagcatattaattaattacactcacagcaaccctaagaggtaggtgccattattatcgtcttcattttacggatgaggtaactgagtcccagggtaattaacttgctccaggtcatgaggccagggagcccgctcccagcaccagcctctccccatgttgggatctcagggtgtgtttgctgagaggctggcactgtgttaattgccgtgggcattaatacaaacttccagggcattggactcaatctttccattgtcagcattgcacctttgctcagcagtggtggatttgtgaagtggaaggttggccaggagctctcatgggtgaacattttcctttcttagagatcttgctgcccgaaactgcctggtaggggagaaccacttggtgaaggtagctgattttggcctgagcaggttgatgacaggggacacctacacagcccatgctggagccaagttccccatcaaatggactgcacccgagagcctggcctacaacaagttctccatcaagtccgacgtctggggtaagggctgctgctgcactgaagtggtccttcctgactacaggagggtttttttctgcctctttcttgctcttccctttcttttcttcctttctttttgtttttttgagacggagtctcactctgtcacccaggctggagtgcagtggtgcaatcttggctcattgcagcctctccctcccgggttcaagcgattctcctgtctcagcatcttgagtagctgggattataggcacccgccaccacacccagctaatttttggtatttttagtagagatggggtttcaccatgttggccaggctggtctagaactcctgacctcaggtgatctgcctgccttggcctcccaaagtgctgggattacaggtgtgagccactgtgcacagccacccttttttttttttttttaactgtgtatttggcctgaggtccaaatatggtgcacagtgtatctgctgatctgttaagtctcctctataagccccctctccatgtctttatttcccttgctgtttattgaagaaaccatccttagagtttcgtacgttctgggttttgctcattgtctcccatggtgtgatttaatatgttcctctgacttcagtattcctagtaatgggtggctggatctggaacggcctcatcacattcaggtttgactgtttctcttttagtaagagtggatcaggggagatggtgtgcccttccatcagtagatacaaaatgcttcatttatttccttccttcctttcctcccctctccctcccctcctctcttctccttctccttccgacggagtttcgctcttgttgcccaggctggagtgcagtggcacgatcttggctcactgcaacctctgccttctggtttcaagcgattctcctgcctcagcctcctgagtagctgggattataggcgcatgccaccacccccggctaatttttgtatttttagtagagacggggttttaccatgttggccaggatggtctccaactcctgacttcgtgatccacccacctcggcctcccaaagtgctgggattacaggcgtgagccaccacgcctggccccaaaatgcttgatttgctatcgtttttttgtgggggtttttttttgagtaatttttggcagttactgatatacagtgcctagatccaatagtttgctaggtattgccaggtaggaattctctaattctgtcattcctgttaagttactagtggaaacttgtatgaggagaaacagttcctcatctgtgtggttactcagtggtacagttcatgtaggaagagcagggtcaattcttgcttctttgtttttatttaccagtttttaaaataacaaattactttttcttttttttttttggagccagagtcttgctttttctggggtacaaagtacaggctggagttcagtagcatgatctcggctcactgcaacctccgcctaccagattcaagcaattcttctgcctcagcctcccaagtagctgggattacaggtgcctgccaccacgcctggctaaatttttttgtatttttagtaaagatggggtttcaccatgttgcccaggctggccttgaacttctgagctcaggcagtccacctgccttggcctcccaaagtgctgggattacaggcgtgagccaccatgccctgccacaagttggtttcttttttttttttttttttttttttttttgagacagtctcactctgtcgcccaggctggagtgcagtggcgcgatcttgatcttggctcactgcaagctccacctcctgggttcacaccattctcctgcctcagcctcccgagtagctgggactataggcatctaccaccacgcccggctaatttttttgtatttttagtagagacagggtttcaccatgttagccaggatggtctcaatctcctgacctcgtgatccgcccgcctcggcctcccaaagtgctgggattacaggtgtgagccaccgtgcccggcccctaatttttgtatttttagtagagatggggtttcgccatgttggccagggtggtcttgaattcctgacctcaaataatcctcccacttcagcctcccaaagtgctgggattacaggcgtgagccaccgcacccagccttgtcctggtcttctgatgataaagagcctggtaaaatgtcagagcctgggctgctgctggggccatcccttctgaggtctgctgcaaaggtaactgattttaaatgtagtgtagtgaaatgctacacatcttgaacagcctttctctttcggttttctttcagcatttggagtattgctttgggaaattgctacctatggcatgtccccttacccgggaattgacctgtcccaggtgtatgagctgctagagaaggactaccgcatggagcgcccagaaggctgcccagagaaggtctatgaactcatgcgagcatgtaagccttcctcagcctgttctcacgagtatatgtgggcattccaggaaattcaactgtgcaggagtgtgtacacaaagttgaaagtttttccatgagctctctccattccagttcttcagatgcagctaatgtagccatttgatacctattgacctttatttacagataaatagtatgtgcgtgacttgtcttttaaagcaaaaatggtattgatagataccaaacctgggtgtattcctaaatacagattcctgggccctgctttcacagacattctgctatagtagctaagctcatgaggtgattttttttttttttttttttgagacggagtttcgctcttgtcgcccaggctggagtacaatggcgcaatgttggctcacttcaacctccacctccctggttcaagcgattctcctgcctcagcctcccaagtagctgggattacaggcatgcaccaccacgcccggctaattttgtatttttagtagagatggggtttctccatgttagtcaggctggtctccaactcccaacctcaggtgatctgcctgcctcggcctcccaaagtgctgcgattacaggcgtgagccaccacgcccagctgcgaggtgatttttatctggtcgttttatactgattacatatgtgttatctgtactatgcacacacaggatgttttcatatatcttataaggtatttatatggccatttcttacactgttttcccacacatgtctttccacgtccatatattcagatctctccctctccctacctcttatttatgtatagctgcccagtactccatttcactcattcatccggtcctcttttgatgtgcatttggttgttttacacatttgtttggtttttgcccttataaacaaagcagaaacaaatattcatgtacacgaatctctgggcactttggctggtatttctaaaagttgaactgttggttccaagaactgtgtgggttttaaattttgatacattttaccaaactgttaaaaaaggttgtgccattgtatgctccagtcagacgcatatgggagtgactgttcctggtccccagtactaggctttgtcagtctgtttagtcctcatgttagtctcattttcatgagaatttctttacttcagactttgataaccgtgaagaaagaacaagatagaaggtgagctgtttggcttagtaattttctacacctactagagcgggactgggaaaaatatatttgtaaatgcagttcttgctgtcactgtctctctggggttttacaatccatattcctgccagcatctaacgtcttttcaaattcttaatgtctataacaggacatgatgacattcatcgttttgacttgttgcagcaaaagatggttagcaggattggaatgttgctttcattctagacttttccttgagaactgctagccccgtattgctagccagatctcatggatgatctgacttgggtttcatctgtccaggttggcagtggaatccctctgaccggccctcctttgctgaaatccaccaagcctttgaaacaatgttccaggaatccagtatctcagacggtaaagtacccatcccggggtacctgcagtggggtgaaagggcagccatgtgggactgcagcctgggtcattcggttcacttcctggtgaaagttcacagaccagcctgtcctgagaccagaaagctgggcagaggtgtggagtattgtgctttcttgtctgctgcagccctgcagagttctaagaaatgctaagggctgtttctccggtatccacgtgccttttctttagttgtatgcagatgagcactgttaccttacaaagaaagagaaccaccacaccaagccaacaccagtactgatggctgctggatttttgtttctgtccctgtatgattcttagaagtggaaaaggagctggggaaacaaggcgtccgtggggctgtgagtaccttgctgcaggccccagagctgcccaccaagacgaggacctccaggagagctgcagagcacagagacaccactgacgtgcctgagatgcctcactccaagggccagggagagagcggtaagtcccccgcttcccccaaccccactgctcttcccttccctgccagaggctacattcaggccatcataggccaacgggaagctgtgaatggagcccgcacagaagggcagccatggcctttgtcaatggttcagcttcggaaggaggaaggttctcctctccccacctgcctcctatcccctccctctgagagtccccgaggagcataggctccagcagtgagttcagtcctgtaggcagaggtgcttctgaagcccgccaaggagctagcccatctcccacctattacccgcggcatctgtggttgctgtctcagagcagattcaacaatagtaagcaccaggctgcgtgacaagcagctcacggtgaaggcactgatgtgagaagctcgctgcagccaggtggaaccaggacacgcacatggacagaacccgtgtcctggtggtctctgggaagagcatctttctggtgccattgcctaggcgagcaagggagttgggatcagctcaggagggggtctcaagacactagcaaaaataataatggccaacatttatgtagtgtgcctactacaggccaggctctgttctatgttcatggttgacccccagaaccagcagtccaggttctgctgcagaccagctgaacaaaagcattgaggggtgtattagtctgttttcatgctgctaataaaggtatacccaagactgggtaatttataaaggaaagaggtttcaccgactcacagttccacatggctggggaggcctcacaatcatggctgaaggtgaatgaggagcaaggtcacatcttacttggcggcaggcaagagagcttgtgcaggggaagtccgctttataaaaccatcagatctcgtgagacttattcactaccacgagaatgtgggagaaacctccccatgattcattgatctccacctgaccccaccgttgacacgtggggcttattacaattcaaggtgagatttgggtggggactcagccaacccatattggaggtgggggataggccaagcatctgggttcatagaggatcctggggatggcaatggtggactccattctaatggactgcagactgggtacatgtgaagggactggacaaagccctacttcttgaagatttatggtgggatgtttactgacagcagaatctataaacctgagttttctttatcacgtactctcattagtaaaaaaaaaaaaaaaaaacagaacatgcagcccatatatatggtatataaagtacgtatgtccactactgtaggagtagagtgcgtatgttatgtaccaaaacgcacatttaaaaggcttgcatgctaaataagtccaaatttgcaatacttcccgccccgctgggccatctcactcacctacttggaggttatggcgtatagactctccagaatcttccacccttcctcctcttatcggttttcctgatttcaggtggctgagcagtagggaggagaggcctctgggaacgctgtgcttattaagaacccagtgatcagcagtcatgttcatttacgcccgtcagtttcatctgaggggtattttgatagtgatctcttggtgagccgagggtgtcaattaactgctcagtgctgaaactgagtggtgcataattcattgcaatttcactctcctggcctccttccactagattaaagttttgggagggctttggtgttccctgattcagatgtcccgcgtgctgccttgggttctgataaatgcatactggtacctctgttgagttacaggtgccaacagaaaacctcttcttgcaagctgacctctgagggagaattctgttactcactagcaggagcttggcaacaccaaaaagatttccttttttttttgagatggagtctcactctgttgccaggctggagtgcaatggcatgataccagctcactgcaacctccacctcctgggttcaagcgattctcctgcctcatcctcctgagtagctgggactacaggcgtgtgccaccacacccagctaatttttgcattttttagtagagacggggtttcaccatgttggccaggatggtctctatctcttgacctcatgatccgcccacctcagcctcccaaagtgctgggatgacaggcttgagccaccgcgcctggctaccagaaagatttcttatgagctatgattcatatttaaagagtgcccattaaaaaactgttggccgggcgtggtggctcacacctgtaatcccagcactttaggaggccgaggtcagcgaatcacaaggtcaggctcccgtggcacaagctgggggctgcccccaccccatgctccccagaggagcacccaagcgtctgggctcagacaggcctggatctgataaccggctctgatgccaccatccctgaggccaggcaagtcccagccgggctacagcactgttgtgagaatgcagatgaggttgtaaaggtgaagcacgtgtcacgcttctctcaataaagccatcattgctgttaggattgtcattaggaaaggctttgggccgggtgcagtggctcatgcctgtaatcccagcactttgggaggccaaggcgggtggatcacctgaggtcaggagtttgagaccagcctaaccaacatggtgaaaccccgtctctactaaaaatacaaaattagccaggcgtggtagcgggtgcctatagtcctagctacttgggaggctgaggcaagagaaccatttgaacctgggaggcggaggttgcagtgagctgagatcgtgccactgcactccagcgtaggcaacaagcgagactccaactcaaaaaaaaaaaaaaaccacacacacgctttggtctctttccctgaagatgggaacaaaaagctggacggccctggcctcttcatccctgcactggtttacttgaaggcagcagccccccacccacccacatcactctctagtgagtataaaaacgatgacaaggccaagcaaagggtcaaaacctgtggctctcctgccagccagctagccgagaggcctatgaggagctctgggaataaggggctgtgtcccacagtggggaagggacaatgggccattatgcacaggagataagaagggatgacctttgacaatttttttgtttgtttgtttgtttgttttgagatggagtctcactctgtctcctgggctggagtgcagcagtggcactctgcctcccgggttcaagcgattctcctctgtcagcctctagagttgtctggagttgtcagctcttccccttgcgtttcagatcctctggaccatgagcctgccgtgtctccattgctccctcgaaaagagcgaggtcccccggagggcggcctgaatgaagatgagcgccttctccccaaagacaaaaagaccaacttgttcagcgccttgatcaagaagaagaagaagacagccccaacccctcccaaacgcagcagctccttccgggagatggacggccagccggagcgcagaggggccggcgaggaagagggccgagacatcagcaacggggcactggctttcacccccttggacacagctgacccagccaagtccccaaagcccagcaatggggctggggtccccaatggagccctccgggagtccgggggctcaggcttccggtctccccacctgtggaagaagtccagcacgctgaccagcagccgcctagccaccggcgaggaggagggcggtggcagctccagcaagcgcttcctgcgctcttgctccgcctcctgcgttccccatggggccaaggacacggagtggaggtcagtcacgctgcctcgggacttgcagtccacgggaagacagtttgactcgtccacatttggagggcacaaaagtgagaagccggctctgcctcggaagagggcaggggagaacaggtctgaccaggtgacccgaggcacagtaacgcctccccccaggctggtgaaaaagaatgaggaagctgctgatgaggtcttcaaagacatcatggagtccagcccgggctccagcccgcccaacctgactccaaaacccctccggcggcaggtcaccgtggcccctgcctcgggcctcccccacaaggaagaagctggaaagggcagtgccttagggacccctgctgcagctgagccagtgacccccaccagcaaagcaggctcaggtgcaccagggggcaccagcaagggccccgccgaggagtccagagtgaggaggcacaagcactcctctgagtcgccagggagggacaaggggaaattgtccaggctcaaacctgccccgccgcccccaccagcagcctctgcagggaaggctggaggaaagccctcgcagagcccgagccaggaggcggccggggaggcagtcctgggcgcaaagacaaaagccacgagtctggttgatgctgtgaacagtgacgctgccaagcccagccagccgggagagggcctcaaaaagcccgtgctcccggccactccaaagccacagtccgccaagccgtcggggacccccatcagcccagcccccgttccctccacgttgccatcagcatcctcggccctggcaggggaccagccgtcttccaccgccttcatccctctcatatcaacccgagtgtctcttcggaaaacccgccagcctccagagcggatcgccagcggcgccatcaccaagggcgtggtcctggacagcaccgaggcgctgtgcctcgccatctctaggaactccgagcagatggccagccacagcgcagtgctggaggccggcaaaaacctctacacgttctgcgtgagctatgtggattccatccagcaaatgaggaacaagtttgccttccgagaggccatcaacaaactggagaataatctccgggagcttcagatctgcccggcgacagcaggcagtggtccggcggccactcaggacttcagcaagctcctcagttcggtgaaggaaatcagtgacatagtgcagaggtagcagcagtcaggggtcaggtgtcaggcccgtcggagctgcctgcagcacatgcgggctcgcccatacccgtgacagtggctgacaagggactagtgagtcagcaccttggcccaggagctctgcgccaggcagagctgagggccctgtggagtccagctctactacctacgtttgcaccgcctgccctcccgcaccttcctcctccccgctccgtctctgtcctcgaattttatctgtggagttcctgctccgtggactgcagtcggcatgccaggacccgccagccccgctcccacctagtgccccagactgagctctccaggccaggtgggaacggctgatgtggactgtctttttcatttttttctctctggagcccctcctcccccggctgggcctccttcttccacttctccaagaatggaagcctgaactgaggccttgtgtgtcaggccctctgcctgcactccctggccttgcccgtcgtgtgctgaagacatgtttcaagaaccgcatttcgggaagggcatgcacgggcatgcacacggctggtcactctgccctctgctgctgcccggggtggggtgcactcgccatttcctcacgtgcaggacagctcttgatttgggtggaaaacagggtgctaaagccaaccagcctttgggtcctgggcaggtgggagctgaaaaggatcgaggcatggggcatgtcctttccatctgtccacatccccagagcccagctcttgctctcttgtgacgtgcactgtgaatcctggcaagaaagcttgagtctcaagggtggcaggtcactgtcactgccgacatccctcccccagcagaatggaggcaggggacaagggaggcagtggctagtggggtgaacagctggtgccaaatagccccagactgggcccaggcaggtctgcaagggcccagagtgaaccgtcctttcacacatctgggtgccctgaaagcccttcccctcccccactcctctaagacaaagtagattcttacaaggccctttcctttggaacaagacagccttcacttttctgagttcttgaagcatttcaaagccctgcctctgtgtagccgccctgagagagaatagagctgccactgggcacctgcgcacaggtgggaggaaagggcctggccagtcctggtcctggctgcactcttgaactgggcgaatgtcttatttaattaccgtgagtgacatagcctcatgttctgtgggggtcatcagggagggttaggaaaaccacaaacggagcccctgaaagcctcacgtatttcacagagcacgcctgccatcttctccccgaggctgccccaggccggagcccagatacgggggctgtgactctgggcagggacccggggtctcctggaccttgacagagcagctaactccgagagcagtgggcaggtggccgcccctgaggcttcacgccgggagaagccaccttcccaccccttcataccgcctcgtgccagcagcctcgcacaggccctagctttacgctcatcacctaaacttgtactttatttttctgatagaaatggtttcctctggatcgttttatgcggttcttacagcacatcacctctttgcccccgacggctgtgacgcagccggagggaggcactagtcaccgacagcggccttgaagacagagcaaagcgcccacccaggtcccccgactgcctgtctccatgaggtactggtcccttccttttgttaatgtgatgtgccactatattttacacgtatctcttggtatgcatcttttatagacgctcttttctaagtggcgtgtgcatagcgtcctgccctgccccctcgggggcctgtggtggctccccctctgcttctcggggtccagtgcattttgtttctgtatatgattctctgtggttttttttgaatccaaatctgtcctctgtagtattttttaaataaatcagtgtttacattagaattcttggcagattgcttcggcctgtgatcctgccctgttgttctgagcctgtgcggtggcggggccgggatgtagtgggttctggtttcccgacggggctggggcccggcatcaggtcttacagagcagaacggtggcaggttgcccccagctgcccagggcctctgcggcctgggtgcccacagccatctttcaggcacttgccctgctatgctcggaccctttctgtacccttggcgcttacctgctggcagcctggccccaccggcatcactgggagtgggctgtgccaccatacaagccacatctgactggcggtatcaggctgtcgcagcgacgtggaagtggggtgaggaggtcacgtcccgtgcttcttgctggctgagggcaaatccctccccacgtgcgcctgttctctctccacctttccgccctaagcccccaggtgcccttactcactcatgttccttgagccaggtgtcttaggtctttgtgtggatgaggaggagcggaggtgtgaggtgtgctgggccttcagggcctgggaaggccatcccagactgagccccaccgccctttcccagctcagtccccaccgagctgacagcttggaaaggggcggttgggaagtgagtagcaccctctgataatgatactgatcaggccagcaggtttgtcaggggtgcacatcctgctcagcagagcatatgaagatcacagcttggtgaagctccactcgagagacctggagcgagactgctgtgcggtgggtgacaggtggaactccagccgggccggggctggtggagcccactgcgagcagtgccaggcacaagattctccccctctcatttcacagggacaaaaccaggctggggcccccaatttccttgccggttgaaccatagctggccaccagatccaccaagcctggggcttctcttgtcctttgaatggctgcttctcccaggtctgaacgaagacataggacaactctggtgacagccacagctggtggccgcttcctcgtgtcagatgtggacggtcaccccgccctcccagcgctaagcgctgagactgcgtgtccagagtcggctcctgcacgtgaggccaattggtcacactgggccagtgtggaggaagatgcctctcatctcccaaatggggatctttcatgggtgtcacctgagcttatagagcttagtttagtctagccattccaagacagtggtttcttaaccttttctaggtcacaaaacctcctgagaacctaatgaaaactggatcccagccccagaaaaatgcacctgtgtgcacacacccagcagtttccaggtcatttcgagtcctgccttcgaggtccattgttattatttacaaaacaccagcctaaggtattggacattttcttaaaaggccaggcaaggtggctcatgcctgtaatcccaacactttgggaggctgaggtgggtggattgcttgaggccgggagttcaagaccagcctgggcaacatagaccccatctcacaaaaaatacaaaaacaagctgggtatggtggcacctgtagtccagctactcaggaagctgaggtgggaggattgcttgagcccaggaggtggaggttgcagcaagctatgatcgtgccactggattccagctccagagtgagaccctgtctcaaaaaaaatttttttttcttttttctttttgagacagagtttcgctcttgtctcccaggctggagtgcaatggcacaatctccgctcactgcaacctctgcctcctgggttcaagcgattctcctgcctcagcctcccgagtagctgggactagaggtgcgcaccaccagacccggctaatttttgtatttttagtagggacggagtttcaccatgttggtcaggatggtctcgatctcttgacctcatgatccgcccaccttggactcccaaagtgcttggattacaggcatgagccagcgcgcccggcccaccactttttttttttttttttttttttaagacgagtctcacactgtcgcccagtctgtagtgcagtggtgccatctcggctcactgcaagctccgcctcccaggttcata